European Patent Specification EP 4 039 800 B1, published October 25, 2023. Title: An Engineered Multi-component System for Identification and Characterisation of T-cell receptors and T-cell antigens. Applicant: Genovie AB. The sequence listing filed with the application follows.

SEQUENCE LISTING (72 sequences)

SEQ ID NO: 1 - protein, 13 aa, Homo sapiens
  Analyte Antigenic Molecule
PKYVKQNTLKLAT

SEQ ID NO: 2 - protein, 4 aa, Homo sapiens
  Analyte Antigenic Molecule
PKYV

SEQ ID NO: 3 - protein, 17 aa, Homo sapiens
  Analyte Antigenic Molecule, APD-2
NLVPMVATNLVPMVATV

SEQ ID NO: 4 - protein, 9 aa, Homo sapiens
  Analyte Antigenic Molecule, APD-21
NLGPMAAGV

SEQ ID NO: 5 - protein, 9 aa, Homo sapiens
  Analyte Antigenic Molecule, APD-11
VYALPLKML

SEQ ID NO: 6 - DNA, 6071 bp, Artificial Sequence
  V1.A.4 pcDNA3.1_GFP
gacggatcgggagatctcccgatcccctatggtgcactctcagtacaatctgctctgatgccgcatagttaagccagtatctgctccctgcttgtgtgttggaggtcgctgagtagtgcgcgagcaaaatttaagctacaacaaggcaaggcttgaccgacaattgcatgaagaatctgcttagggttaggcgttttgcgctgcttcgcgatgtacgggccagatatacgcgttgacattgattattgactagttattaatagtaatcaattacggggtcattagttcatagcccatatatggagttccgcgttacataacttacggtaaatggcccgcctggctgaccgcccaacgacccccgcccattgacgtcaataatgacgtatgttcccatagtaacgccaatagggactttccattgacgtcaatgggtggagtatttacggtaaactgcccacttggcagtacatcaagtgtatcatatgccaagtacgccccctattgacgtcaatgacggtaaatggcccgcctggcattatgcccagtacatgaccttatgggactttcctacttggcagtacatctacgtattagtcatcgctattaccatggtgatgcggttttggcagtacatcaatgggcgtggatagcggtttgactcacggggatttccaagtctccaccccattgacgtcaatgggagtttgttttggcaccaaaatcaacgggactttccaaaatgtcgtaacaactccgccccattgacgcaaatgggcggtaggcgtgtacggtgggaggtctatataagcagagctctctggctaactagagaacccactgcttactggcttatcgaaattaatacgactcactatagggagacccaagctggctagcgtttaaacttaagcttggtaccgccaccatggaatccgatgagtctggcctgcccgccatggaaatcgagtgcagaatcaccggcaccctgaacggcgtggaatttgagctcgtgggcggaggcgagggcacacctgaacagggcagaatgaccaacaagatgaagtccaccaagggggccctgaccttcagcccctacctgctgtctcacgtgatgggctacggcttctaccacttcggcacctaccccagcggctacgagaaccctttcctgcacgccatcaacaacggcggctacaccaacacccggatcgagaagtacgaggacggcggcgtgctgcacgtgtccttcagctacagatacgaggccggcagagtgatcggcgacttcaaagtgatgggcaccggattccccgaggacagcgtgatcttcaccgacaagatcatccggtccaacgccaccgtggaacatctgcaccccatgggcgacaacgacctggacggcagcttcaccagaaccttctccctgcgggatggcggctactacagcagcgtggtggacagccacatgcacttcaagagcgccatccaccccagcatcctccagaacggcggacccatgttcgccttcagacgggtggaagaggaccacagcaacaccgagctgggcatcgtggaataccagcacgccttcaagacccccgatgccgatgccggcgaggaatgagtcgagtctagagggcccgtttaaacccgctgatcagcctcgactgtgccttctagttgccagccatctgttgtttgcccctcccccgtgccttccttgaccctggaaggtgccactcccactgtcctttcctaataaaatgaggaaattgcatcgcattgtctgagtaggtgtcattctattctggggggtggggtggggcaggacagcaagggggaggattgggaagacaatagcaggcatgctggggatgcggtgggctctatggcttctgaggcggaaagaaccagctggggctctagggggtatccccacgcgccctgtagcggcgcattaagcgcggcgggtgtggtggttacgcgcagcgtgaccgctacacttgccagcgccctagcgcccgctcctttcgctttcttcccttcctttctcgccacgttcgccggctttccccgtcaagctctaaatcgggggctccctttagggttccgatttagtgctttacggcacctcgaccccaaaaaacttgattagggtgatggttcacgtagtgggccatcgccctgatagacggtttttcgccctttgacgttggagtccacgttctttaatagtggactcttgttccaaactggaacaacactcaaccctatctcggtctattcttttgatttataagggattttgccgatttcggcctattggttaaaaaatgagctgatttaacaaaaatttaacgcgaattaattctgtggaatgtgtgtcagttagggtgtggaaagtccccaggctccccagcaggcagaagtatgcaaagcatgcatctcaattagtcagcaaccaggtgtggaaagtccccaggctccccagcaggcagaagtatgcaaagcatgcatctcaattagtcagcaaccatagtcccgcccctaactccgcccatcccgcccctaactccgcccagttccgcccattctccgccccatggctgactaattttttttatttatgcagaggccgaggccgcctctgcctctgagctattccagaagtagtgaggaggcttttttggaggcctaggcttttgcaaaaagctcccgggagcttgtatatccattttcggatctgatcaagagacaggatgaggatcgtttcgcatgattgaacaagatggattgcacgcaggttctccggccgcttgggtggagaggctattcggctatgactgggcacaacagacaatcggctgctctgatgccgccgtgttccggctgtcagcgcaggggcgcccggttctttttgtcaagaccgacctgtccggtgccctgaatgaactgcaggacgaggcagcgcggctatcgtggctggccacgacgggcgttccttgcgcagctgtgctcgacgttgtcactgaagcgggaagggactggctgctattgggcgaagtgccggggcaggatctcctgtcatctcaccttgctcctgccgagaaagtatccatcatggctgatgcaatgcggcggctgcatacgcttgatccggctacctgcccattcgaccaccaagcgaaacatcgcatcgagcgagcacgtactcggatggaagccggtcttgtcgatcaggatgatctggacgaagagcatcaggggctcgcgccagccgaactgttcgccaggctcaaggcgcgcatgcccgacggcgaggatctcgtcgtgacccatggcgatgcctgcttgccgaatatcatggtggaaaatggccgcttttctggattcatcgactgtggccggctgggtgtggcggaccgctatcaggacatagcgttggctacccgtgatattgctgaagagcttggcggcgaatgggctgaccgcttcctcgtgctttacggtatcgccgctcccgattcgcagcgcatcgccttctatcgccttcttgacgagttcttctgagcgggactctggggttcgaaatgaccgaccaagcgacgcccaacctgccatcacgagatttcgattccaccgccgccttctatgaaaggttgggcttcggaatcgttttccgggacgccggctggatgatcctccagcgcggggatctcatgctggagttcttcgcccaccccaacttgtttattgcagcttataatggttacaaataaagcaatagcatcacaaatttcacaaataaagcatttttttcactgcattctagttgtggtttgtccaaactcatcaatgtatcttatcatgtctgtataccgtcgacctctagctagagcttggcgtaatcatggtcatagctgtttcctgtgtgaaattgttatccgctcacaattccacacaacatacgagccggaagcataaagtgtaaagcctggggtgcctaatgagtgagctaactcacattaattgcgttgcgctcactgcccgctttccagtcgggaaacctgtcgtgccagctgcattaatgaatcggccaacgcgcggggagaggcggtttgcgtattgggcgctcttccgcttcctcgctcactgactcgctgcgctcggtcgttcggctgcggcgagcggtatcagctcactcaaaggcggtaatacggttatccacagaatcaggggataacgcaggaaagaacatgtgagcaaaaggccagcaaaaggccaggaaccgtaaaaaggccgcgttgctggcgtttttccataggctccgcccccctgacgagcatcacaaaaatcgacgctcaagtcagaggtggcgaaacccgacaggactataaagataccaggcgtttccccctggaagctccctcgtgcgctctcctgttccgaccctgccgcttaccggatacctgtccgcctttctcccttcgggaagcgtggcgctttctcatagctcacgctgtaggtatctcagttcggtgtaggtcgttcgctccaagctgggctgtgtgcacgaaccccccgttcagcccgaccgctgcgccttatccggtaactatcgtcttgagtccaacccggtaagacacgacttatcgccactggcagcagccactggtaacaggattagcagagcgaggtatgtaggcggtgctacagagttcttgaagtggtggcctaactacggctacactagaagaacagtatttggtatctgcgctctgctgaagccagttaccttcggaaaaagagttggtagctcttgatccggcaaacaaaccaccgctggtagcggtttttttgtttgcaagcagcagattacgcgcagaaaaaaaggatctcaagaagatcctttgatcttttctacggggtctgacgctcagtggaacgaaaactcacgttaagggattttggtcatgagattatcaaaaaggatcttcacctagatccttttaaattaaaaatgaagttttaaatcaatctaaagtatatatgagtaaacttggtctgacagttaccaatgcttaatcagtgaggcacctatctcagcgatctgtctatttcgttcatccatagttgcctgactccccgtcgtgtagataactacgatacgggagggcttaccatctggccccagtgctgcaatgataccgcgagacccacgctcaccggctccagatttatcagcaataaaccagccagccggaagggccgagcgcagaagtggtcctgcaactttatccgcctccatccagtctattaattgttgccgggaagctagagtaagtagttcgccagttaatagtttgcgcaacgttgttgccattgctacaggcatcgtggtgtcacgctcgtcgtttggtatggcttcattcagctccggttcccaacgatcaaggcgagttacatgatcccccatgttgtgcaaaaaagcggttagctccttcggtcctccgatcgttgtcagaagtaagttggccgcagtgttatcactcatggttatggcagcactgcataattctcttactgtcatgccatccgtaagatgcttttctgtgactggtgagtactcaaccaagtcattctgagaatagtgtatgcggcgaccgagttgctcttgcccggcgtcaatacgggataataccgcgccacatagcagaactttaaaagtgctcatcattggaaaacgttcttcggggcgaaaactctcaaggatcttaccgctgttgagatccagttcgatgtaacccactcgtgcacccaactgatcttcagcatcttttactttcaccagcgtttctgggtgagcaaaaacaggaaggcaaaatgccgcaaaaaagggaataagggcgacacggaaatgttgaatactcatactcttcctttttcaatattattgaagcatttatcagggttattgtctcatgagcggatacatatttgaatgtatttagaaaaataaacaaataggggttccgcgcacatttccccgaaaagtgccacctgacgtc

SEQ ID NO: 7 - DNA, 10428 bp, Artificial Sequence
  SpCas9-2A-GFP Vector V1.A.8
gacggatcgggagatctcccgatcccctatggtgcactctcagtacaatctgctctgatgccgcatagttaagccagtatctgctccctgcttgtgtgttggaggtcgctgagtagtgcgcgagcaaaatttaagctacaacaaggcaaggcttgaccgacaattgcatgaagaatctgcttagggttaggcgttttgcgctgcttcgcgatgtacgggccagatatacgcgttgacattgattattgactagttattaatagtaatcaattacggggtcattagttcatagcccatatatggagttccgcgttacataacttacggtaaatggcccgcctggctgaccgcccaacgacccccgcccattgacgtcaataatgacgtatgttcccatagtaacgccaatagggactttccattgacgtcaatgggtggagtatttacggtaaactgcccacttggcagtacatcaagtgtatcatatgccaagtacgccccctattgacgtcaatgacggtaaatggcccgcctggcattatgcccagtacatgaccttatgggactttcctacttggcagtacatctacgtattagtcatcgctattaccatggtgatgcggttttggcagtacatcaatgggcgtggatagcggtttgactcacggggatttccaagtctccaccccattgacgtcaatgggagtttgttttggcaccaaaatcaacgggactttccaaaatgtcgtaacaactccgccccattgacgcaaatgggcggtaggcgtgtacggtgggaggtctatataagcagagctctctggctaactagagaacccactgcttactggcttatcgaaattaatacgactcactatagggagacccaagctggctagcgtttaaacttaagcttggtaccgccaccatggactataaggaccacgacggagactacaaggatcatgatattgattacaaagacgatgacgataagatggccccaaagaagaagcggaaggtcggtatccacggagtcccagcagccgacaagaagtacagcatcggcctggacatcggcaccaactctgtgggctgggccgtgatcaccgacgagtacaaggtgcccagcaagaaattcaaggtgctgggcaacaccgaccggcacagcatcaagaagaacctgatcggagccctgctgttcgacagcggcgaaacagccgaggccacccggctgaagagaaccgccagaagaagatacaccagacggaagaaccggatctgctatctgcaagagatcttcagcaacgagatggccaaggtggacgacagcttcttccacagactggaagagtccttcctggtggaagaggataagaagcacgagcggcaccccatcttcggcaacatcgtggacgaggtggcctaccacgagaagtaccccaccatctaccacctgagaaagaaactggtggacagcaccgacaaggccgacctgcggctgatctatctggccctggcccacatgatcaagttccggggccacttcctgatcgagggcgacctgaaccccgacaacagcgacgtggacaagctgttcatccagctggtgcagacctacaaccagctgttcgaggaaaaccccatcaacgccagcggcgtggacgccaaggccatcctgtctgccagactgagcaagagcagacggctggaaaatctgatcgcccagctgcccggcgagaagaagaatggcctgttcggaaacctgattgccctgagcctgggcctgacccccaacttcaagagcaacttcgacctggccgaggatgccaaactgcagctgagcaaggacacctacgacgacgacctggacaacctgctggcccagatcggcgaccagtacgccgacctgtttctggccgccaagaacctgtccgacgccatcctgctgagcgacatcctgagagtgaacaccgagatcaccaaggcccccctgagcgcctctatgatcaagagatacgacgagcaccaccaggacctgaccctgctgaaagctctcgtgcggcagcagctgcctgagaagtacaaagagattttcttcgaccagagcaagaacggctacgccggctacattgacggcggagccagccaggaagagttctacaagttcatcaagcccatcctggaaaagatggacggcaccgaggaactgctcgtgaagctgaacagagaggacctgctgcggaagcagcggaccttcgacaacggcagcatcccccaccagatccacctgggagagctgcacgccattctgcggcggcaggaagatttttacccattcctgaaggacaaccgggaaaagatcgagaagatcctgaccttccgcatcccctactacgtgggccctctggccaggggaaacagcagattcgcctggatgaccagaaagagcgaggaaaccatcaccccctggaacttcgaggaagtggtggacaagggcgcttccgcccagagcttcatcgagcggatgaccaacttcgataagaacctgcccaacgagaaggtgctgcccaagcacagcctgctgtacgagtacttcaccgtgtataacgagctgaccaaagtgaaatacgtgaccgagggaatgagaaagcccgccttcctgagcggcgagcagaaaaaggccatcgtggacctgctgttcaagaccaaccggaaagtgaccgtgaagcagctgaaagaggactacttcaagaaaatcgagtgcttcgactccgtggaaatctccggcgtggaagatcggttcaacgcctccctgggcacataccacgatctgctgaaaattatcaaggacaaggacttcctggacaatgaggaaaacgaggacattctggaagatatcgtgctgaccctgacactgtttgaggacagagagatgatcgaggaacggctgaaaacctatgcccacctgttcgacgacaaagtgatgaagcagctgaagcggcggagatacaccggctggggcaggctgagccggaagctgatcaacggcatccgggacaagcagtccggcaagacaatcctggatttcctgaagtccgacggcttcgccaacagaaacttcatgcagctgatccacgacgacagcctgacctttaaagaggacatccagaaagcccaggtgtccggccagggcgatagcctgcacgagcacattgccaatctggccggcagccccgccattaagaagggcatcctgcagacagtgaaggtggtggacgagctcgtgaaagtgatgggccggcacaagcccgagaacatcgtgatcgaaatggccagagagaaccagaccacccagaagggacagaagaacagccgcgagagaatgaagcggatcgaagagggcatcaaagagctgggcagccagatcctgaaagaacaccccgtggaaaacacccagctgcagaacgagaagctgtacctgtactacctgcagaatgggcgggatatgtacgtggaccaggaactggacatcaaccggctgtccgactacgatgtggaccatatcgtgcctcagagctttctgaaggacgactccatcgacaacaaggtgctgaccagaagcgacaagaaccggggcaagagcgacaacgtgccctccgaagaggtcgtgaagaagatgaagaactactggcggcagctgctgaacgccaagctgattacccagagaaagttcgacaatctgaccaaggccgagagaggcggcctgagcgaactggataaggccggcttcatcaagagacagctggtggaaacccggcagatcacaaagcacgtggcacagatcctggactcccggatgaacactaagtacgacgagaatgacaagctgatccgggaagtgaaagtgatcaccctgaagtccaagctggtgtccgatttccggaaggatttccagttttacaaagtgcgcgagatcaacaactaccaccacgcccacgacgcctacctgaacgccgtcgtgggaaccgccctgatcaaaaagtaccctaagctggaaagcgagttcgtgtacggcgactacaaggtgtacgacgtgcggaagatgatcgccaagagcgagcaggaaatcggcaaggctaccgccaagtacttcttctacagcaacatcatgaactttttcaagaccgagattaccctggccaacggcgagatccggaagcggcctctgatcgagacaaacggcgaaaccggggagatcgtgtgggataagggccgggattttgccaccgtgcggaaagtgctgagcatgccccaagtgaatatcgtgaaaaagaccgaggtgcagacaggcggcttcagcaaagagtctatcctgcccaagaggaacagcgataagctgatcgccagaaagaaggactgggaccctaagaagtacggcggcttcgacagccccaccgtggcctattctgtgctggtggtggccaaagtggaaaagggcaagtccaagaaactgaagagtgtgaaagagctgctggggatcaccatcatggaaagaagcagcttcgagaagaatcccatcgactttctggaagccaagggctacaaagaagtgaaaaaggacctgatcatcaagctgcctaagtactccctgttcgagctggaaaacggccggaagagaatgctggcctctgccggcgaactgcagaagggaaacgaactggccctgccctccaaatatgtgaacttcctgtacctggccagccactatgagaagctgaagggctcccccgaggataatgagcagaaacagctgtttgtggaacagcacaagcactacctggacgagatcatcgagcagatcagcgagttctccaagagagtgatcctggccgacgctaatctggacaaagtgctgtccgcctacaacaagcaccgggataagcccatcagagagcaggccgagaatatcatccacctgtttaccctgaccaatctgggagcccctgccgccttcaagtactttgacaccaccatcgaccggaagaggtacaccagcaccaaagaggtgctggacgccaccctgatccaccagagcatcaccggcctgtacgagacacggatcgacctgtctcagctgggaggcgacaaaaggccggcggccacgaaaaaggccggccaggcaaaaaagaaaaaggaattcggcagtggagagggcagaggaagtctgctaacatgcggtgacgtcgaggagaatcctggcccagtgagcaagggcgaggagctgttcaccggggtggtgcccatcctggtcgagctggacggcgacgtaaacggccacaagttcagcgtgtccggcgagggcgagggcgatgccacctacggcaagctgaccctgaagttcatctgcaccaccggcaagctgcccgtgccctggcccaccctcgtgaccaccctgacctacggcgtgcagtgcttcagccgctaccccgaccacatgaagcagcacgacttcttcaagtccgccatgcccgaaggctacgtccaggagcgcaccatcttcttcaaggacgacggcaactacaagacccgcgccgaggtgaagttcgagggcgacaccctggtgaaccgcatcgagctgaagggcatcgacttcaaggaggacggcaacatcctggggcacaagctggagtacaactacaacagccacaacgtctatatcatggccgacaagcagaagaacggcatcaaggtgaacttcaagatccgccacaacatcgaggacggcagcgtgcagctcgccgaccactaccagcagaacacccccatcggcgacggccccgtgctgctgcccgacaaccactacctgagcacccagtccgccctgagcaaagaccccaacgagaagcgcgatcacatggtcctgctggagttcgtgaccgccgccgggatcactctcggcatggacgagctgtacaaggaattctaacgctagagggcccgtttaaacccgctgatcagcctcgactgtgccttctagttgccagccatctgttgtttgcccctcccccgtgccttccttgaccctggaaggtgccactcccactgtcctttcctaataaaatgaggaaattgcatcgcattgtctgagtaggtgtcattctattctggggggtggggtggggcaggacagcaagggggaggattgggaagacaatagcaggcatgctggggatgcggtgggctctatggcttctgaggcggaaagaaccagctggggctctagggggtatccccacgcgccctgtagcggcgcattaagcgcggcgggtgtggtggttacgcgcagcgtgaccgctacacttgccagcgccctagcgcccgctcctttcgctttcttcccttcctttctcgccacgttcgccggctttccccgtcaagctctaaatcgggggctccctttagggttccgatttagtgctttacggcacctcgaccccaaaaaacttgattagggtgatggttcacgtagtgggccatcgccctgatagacggtttttcgccctttgacgttggagtccacgttctttaatagtggactcttgttccaaactggaacaacactcaaccctatctcggtctattcttttgatttataagggattttgccgatttcggcctattggttaaaaaatgagctgatttaacaaaaatttaacgcgaattaattctgtggaatgtgtgtcagttagggtgtggaaagtccccaggctccccagcaggcagaagtatgcaaagcatgcatctcaattagtcagcaaccaggtgtggaaagtccccaggctccccagcaggcagaagtatgcaaagcatgcatctcaattagtcagcaaccatagtcccgcccctaactccgcccatcccgcccctaactccgcccagttccgcccattctccgccccatggctgactaattttttttatttatgcagaggccgaggccgcctctgcctctgagctattccagaagtagtgaggaggcttttttggaggcctaggcttttgcaaaaagctcccgggagcttgtatatccattttcggatctgatcaagagacaggatgaggatcgtttcgcatgattgaacaagatggattgcacgcaggttctccggccgcttgggtggagaggctattcggctatgactgggcacaacagacaatcggctgctctgatgccgccgtgttccggctgtcagcgcaggggcgcccggttctttttgtcaagaccgacctgtccggtgccctgaatgaactgcaggacgaggcagcgcggctatcgtggctggccacgacgggcgttccttgcgcagctgtgctcgacgttgtcactgaagcgggaagggactggctgctattgggcgaagtgccggggcaggatctcctgtcatctcaccttgctcctgccgagaaagtatccatcatggctgatgcaatgcggcggctgcatacgcttgatccggctacctgcccattcgaccaccaagcgaaacatcgcatcgagcgagcacgtactcggatggaagccggtcttgtcgatcaggatgatctggacgaagagcatcaggggctcgcgccagccgaactgttcgccaggctcaaggcgcgcatgcccgacggcgaggatctcgtcgtgacccatggcgatgcctgcttgccgaatatcatggtggaaaatggccgcttttctggattcatcgactgtggccggctgggtgtggcggaccgctatcaggacatagcgttggctacccgtgatattgctgaagagcttggcggcgaatgggctgaccgcttcctcgtgctttacggtatcgccgctcccgattcgcagcgcatcgccttctatcgccttcttgacgagttcttctgagcgggactctggggttcgaaatgaccgaccaagcgacgcccaacctgccatcacgagatttcgattccaccgccgccttctatgaaaggttgggcttcggaatcgttttccgggacgccggctggatgatcctccagcgcggggatctcatgctggagttcttcgcccaccccaacttgtttattgcagcttataatggttacaaataaagcaatagcatcacaaatttcacaaataaagcatttttttcactgcattctagttgtggtttgtccaaactcatcaatgtatcttatcatgtctgtataccgtcgacctctagctagagcttggcgtaatcatggtcatagctgtttcctgtgtgaaattgttatccgctcacaattccacacaacatacgagccggaagcataaagtgtaaagcctggggtgcctaatgagtgagctaactcacattaattgcgttgcgctcactgcccgctttccagtcgggaaacctgtcgtgccagctgcattaatgaatcggccaacgcgcggggagaggcggtttgcgtattgggcgctcttccgcttcctcgctcactgactcgctgcgctcggtcgttcggctgcggcgagcggtatcagctcactcaaaggcggtaatacggttatccacagaatcaggggataacgcaggaaagaacatgtgagcaaaaggccagcaaaaggccaggaaccgtaaaaaggccgcgttgctggcgtttttccataggctccgcccccctgacgagcatcacaaaaatcgacgctcaagtcagaggtggcgaaacccgacaggactataaagataccaggcgtttccccctggaagctccctcgtgcgctctcctgttccgaccctgccgcttaccggatacctgtccgcctttctcccttcgggaagcgtggcgctttctcatagctcacgctgtaggtatctcagttcggtgtaggtcgttcgctccaagctgggctgtgtgcacgaaccccccgttcagcccgaccgctgcgccttatccggtaactatcgtcttgagtccaacccggtaagacacgacttatcgccactggcagcagccactggtaacaggattagcagagcgaggtatgtaggcggtgctacagagttcttgaagtggtggcctaactacggctacactagaagaacagtatttggtatctgcgctctgctgaagccagttaccttcggaaaaagagttggtagctcttgatccggcaaacaaaccaccgctggtagcggtttttttgtttgcaagcagcagattacgcgcagaaaaaaaggatctcaagaagatcctttgatcttttctacggggtctgacgctcagtggaacgaaaactcacgttaagggattttggtcatgagattatcaaaaaggatcttcacctagatccttttaaattaaaaatgaagttttaaatcaatctaaagtatatatgagtaaacttggtctgacagttaccaatgcttaatcagtgaggcacctatctcagcgatctgtctatttcgttcatccatagttgcctgactccccgtcgtgtagataactacgatacgggagggcttaccatctggccccagtgctgcaatgataccgcgagacccacgctcaccggctccagatttatcagcaataaaccagccagccggaagggccgagcgcagaagtggtcctgcaactttatccgcctccatccagtctattaattgttgccgggaagctagagtaagtagttcgccagttaatagtttgcgcaacgttgttgccattgctacaggcatcgtggtgtcacgctcgtcgtttggtatggcttcattcagctccggttcccaacgatcaaggcgagttacatgatcccccatgttgtgcaaaaaagcggttagctccttcggtcctccgatcgttgtcagaagtaagttggccgcagtgttatcactcatggttatggcagcactgcataattctcttactgtcatgccatccgtaagatgcttttctgtgactggtgagtactcaaccaagtcattctgagaatagtgtatgcggcgaccgagttgctcttgcccggcgtcaatacgggataataccgcgccacatagcagaactttaaaagtgctcatcattggaaaacgttcttcggggcgaaaactctcaaggatcttaccgctgttgagatccagttcgatgtaacccactcgtgcacccaactgatcttcagcatcttttactttcaccagcgtttctgggtgagcaaaaacaggaaggcaaaatgccgcaaaaaagggaataagggcgacacggaaatgttgaatactcatactcttcctttttcaatattattgaagcatttatcagggttattgtctcatgagcggatacatatttgaatgtatttagaaaaataaacaaataggggttccgcgcacatttccccgaaaagtgccacctgacgtc

SEQ ID NO: 8 - DNA, 2508 bp, Artificial Sequence
  pMA-SV40pA vector V1.C.2
ctaaattgtaagcgttaatattttgttaaaattcgcgttaaatttttgttaaatcagctcattttttaaccaataggccgaaatcggcaaaatcccttataaatcaaaagaatagaccgagatagggttgagtggccgctacagggcgctcccattcgccattcaggctgcgcaactgttgggaagggcgtttcggtgcgggcctcttcgctattacgccagctggcgaaagggggatgtgctgcaaggcgattaagttgggtaacgccagggttttcccagtcacgacgttgtaaaacgacggccagtgagcgcgacgtaatacgactcactatagggcgaattggcggaaggccgtcaaggccgcatgaattgttgttgttaacttgtttattgcagcttataatggttacaaataaagcaatagcatcacaaatttcacaaataaagcatttttttcactgcattctagttgtggtttgtccaaactcatcaatgtatcttatcatgtctggatctgcggatccaatctcgagctgggcctcatgggccttccgctcactgcccgctttccagtcgggaaacctgtcgtgccagctgcattaacatggtcatagctgtttccttgcgtattgggcgctctccgcttcctcgctcactgactcgctgcgctcggtcgttcgggtaaagcctggggtgcctaatgagcaaaaggccagcaaaaggccaggaaccgtaaaaaggccgcgttgctggcgtttttccataggctccgcccccctgacgagcatcacaaaaatcgacgctcaagtcagaggtggcgaaacccgacaggactataaagataccaggcgtttccccctggaagctccctcgtgcgctctcctgttccgaccctgccgcttaccggatacctgtccgcctttctcccttcgggaagcgtggcgctttctcatagctcacgctgtaggtatctcagttcggtgtaggtcgttcgctccaagctgggctgtgtgcacgaaccccccgttcagcccgaccgctgcgccttatccggtaactatcgtcttgagtccaacccggtaagacacgacttatcgccactggcagcagccactggtaacaggattagcagagcgaggtatgtaggcggtgctacagagttcttgaagtggtggcctaactacggctacactagaagaacagtatttggtatctgcgctctgctgaagccagttaccttcggaaaaagagttggtagctcttgatccggcaaacaaaccaccgctggtagcggtggtttttttgtttgcaagcagcagattacgcgcagaaaaaaaggatctcaagaagatcctttgatcttttctacggggtctgacgctcagtggaacgaaaactcacgttaagggattttggtcatgagattatcaaaaaggatcttcacctagatccttttaaattaaaaatgaagttttaaatcaatctaaagtatatatgagtaaacttggtctgacagttaccaatgcttaatcagtgaggcacctatctcagcgatctgtctatttcgttcatccatagttgcctgactccccgtcgtgtagataactacgatacgggagggcttaccatctggccccagtgctgcaatgataccgcgagaaccacgctcaccggctccagatttatcagcaataaaccagccagccggaagggccgagcgcagaagtggtcctgcaactttatccgcctccatccagtctattaattgttgccgggaagctagagtaagtagttcgccagttaatagtttgcgcaacgttgttgccattgctacaggcatcgtggtgtcacgctcgtcgtttggtatggcttcattcagctccggttcccaacgatcaaggcgagttacatgatcccccatgttgtgcaaaaaagcggttagctccttcggtcctccgatcgttgtcagaagtaagttggccgcagtgttatcactcatggttatggcagcactgcataattctcttactgtcatgccatccgtaagatgcttttctgtgactggtgagtactcaaccaagtcattctgagaatagtgtatgcggcgaccgagttgctcttgcccggcgtcaatacgggataataccgcgccacatagcagaactttaaaagtgctcatcattggaaaacgttcttcggggcgaaaactctcaaggatcttaccgctgttgagatccagttcgatgtaacccactcgtgcacccaactgatcttcagcatcttttactttcaccagcgtttctgggtgagcaaaaacaggaaggcaaaatgccgcaaaaaagggaataagggcgacacggaaatgttgaatactcatactcttcctttttcaatattattgaagcatttatcagggttattgtctcatgagcggatacatatttgaatgtatttagaaaaataaacaaataggggttccgcgcacatttccccgaaaagtgccac

SEQ ID NO: 9 - DNA, 4341 bp, Artificial Sequence
  HLA-A 02:01 6xHis + Exon2/3-HA-L+R vector V1.C.6
ctaaattgtaagcgttaatattttgttaaaattcgcgttaaatttttgttaaatcagctcattttttaaccaataggccgaaatcggcaaaatcccttataaatcaaaagaatagaccgagatagggttgagtggccgctacagggcgctcccattcgccattcaggctgcgcaactgttgggaagggcgtttcggtgcgggcctcttcgctattacgccagctggcgaaagggggatgtgctgcaaggcgattaagttgggtaacgccagggttttcccagtcacgacgttgtaaaacgacggccagtgagcgcgacgtaatacgactcactatagggcgaattggcggaaggccgtcaaggccgcatgaattcgctaccggtatagtaatcaattacggggtcattagttcatagcccatatatggagttccgcgttacataacttacggtaaatggcccgcctggctgaccgcccaacgacccccgcccattgacgtcaataatgacgtatgttcccatagtaacgccaatagggactttccattgacgtcaatgggtggagtatttacggtaaactgcccacttggcagtacatcaagtgtatcatatgccaagtacgccccctattgacgtcaatgacggtaaatggcccgcctggcattatgcccagtacatgaccttatgggactttcctacttggcagtacatctacgtattagtcatcgctattaccatggtgatgcggttttggcagtacatcaatgggcgtggatagcggtttgactcacggggatttccaagtctccaccccattgacgtcaatgggagtttgttttggcaccaaaatcaacgggactttccaaaatgtcgtaacaactccgccccattgacgcaaatgggcggtaggcgtgtacggtgggaggtctatataagcagagctggtttagtgaaccgtcagatcaggtaccatggccgtcatggcgccccgaaccctcgtcctgctactctcgggggctctggccctgacccagacctgggcgggctctcactccatgaggtatttcttcacatccgtgtctcggccaggacgcggagagccacgcttcatcgcagtgggctacgtggacgacacgcagttcgtgcggttcgacagcgacgccgcgagccagaggatggagccgcgggcgccgtggatagagcaggagggtccggagtattgggacggggagacacggaaagtgaaggcccactcacagactcaccgagtggacctggggaccctgcgcggctactacaaccagagcgaggccggttctcacaccgtccagaggatgtatggctgcgacgtggggtcggactggcgcttcctccgcggataccaccagtacgcctacgacggcaaggattacatcgccctgaaagaggacctgcgctcttggaccgcggcggacatggcagctcagaccaccaagcacaagtgggaggcggcccatgtggcggagcagttgagagcctacctggagggcacgtgcgtggagtggctccgcagatacctggagaacgggaaggagacgctgcagcgcacggacgcccccaaaacgcatatgactcaccacgctgtctctgaccatgaagccaccctgaggtgctgggccctgagcttctaccctgcggagatcacactgacctggcagcgggatggggaggaccagacccaggacacggagctcgtggagaccaggcctgcaggggatggaaccttccagaagtgggcggctgtggtggtgccttctggacaggagcagagatacacctgccatgtgcagcatgagggtttgcccaagcccctcaccctgagatgggagccgtcttcccagcccaccatccccatcgtgggcatcattgctggcctggttctctttggagctgtgatcactggagctgtggtcgctgctgtgatgtggaggaggaagagctcagatagaaaaggagggagctactctcaggctgcaagcagtgacagtgcccagggctctgatgtgtctctcacagcttgtaaagtgcccgggcatcatcaccatcaccactgactatagtcgtctagacctgatcataatcaagccatatcacatctgtagaggtttacttgctttaaaaaacctccacacctccccctgaacctgaaacataaaatgaatgcaattgttgttgttaacttgtttattgcagcttataatggttacaaataaagcaatagcatcacaaatttcacaaataaagcatttttttcactgcattctagttgtggtttgtccaaactcatcaatgtatcttatcatgtctggatctgcggatccaatctcgagctgggcctcatgggccttccgctcactgcccgctttccagtcgggaaacctgtcgtgccagctgcattaacatggtcatagctgtttccttgcgtattgggcgctctccgcttcctcgctcactgactcgctgcgctcggtcgttcgggtaaagcctggggtgcctaatgagcaaaaggccagcaaaaggccaggaaccgtaaaaaggccgcgttgctggcgtttttccataggctccgcccccctgacgagcatcacaaaaatcgacgctcaagtcagaggtggcgaaacccgacaggactataaagataccaggcgtttccccctggaagctccctcgtgcgctctcctgttccgaccctgccgcttaccggatacctgtccgcctttctcccttcgggaagcgtggcgctttctcatagctcacgctgtaggtatctcagttcggtgtaggtcgttcgctccaagctgggctgtgtgcacgaaccccccgttcagcccgaccgctgcgccttatccggtaactatcgtcttgagtccaacccggtaagacacgacttatcgccactggcagcagccactggtaacaggattagcagagcgaggtatgtaggcggtgctacagagttcttgaagtggtggcctaactacggctacactagaagaacagtatttggtatctgcgctctgctgaagccagttaccttcggaaaaagagttggtagctcttgatccggcaaacaaaccaccgctggtagcggtggtttttttgtttgcaagcagcagattacgcgcagaaaaaaaggatctcaagaagatcctttgatcttttctacggggtctgacgctcagtggaacgaaaactcacgttaagggattttggtcatgagattatcaaaaaggatcttcacctagatccttttaaattaaaaatgaagttttaaatcaatctaaagtatatatgagtaaacttggtctgacagttaccaatgcttaatcagtgaggcacctatctcagcgatctgtctatttcgttcatccatagttgcctgactccccgtcgtgtagataactacgatacgggagggcttaccatctggccccagtgctgcaatgataccgcgagaaccacgctcaccggctccagatttatcagcaataaaccagccagccggaagggccgagcgcagaagtggtcctgcaactttatccgcctccatccagtctattaattgttgccgggaagctagagtaagtagttcgccagttaatagtttgcgcaacgttgttgccattgctacaggcatcgtggtgtcacgctcgtcgtttggtatggcttcattcagctccggttcccaacgatcaaggcgagttacatgatcccccatgttgtgcaaaaaagcggttagctccttcggtcctccgatcgttgtcagaagtaagttggccgcagtgttatcactcatggttatggcagcactgcataattctcttactgtcatgccatccgtaagatgcttttctgtgactggtgagtactcaaccaagtcattctgagaatagtgtatgcggcgaccgagttgctcttgcccggcgtcaatacgggataataccgcgccacatagcagaactttaaaagtgctcatcattggaaaacgttcttcggggcgaaaactctcaaggatcttaccgctgttgagatccagttcgatgtaacccactcgtgcacccaactgatcttcagcatcttttactttcaccagcgtttctgggtgagcaaaaacaggaaggcaaaatgccgcaaaaaagggaataagggcgacacggaaatgttgaatactcatactcttcctttttcaatattattgaagcatttatcagggttattgtctcatgagcggatacatatttgaatgtatttagaaaaataaacaaataggggttccgcgcacatttccccgaaaagtgccac

SEQ ID NO: 10 - DNA, 4332 bp, Artificial Sequence
  HLA-B 35:01 6xHis + Exon2/3-HA-L+R vector V1.C.9
ctaaattgtaagcgttaatattttgttaaaattcgcgttaaatttttgttaaatcagctcattttttaaccaataggccgaaatcggcaaaatcccttataaatcaaaagaatagaccgagatagggttgagtggccgctacagggcgctcccattcgccattcaggctgcgcaactgttgggaagggcgtttcggtgcgggcctcttcgctattacgccagctggcgaaagggggatgtgctgcaaggcgattaagttgggtaacgccagggttttcccagtcacgacgttgtaaaacgacggccagtgagcgcgacgtaatacgactcactatagggcgaattggcggaaggccgtcaaggccgcatgaattcgctaccggtatagtaatcaattacggggtcattagttcatagcccatatatggagttccgcgttacataacttacggtaaatggcccgcctggctgaccgcccaacgacccccgcccattgacgtcaataatgacgtatgttcccatagtaacgccaatagggactttccattgacgtcaatgggtggagtatttacggtaaactgcccacttggcagtacatcaagtgtatcatatgccaagtacgccccctattgacgtcaatgacggtaaatggcccgcctggcattatgcccagtacatgaccttatgggactttcctacttggcagtacatctacgtattagtcatcgctattaccatggtgatgcggttttggcagtacatcaatgggcgtggatagcggtttgactcacggggatttccaagtctccaccccattgacgtcaatgggagtttgttttggcaccaaaatcaacgggactttccaaaatgtcgtaacaactccgccccattgacgcaaatgggcggtaggcgtgtacggtgggaggtctatataagcagagctggtttagtgaaccgtcagatcaggtaccatgcgggtcacggcgccccgaaccgtcctcctgctgctctggggggcagtggccctgaccgagacctgggccggctcccactccatgaggtatttctacaccgccatgtcccggccaggacgcggagagccacgcttcatcgcagtgggctacgtggacgacacccagttcgtgaggttcgacagcgacgccgcgagtccgaggacggagcctcgggcgccatggatagagcaggaggggccggagtattgggaccggaacacacagatcttcaagaccaacacacagacttaccgagagagcctgcggaacctgcgcggctactacaaccagagcgaggccgggtctcacatcatccagaggatgtatggctgcgacctggggcccgacgggcgcctcctccgcgggcatgaccagtccgcctacgacggcaaggattacatcgccctgaacgaggacctgagctcctggaccgcggcggacaccgcggctcagatcacccagcgcaagtgggaggcggcccgtgtggcggagcagctgagagcctacctggagggcctgtgcgtggagtggctccgcagatacctggagaacgggaaggagactcttcagcgcgcagatcctccaaagacacacgtgacccaccaccccgtctctgaccatgaggccaccctgaggtgctgggccctgggcttctaccctgcggagatcacactgacctggcagcgggatggcgaggaccaaactcaggacactgagcttgtggagaccagaccagcaggagatagaaccttccagaagtgggcagctgtggtggtgccttctggagaagagcagagatacacatgccatgtacagcatgaggggctgccgaagcccctcaccctgagatgggagccatcttcccagtccaccatccccatcgtgggcattgttgctggcctggctgtcctagcagttgtggtcatcggagctgtggtcgctactgtgatgtgtaggaggaagagctcaggtggaaaaggagggagctactctcaggctgcgtccagcgacagtgcccagggctctgatgtgtctctcacagctcccgggcatcatcaccatcaccactgactatagtcgtctagacctgatcataatcaagccatatcacatctgtagaggtttacttgctttaaaaaacctccacacctccccctgaacctgaaacataaaatgaatgcaattgttgttgttaacttgtttattgcagcttataatggttacaaataaagcaatagcatcacaaatttcacaaataaagcatttttttcactgcattctagttgtggtttgtccaaactcatcaatgtatcttatcatgtctggatctgcggatccaatctcgagctgggcctcatgggccttccgctcactgcccgctttccagtcgggaaacctgtcgtgccagctgcattaacatggtcatagctgtttccttgcgtattgggcgctctccgcttcctcgctcactgactcgctgcgctcggtcgttcgggtaaagcctggggtgcctaatgagcaaaaggccagcaaaaggccaggaaccgtaaaaaggccgcgttgctggcgtttttccataggctccgcccccctgacgagcatcacaaaaatcgacgctcaagtcagaggtggcgaaacccgacaggactataaagataccaggcgtttccccctggaagctccctcgtgcgctctcctgttccgaccctgccgcttaccggatacctgtccgcctttctcccttcgggaagcgtggcgctttctcatagctcacgctgtaggtatctcagttcggtgtaggtcgttcgctccaagctgggctgtgtgcacgaaccccccgttcagcccgaccgctgcgccttatccggtaactatcgtcttgagtccaacccggtaagacacgacttatcgccactggcagcagccactggtaacaggattagcagagcgaggtatgtaggcggtgctacagagttcttgaagtggtggcctaactacggctacactagaagaacagtatttggtatctgcgctctgctgaagccagttaccttcggaaaaagagttggtagctcttgatccggcaaacaaaccaccgctggtagcggtggtttttttgtttgcaagcagcagattacgcgcagaaaaaaaggatctcaagaagatcctttgatcttttctacggggtctgacgctcagtggaacgaaaactcacgttaagggattttggtcatgagattatcaaaaaggatcttcacctagatccttttaaattaaaaatgaagttttaaatcaatctaaagtatatatgagtaaacttggtctgacagttaccaatgcttaatcagtgaggcacctatctcagcgatctgtctatttcgttcatccatagttgcctgactccccgtcgtgtagataactacgatacgggagggcttaccatctggccccagtgctgcaatgataccgcgagaaccacgctcaccggctccagatttatcagcaataaaccagccagccggaagggccgagcgcagaagtggtcctgcaactttatccgcctccatccagtctattaattgttgccgggaagctagagtaagtagttcgccagttaatagtttgcgcaacgttgttgccattgctacaggcatcgtggtgtcacgctcgtcgtttggtatggcttcattcagctccggttcccaacgatcaaggcgagttacatgatcccccatgttgtgcaaaaaagcggttagctccttcggtcctccgatcgttgtcagaagtaagttggccgcagtgttatcactcatggttatggcagcactgcataattctcttactgtcatgccatccgtaagatgcttttctgtgactggtgagtactcaaccaagtcattctgagaatagtgtatgcggcgaccgagttgctcttgcccggcgtcaatacgggataataccgcgccacatagcagaactttaaaagtgctcatcattggaaaacgttcttcggggcgaaaactctcaaggatcttaccgctgttgagatccagttcgatgtaacccactcgtgcacccaactgatcttcagcatcttttactttcaccagcgtttctgggtgagcaaaaacaggaaggcaaaatgccgcaaaaaagggaataagggcgacacggaaatgttgaatactcatactcttcctttttcaatattattgaagcatttatcagggttattgtctcatgagcggatacatatttgaatgtatttagaaaaataaacaaataggggttccgcgcacatttccccgaaaagtgccac

SEQ ID NO: 11 - DNA, 5520 bp, Artificial Sequence
  AAVS1-S_A24_6xH vector V1.F.8
ctaaattgtaagcgttaatattttgttaaaattcgcgttaaatttttgttaaatcagctcattttttaaccaataggccgaaatcggcaaaatcccttataaatcaaaagaatagaccgagatagggttgagtggccgctacagggcgctcccattcgccattcaggctgcgcaactgttgggaagggcgtttcggtgcgggcctcttcgctattacgccagctggcgaaagggggatgtgctgcaaggcgattaagttgggtaacgccagggttttcccagtcacgacgttgtaaaacgacggccagtgagcgcgacgtaatacgactcactatagggcgaattggcggaaggccgtcaaggccgcatgaattgctgcccaaggatgctctttccggagcacttccttctcggcgctgcaccacgtgatgtcctctgagcggatcctccccgtgtctgggtcctctccgggcatctctcctccctcacccaaccccatgccgtgttcactcgctgggttcccttttccttctccttctggggcctgtgccatctctcgtttcttaggatggccttctccgacggatgtctcccttgcgtcccgcctccccttcttgtaggcctgcatcatcaccgtttttctggacaaccccaaagtaccccgtctccctggcttagcacctctccatcctcttgctttctttgcctggacaccccgttctcctgtggattcgggtcacctctcactcctttcatttgggcagctcccctaccccccttacctctctagtctgtgctagctcttccagccccctgtcatggcatcttccaggggtccgagagctcagctagtcttcttcctccaacccgggccctatgtccacttcaggacagcatgtttgctgcctccagggatcctgtgtccccgagctgggaccaccttatattcccagggccggttaatgtggctctggttctgggtacttttatctgtcccctccaccggtatagtaatcaattacggggtcattagttcatagcccatatatggagttccgcgttacataacttacggtaaatggcccgcctggctgaccgcccaacgacccccgcccattgacgtcaataatgacgtatgttcccatagtaacgccaatagggactttccattgacgtcaatgggtggagtatttacggtaaactgcccacttggcagtacatcaagtgtatcatatgccaagtacgccccctattgacgtcaatgacggtaaatggcccgcctggcattatgcccagtacatgaccttatgggactttcctacttggcagtacatctacgtattagtcatcgctattaccatggtgatgcggttttggcagtacatcaatgggcgtggatagcggtttgactcacggggatttccaagtctccaccccattgacgtcaatgggagtttgttttggcaccaaaatcaacgggactttccaaaatgtcgtaacaactccgccccattgacgcaaatgggcggtaggcgtgtacggtgggaggtctatataagcagagctggtttagtgaaccgtcagatcaggtaccatggccgtcatggcgccccgaaccctcgtcctgctactctcgggggccctggccctgacccagacctgggcaggctcccactccatgaggtatttctccacatccgtgtctcggccaggacgcggagagccacgcttcatcgccgtgggctacgtggacgacacgcagttcgtgcggttcgacagcgacgccgcgagccagaggatggagccgcgggcgccgtggatagagcaggaggggccggagtattgggacgaggagacagggaaagtgaaggcccactcacagactgaccgagagaacctgcggatcgcgctccgctactacaaccagagcgaggccggttctcacaccctccagatgatgtttggctgcgacgtggggtcggacgggcgcttcctccgcggataccaccagtacgcctacgacggcaaggattacatcgccctgaaagaggacctgcgctcttggaccgcggcggacatggcggctcagatcaccaagcgcaagtgggaggcggcccatgtggcggagcagcagagagcctacctggagggcacgtgcgtggacgggctccgcagatacctggagaacgggaaggagacgctgcagcgcacggacccccccaagacacatatgacccaccaccccatctctgaccatgaggccactctgagatgctgggccctgggcttctaccctgcggagatcacactgacctggcagcgggatggggaggaccagacccaggacacggagcttgtggagaccaggcctgcaggggatggaaccttccagaagtgggcagctgtggtggttccttctggagaggagcagagatacacctgccatgtgcagcatgagggtctgcccaagcccctcaccctgagatgggagccatcttcccagcccaccgtccccatcgtgggcatcattgctggcctggttctccttggagctgtgatcactggagctgtggtcgctgctgtgatgtggaggaggaacagctcagatagaaaaggagggagctactctcaggctgcaagcagtgacagtgcccagggctctgatgtgtctctcacagcttgtaaagtgcccgggcatcatcaccatcaccactgactatagtcgtctagacctgatcataatcaagccatatcacatctgtagaggtttacttgctttaaaaaacctccacacctccccctgaacctgaaacataaaatgaatgcaattgttgttgttaacttgtttattgcagcttataatggttacaaataaagcaatagcatcacaaatttcacaaataaagcatttttttcactgcattctagttgtggtttgtccaaactcatcaatgtatcttatcatgtctggatctgcggatcaggattggtgacagaaaagcccccatccttaggcctcctccttcctagtctcctgatattcgtctaacccccacctcctgttaggcagattccttatctggtgacacacccccatttcctggagccatctctctccttgccagaacctctaaggtttgcttacgatggagccagagaggatcctgggagggagacttggcagggggtgggagggaagggggggatgcgtgacctgcccggttctcagtggccaccctgcgctaccctctcccagaacctgagctgctctgacgcggctgtctggtgcgtttcactgatcctggtgctgcagcttccttacacttcccaagaggagaagcagtttggaaaaacaaaatcagaataagttggtcctgagttctaactttggctcttcacctttctagcccccaatttatattgttcctccgtgcgtcagttttacctgtgagataaggccagtagccacccccgtcctggcagggctgtggtgaggaggggggtgtccgtgtggaaaactccctttgtgagaatggtgcgtcctcgagctgggcctcatgggccttccgctcactgcccgctttccagtcgggaaacctgtcgtgccagctgcattaacatggtcatagctgtttccttgcgtattgggcgctctccgcttcctcgctcactgactcgctgcgctcggtcgttcgggtaaagcctggggtgcctaatgagcaaaaggccagcaaaaggccaggaaccgtaaaaaggccgcgttgctggcgtttttccataggctccgcccccctgacgagcatcacaaaaatcgacgctcaagtcagaggtggcgaaacccgacaggactataaagataccaggcgtttccccctggaagctccctcgtgcgctctcctgttccgaccctgccgcttaccggatacctgtccgcctttctcccttcgggaagcgtggcgctttctcatagctcacgctgtaggtatctcagttcggtgtaggtcgttcgctccaagctgggctgtgtgcacgaaccccccgttcagcccgaccgctgcgccttatccggtaactatcgtcttgagtccaacccggtaagacacgacttatcgccactggcagcagccactggtaacaggattagcagagcgaggtatgtaggcggtgctacagagttcttgaagtggtggcctaactacggctacactagaagaacagtatttggtatctgcgctctgctgaagccagttaccttcggaaaaagagttggtagctcttgatccggcaaacaaaccaccgctggtagcggtggtttttttgtttgcaagcagcagattacgcgcagaaaaaaaggatctcaagaagatcctttgatcttttctacggggtctgacgctcagtggaacgaaaactcacgttaagggattttggtcatgagattatcaaaaaggatcttcacctagatccttttaaattaaaaatgaagttttaaatcaatctaaagtatatatgagtaaacttggtctgacagttaccaatgcttaatcagtgaggcacctatctcagcgatctgtctatttcgttcatccatagttgcctgactccccgtcgtgtagataactacgatacgggagggcttaccatctggccccagtgctgcaatgataccgcgagaaccacgctcaccggctccagatttatcagcaataaaccagccagccggaagggccgagcgcagaagtggtcctgcaactttatccgcctccatccagtctattaattgttgccgggaagctagagtaagtagttcgccagttaatagtttgcgcaacgttgttgccattgctacaggcatcgtggtgtcacgctcgtcgtttggtatggcttcattcagctccggttcccaacgatcaaggcgagttacatgatcccccatgttgtgcaaaaaagcggttagctccttcggtcctccgatcgttgtcagaagtaagttggccgcagtgttatcactcatggttatggcagcactgcataattctcttactgtcatgccatccgtaagatgcttttctgtgactggtgagtactcaaccaagtcattctgagaatagtgtatgcggcgaccgagttgctcttgcccggcgtcaatacgggataataccgcgccacatagcagaactttaaaagtgctcatcattggaaaacgttcttcggggcgaaaactctcaaggatcttaccgctgttgagatccagttcgatgtaacccactcgtgcacccaactgatcttcagcatcttttactttcaccagcgtttctgggtgagcaaaaacaggaaggcaaaatgccgcaaaaaagggaataagggcgacacggaaatgttgaatactcatactcttcctttttcaatattattgaagcatttatcagggttattgtctcatgagcggatacatatttgaatgtatttagaaaaataaacaaataggggttccgcgcacatttccccgaaaagtgccac

SEQ ID NO: 12 - DNA, 5733 bp, Artificial Sequence
  AAVS1-L_B07_6xH vector V1.F.10
ctaaattgtaagcgttaatattttgttaaaattcgcgttaaatttttgttaaatcagctcattttttaaccaataggccgaaatcggcaaaatcccttataaatcaaaagaatagaccgagatagggttgagtggccgctacagggcgctcccattcgccattcaggctgcgcaactgttgggaagggcgtttcggtgcgggcctcttcgctattacgccagctggcgaaagggggatgtgctgcaaggcgattaagttgggtaacgccagggttttcccagtcacgacgttgtaaaacgacggccagtgagcgcgacgtaatacgactcactatagggcgaattggcggaaggccgtcaaggccgcatgaattgagctctactggcttctgcgccgcctctggcccactgtttccccttcccaggcaggtcctgctttctctgacctgcattctctcccctgggcctgtgccgctttctgtctgcagcttgtggcctgggtcacctctacggctggcccagatccttccctgccgcctccttcaggttccgtcttcctccactccctcttccccttgctctctgctgtgttgctgcccaaggatgctctttccggagcacttccttctcggcgctgcaccacgtgatgtcctctgagcggatcctccccgtgtctgggtcctctccgggcatctctcctccctcacccaaccccatgccgtcttcactcgctgggttcccttttccttctccttctggggcctgtgccatctctcgtttcttaggatggccttctccgacggatgtctcccttgcgtcccgcctccccttcttgtaggcctgcatcatcaccgtttttctggacaaccccaaagtaccccgtctccctggctttagccacctctccatcctcttgctttctttgcctggacaccccgttctcctgtggattcgggtcacctctcactcctttcatttgggcagctcccctaccccccttacctctctagtctgtgctagctcttccagccccctgtcatggcatcttccaggggtccgagagctcagctagtcttcttcctccaacccgggcccctatgtccacttcaggacagcatgtttgctgcctccagggatcctgtgtccccgagctgggaccaccttatattcccagggccggttaatgtggctctggttctgggtacttttatctgtcccctccaccggtatagtaatcaattacggggtcattagttcatagcccatatatggagttccgcgttacataacttacggtaaatggcccgcctggctgaccgcccaacgacccccgcccattgacgtcaataatgacgtatgttcccatagtaacgccaatagggactttccattgacgtcaatgggtggagtatttacggtaaactgcccacttggcagtacatcaagtgtatcatatgccaagtacgccccctattgacgtcaatgacggtaaatggcccgcctggcattatgcccagtacatgaccttatgggactttcctacttggcagtacatctacgtattagtcatcgctattaccatggtgatgcggttttggcagtacatcaatgggcgtggatagcggtttgactcacggggatttccaagtctccaccccattgacgtcaatgggagtttgttttggcaccaaaatcaacgggactttccaaaatgtcgtaacaactccgccccattgacgcaaatgggcggtaggcgtgtacggtgggaggtctatataagcagagctggtttagtgaaccgtcagatcaggtaccatgctggtcatggcgccccgaaccgtcctcctgctgctctcggcggccctggccctgaccgagacctgggccggctcccactccatgaggtatttctacacctccgtgtctcggccaggacgcggagagccacgcttcatctcagtgggctacgtggacgacacccagttcgtgaggttcgacagcgacgccgcgagtccgagagaggagccgcgggcgccgtggatagagcaggaggggccggagtattgggaccggaacacacagatctacaaggcccaggcacagactgaccgagagagcctgcggaacctgcgcggctactacaaccagagcgaggccgggtctcacaccctccagagcatgtacggctgcgacgtggggccggacgggcgcctcctccgcgggcatgaccagtacgcctacgacggcaaggattacatcgccctgaacgaggacctgcgctcctggaccgccgcggacacggcggctcagatcacccagcgcaagtgggaggcggcccgtgaggcggagcagcggagagcctacctggagggcgagtgcgtggagtggctccgcagatacctggagaacgggaaggacaaacttgagcgcgcagaccctccaaagacacacgtgacccaccaccccatctctgaccatgaggccaccctgaggtgctgggccctgggtttctaccctgcggagatcacactgacctggcagcgggatggcgaggaccaaactcaggacactgagcttgtggagaccagaccagcaggagatagaaccttccagaagtgggcagctgtggtggtgccttctggagaagagcagagatacacatgccatgtacagcatgaggggctgccgaagcccctcaccctgagatgggagccgtcttcccagtccaccgtccccatcgtgggcattgttgctggcctggctgtcctagcagttgtggtcatcggagctgtggtcgctgctgtgatgtgtaggaggaagagttcaggtggaaaaggagggagctactctcaggctgcgtgcagcgacagtgcccagggctctgatgtgtctctcacagctcccgggcatcatcaccatcaccactgactatagtcgtctagacctgatcataatcaagccatatcacatctgtagaggtttacttgctttaaaaaacctccacacctccccctgaacctgaaacataaaatgaatgcaattgttgttgttaacttgtttattgcagcttataatggttacaaataaagcaatagcatcacaaatttcacaaataaagcatttttttcactgcattctagttgtggtttgtccaaactcatcaatgtatcttatcatgtctggatctgcggatcaggattggtgacagaaaagccccatccttaggcctcctccttcctagtctcctgatattgggtctaacccccacctcctgttaggcagattccttatctggtgacacacccccatttcctggagccatctctctccttgccagaacctctaaggtttgcttacgatggagccagagaggatcctgggagggagagcttggcagggggtgggagggaagggggggatgcgtgacctgcccggttctcagtggccaccctgcgctaccctctcccagaacctgagctgctctgacgcggctgtctggtgcgtttcactgatcctggtgctgcagcttccttacacttcccaagaggagaagcagtttggaaaaacaaaatcagaataagttggtcctgagttctaactttggctcttcacctttctagtccccaatttatattgttcctccgtgcgtcagttttacctgtgagataaggccagtagccagccccgtcctggcagggctgtggtgaggaggggggtgtccgtgtggaaaactccctttgtgagaatggtgcgtcctcgagctgggcctcatgggccttccgctcactgcccgctttccagtcgggaaacctgtcgtgccagctgcattaacatggtcatagctgtttccttgcgtattgggcgctctccgcttcctcgctcactgactcgctgcgctcggtcgttcgggtaaagcctggggtgcctaatgagcaaaaggccagcaaaaggccaggaaccgtaaaaaggccgcgttgctggcgtttttccataggctccgcccccctgacgagcatcacaaaaatcgacgctcaagtcagaggtggcgaaacccgacaggactataaagataccaggcgtttccccctggaagctccctcgtgcgctctcctgttccgaccctgccgcttaccggatacctgtccgcctttctcccttcgggaagcgtggcgctttctcatagctcacgctgtaggtatctcagttcggtgtaggtcgttcgctccaagctgggctgtgtgcacgaaccccccgttcagcccgaccgctgcgccttatccggtaactatcgtcttgagtccaacccggtaagacacgacttatcgccactggcagcagccactggtaacaggattagcagagcgaggtatgtaggcggtgctacagagttcttgaagtggtggcctaactacggctacactagaagaacagtatttggtatctgcgctctgctgaagccagttaccttcggaaaaagagttggtagctcttgatccggcaaacaaaccaccgctggtagcggtggtttttttgtttgcaagcagcagattacgcgcagaaaaaaaggatctcaagaagatcctttgatcttttctacggggtctgacgctcagtggaacgaaaactcacgttaagggattttggtcatgagattatcaaaaaggatcttcacctagatccttttaaattaaaaatgaagttttaaatcaatctaaagtatatatgagtaaacttggtctgacagttaccaatgcttaatcagtgaggcacctatctcagcgatctgtctatttcgttcatccatagttgcctgactccccgtcgtgtagataactacgatacgggagggcttaccatctggccccagtgctgcaatgataccgcgagaaccacgctcaccggctccagatttatcagcaataaaccagccagccggaagggccgagcgcagaagtggtcctgcaactttatccgcctccatccagtctattaattgttgccgggaagctagagtaagtagttcgccagttaatagtttgcgcaacgttgttgccattgctacaggcatcgtggtgtcacgctcgtcgtttggtatggcttcattcagctccggttcccaacgatcaaggcgagttacatgatcccccatgttgtgcaaaaaagcggttagctccttcggtcctccgatcgttgtcagaagtaagttggccgcagtgttatcactcatggttatggcagcactgcataattctcttactgtcatgccatccgtaagatgcttttctgtgactggtgagtactcaaccaagtcattctgagaatagtgtatgcggcgaccgagttgctcttgcccggcgtcaatacgggataataccgcgccacatagcagaactttaaaagtgctcatcattggaaaacgttcttcggggcgaaaactctcaaggatcttaccgctgttgagatccagttcgatgtaacccactcgtgcacccaactgatcttcagcatcttttactttcaccagcgtttctgggtgagcaaaaacaggaaggcaaaatgccgcaaaaaagggaataagggcgacacggaaatgttgaatactcatactcttcctttttcaatattattgaagcatttatcagggttattgtctcatgagcggatacatatttgaatgtatttagaaaaataaacaaataggggttccgcgcacatttccccgaaaagtgccac

SEQ ID NO: 13 - DNA, 7062 bp, Artificial Sequence
  AAVS1-l_GFP_HCMVpp65_WT vector V1.G.10
ctaaattgtaagcgttaatattttgttaaaattcgcgttaaatttttgttaaatcagctcattttttaaccaataggccgaaatcggcaaaatcccttataaatcaaaagaatagaccgagatagggttgagtggccgctacagggcgctcccattcgccattcaggctgcgcaactgttgggaagggcgtttcggtgcgggcctcttcgctattacgccagctggcgaaagggggatgtgctgcaaggcgattaagttgggtaacgccagggttttcccagtcacgacgttgtaaaacgacggccagtgagcgcgacgtaatacgactcactatagggcgaattggcggaaggccgtcaaggccgcatgaattgagctctactggcttctgcgccgcctctggcccactgtttccccttcccaggcaggtcctgctttctctgacctgcattctctcccctgggcctgtgccgctttctgtctgcagcttgtggcctgggtcacctctacggctggcccagatccttccctgccgcctccttcaggttccgtcttcctccactccctcttccccttgctctctgctgtgttgctgcccaaggatgctctttccggagcacttccttctcggcgctgcaccacgtgatgtcctctgagcggatcctccccgtgtctgggtcctctccgggcatctctcctccctcacccaaccccatgccgtcttcactcgctgggttcccttttccttctccttctggggcctgtgccatctctcgtttcttaggatggccttctccgacggatgtctcccttgcgtcccgcctccccttcttgtaggcctgcatcatcaccgtttttctggacaaccccaaagtaccccgtctccctggctttagccacctctccatcctcttgctttctttgcctggacaccccgttctcctgtggattcgggtcacctctcactcctttcatttgggcagctcccctaccccccttacctctctagtctgtgctagctcttccagccccctgtcatggcatcttccaggggtccgagagctcagctagtcttcttcctccaacccgggcccctatgtccacttcaggacagcatgtttgctgcctccagggatcctgtgtccccgagctgggaccaccttatattcccagggccggttaatgtggctctggttctgggtacttttatctgtcccctccaccggtatagtaatcaattacggggtcattagttcatagcccatatatggagttccgcgttacataacttacggtaaatggcccgcctggctgaccgcccaacgacccccgcccattgacgtcaataatgacgtatgttcccatagtaacgccaatagggactttccattgacgtcaatgggtggagtatttacggtaaactgcccacttggcagtacatcaagtgtatcatatgccaagtacgccccctattgacgtcaatgacggtaaatggcccgcctggcattatgcccagtacatgaccttatgggactttcctacttggcagtacatctacgtattagtcatcgctattaccatggtgatgcggttttggcagtacatcaatgggcgtggatagcggtttgactcacggggatttccaagtctccaccccattgacgtcaatgggagtttgttttggcaccaaaatcaacgggactttccaaaatgtcgtaacaactccgccccattgacgcaaatgggcggtaggcgtgtacggtgggaggtctatataagcagagctggtttagtgaaccgtcagatcaggtaccgccaccatggaatccgatgagtctggcctgcccgccatggaaatcgagtgcagaatcaccggcaccctgaacggcgtggaatttgagctcgtgggcggaggcgagggcacacctgaacagggcagaatgaccaacaagatgaagtccaccaagggggccctgaccttcagcccctacctgctgtctcacgtgatgggctacggcttctaccacttcggcacctaccccagcggctacgagaaccctttcctgcacgccatcaacaacggcggctacaccaacacccggatcgagaagtacgaggacggcggcgtgctgcacgtgtccttcagctacagatacgaggccggcagagtgatcggcgacttcaaagtgatgggcaccggattccccgaggacagcgtgatcttcaccgacaagatcatccggtccaacgccaccgtggaacatctgcaccccatgggcgacaacgacctggacggcagcttcaccagaaccttctccctgcgggatggcggctactacagcagcgtggtggacagccacatgcacttcaagagcgccatccaccccagcatcctccagaacggcggacccatgttcgccttcagacgggtggaagaggaccacagcaacaccgagctgggcatcgtggaataccagcacgccttcaagacccccgatgccgatgccggcgaggaaggcagtggagagggcagaggaagtctgctaacatgtggtgacgtcgaggagaatcctggcccaatggagtcgcgcggtcgccgttgtcccgaaatgatatccgtactgggtcccatttcggggcacgtgctgaaagccgtgtttagtcgcggcgatacgccggtgctgccgcacgagacgcgactcctgcagacgggtatccacgtacgcgtgagccagccctcgctgatcttggtatcgcagtacacgcccgactcgacgccatgccaccgcggcgacaatcagctgcaggtgcagcacacgtactttacgggcagcgaggtggagaacgtgtcggtcaacgtgcacaaccccacgggccgaagcatctgccccagccaggagcccatgtcgatctatgtgtacgcgctgccgctcaagatgctgaacatccccagcatcaacgtgcaccactacccgtcggcggccgagcgcaaacaccgacacctgcccgtagctgacgctgtgattcacgcgtcgggcaagcagatgtggcaggcgcgtctcacggtctcgggactggcctggacgcgtcagcagaaccagtggaaagagcccgacgtctactacacgtcagcgttcgtgtttcccaccaaggacgtggcactgcggcacgtggtgtgcgcgcacgagctggtttgctccatggagaacacgcgcgcaaccaagatgcaggtgataggtgaccagtacgtcaaggtgtacctggagtccttctgcgaggacgtgccctccggcaagctctttatgcacgtcacgctgggctctgacgtggaagaggacctgacgatgacccgcaacccgcaacccttcatgcgcccccacgagcgcaacggctttacggtgttgtgtcccaaaaatatgataatcaaaccgggcaagatctcgcacatcatgctggatgtggcttttacctcacacgagcattttgggctgctgtgtcccaagagcatcccgggcctgagcatctcaggtaacctgttgatgaacgggcagcagatcttcctggaggtacaagccatacgcgagaccgtggaactgcgtcagtacgatcccgtggctgcgctcttctttttcgatatcgacttgctgctgcagcgcgggcctcagtacagcgagcaccccaccttcaccagccagtatcgcatccagggcaagcttgagtaccgacacacctgggaccggcacgacgagggtgccgcccagggcgacgacgacgtctggaccagcggatcggactccgacgaagaactcgtaaccaccgagcgcaagacgccccgcgtcaccggcggcggcgccatggcgggcgcctccacttccgcgggccgcaaacgcaaatcagcatcctcggcgacggcgtgcacgtcgggcgttatgacacgcggccgccttaaggccgagtccaccgtcgcgcccgaagaggacaccgacgaggattccgacaacgaaatccacaatccggccgtgttcacctggccgccctggcaggccggcatcctggcccgcaacctggtgcccatggtggctacggttcagggtcagaatctgaagtaccaggagttcttctgggacgccaacgacatctaccgcatcttcgccgaattggaaggcgtatggcagcccgctgcgcaacccaaacgtcgccgccaccggcaagacgccttgcccgggccatgcatcgcctcgacgcccaaaaagcaccgaggttgatctagacctgatcataatcaagccatatcacatctgtagaggtttacttgctttaaaaaacctccacacctccccctgaacctgaaacataaaatgaatgcaattgttgttgttaacttgtttattgcagcttataatggttacaaataaagcaatagcatcacaaatttcacaaataaagcatttttttcactgcattctagttgtggtttgtccaaactcatcaatgtatcttatcatgtctggatctgcggatcaggattggtgacagaaaagccccatccttaggcctcctccttcctagtctcctgatattgggtctaacccccacctcctgttaggcagattccttatctggtgacacacccccatttcctggagccatctctctccttgccagaacctctaaggtttgcttacgatggagccagagaggatcctgggagggagagcttggcagggggtgggagggaagggggggatgcgtgacctgcccggttctcagtggccaccctgcgctaccctctcccagaacctgagctgctctgacgcggctgtctggtgcgtttcactgatcctggtgctgcagcttccttacacttcccaagaggagaagcagtttggaaaaacaaaatcagaataagttggtcctgagttctaactttggctcttcacctttctagtccccaatttatattgttcctccgtgcgtcagttttacctgtgagataaggccagtagccagccccgtcctggcagggctgtggtgaggaggggggtgtccgtgtggaaaactccctttgtgagaatggtgcgtcctcgagctgggcctcatgggccttccgctcactgcccgctttccagtcgggaaacctgtcgtgccagctgcattaacatggtcatagctgtttccttgcgtattgggcgctctccgcttcctcgctcactgactcgctgcgctcggtcgttcgggtaaagcctggggtgcctaatgagcaaaaggccagcaaaaggccaggaaccgtaaaaaggccgcgttgctggcgtttttccataggctccgcccccctgacgagcatcacaaaaatcgacgctcaagtcagaggtggcgaaacccgacaggactataaagataccaggcgtttccccctggaagctccctcgtgcgctctcctgttccgaccctgccgcttaccggatacctgtccgcctttctcccttcgggaagcgtggcgctttctcatagctcacgctgtaggtatctcagttcggtgtaggtcgttcgctccaagctgggctgtgtgcacgaaccccccgttcagcccgaccgctgcgccttatccggtaactatcgtcttgagtccaacccggtaagacacgacttatcgccactggcagcagccactggtaacaggattagcagagcgaggtatgtaggcggtgctacagagttcttgaagtggtggcctaactacggctacactagaagaacagtatttggtatctgcgctctgctgaagccagttaccttcggaaaaagagttggtagctcttgatccggcaaacaaaccaccgctggtagcggtggtttttttgtttgcaagcagcagattacgcgcagaaaaaaaggatctcaagaagatcctttgatcttttctacggggtctgacgctcagtggaacgaaaactcacgttaagggattttggtcatgagattatcaaaaaggatcttcacctagatccttttaaattaaaaatgaagttttaaatcaatctaaagtatatatgagtaaacttggtctgacagttaccaatgcttaatcagtgaggcacctatctcagcgatctgtctatttcgttcatccatagttgcctgactccccgtcgtgtagataactacgatacgggagggcttaccatctggccccagtgctgcaatgataccgcgagaaccacgctcaccggctccagatttatcagcaataaaccagccagccggaagggccgagcgcagaagtggtcctgcaactttatccgcctccatccagtctattaattgttgccgggaagctagagtaagtagttcgccagttaatagtttgcgcaacgttgttgccattgctacaggcatcgtggtgtcacgctcgtcgtttggtatggcttcattcagctccggttcccaacgatcaaggcgagttacatgatcccccatgttgtgcaaaaaagcggttagctccttcggtcctccgatcgttgtcagaagtaagttggccgcagtgttatcactcatggttatggcagcactgcataattctcttactgtcatgccatccgtaagatgcttttctgtgactggtgagtactcaaccaagtcattctgagaatagtgtatgcggcgaccgagttgctcttgcccggcgtcaatacgggataataccgcgccacatagcagaactttaaaagtgctcatcattggaaaacgttcttcggggcgaaaactctcaaggatcttaccgctgttgagatccagttcgatgtaacccactcgtgcacccaactgatcttcagcatcttttactttcaccagcgtttctgggtgagcaaaaacaggaaggcaaaatgccgcaaaaaagggaataagggcgacacggaaatgttgaatactcatactcttcctttttcaatattattgaagcatttatcagggttattgtctcatgagcggatacatatttgaatgtatttagaaaaataaacaaataggggttccgcgcacatttccccgaaaagtgccac

SEQ ID NO: 14 - DNA, 7062 bp, Artificial Sequence
  AAVS1-l_GFP_HCMVpp65 ANET vector V1.G.9
ctaaattgtaagcgttaatattttgttaaaattcgcgttaaatttttgttaaatcagctcattttttaaccaataggccgaaatcggcaaaatcccttataaatcaaaagaatagaccgagatagggttgagtggccgctacagggcgctcccattcgccattcaggctgcgcaactgttgggaagggcgtttcggtgcgggcctcttcgctattacgccagctggcgaaagggggatgtgctgcaaggcgattaagttgggtaacgccagggttttcccagtcacgacgttgtaaaacgacggccagtgagcgcgacgtaatacgactcactatagggcgaattggcggaaggccgtcaaggccgcatgaattgagctctactggcttctgcgccgcctctggcccactgtttccccttcccaggcaggtcctgctttctctgacctgcattctctcccctgggcctgtgccgctttctgtctgcagcttgtggcctgggtcacctctacggctggcccagatccttccctgccgcctccttcaggttccgtcttcctccactccctcttccccttgctctctgctgtgttgctgcccaaggatgctctttccggagcacttccttctcggcgctgcaccacgtgatgtcctctgagcggatcctccccgtgtctgggtcctctccgggcatctctcctccctcacccaaccccatgccgtcttcactcgctgggttcccttttccttctccttctggggcctgtgccatctctcgtttcttaggatggccttctccgacggatgtctcccttgcgtcccgcctccccttcttgtaggcctgcatcatcaccgtttttctggacaaccccaaagtaccccgtctccctggctttagccacctctccatcctcttgctttctttgcctggacaccccgttctcctgtggattcgggtcacctctcactcctttcatttgggcagctcccctaccccccttacctctctagtctgtgctagctcttccagccccctgtcatggcatcttccaggggtccgagagctcagctagtcttcttcctccaacccgggcccctatgtccacttcaggacagcatgtttgctgcctccagggatcctgtgtccccgagctgggaccaccttatattcccagggccggttaatgtggctctggttctgggtacttttatctgtcccctccaccggtatagtaatcaattacggggtcattagttcatagcccatatatggagttccgcgttacataacttacggtaaatggcccgcctggctgaccgcccaacgacccccgcccattgacgtcaataatgacgtatgttcccatagtaacgccaatagggactttccattgacgtcaatgggtggagtatttacggtaaactgcccacttggcagtacatcaagtgtatcatatgccaagtacgccccctattgacgtcaatgacggtaaatggcccgcctggcattatgcccagtacatgaccttatgggactttcctacttggcagtacatctacgtattagtcatcgctattaccatggtgatgcggttttggcagtacatcaatgggcgtggatagcggtttgactcacggggatttccaagtctccaccccattgacgtcaatgggagtttgttttggcaccaaaatcaacgggactttccaaaatgtcgtaacaactccgccccattgacgcaaatgggcggtaggcgtgtacggtgggaggtctatataagcagagctggtttagtgaaccgtcagatcaggtaccgccaccatggaatccgatgagtctggcctgcccgccatggaaatcgagtgcagaatcaccggcaccctgaacggcgtggaatttgagctcgtgggcggaggcgagggcacacctgaacagggcagaatgaccaacaagatgaagtccaccaagggggccctgaccttcagcccctacctgctgtctcacgtgatgggctacggcttctaccacttcggcacctaccccagcggctacgagaaccctttcctgcacgccatcaacaacggcggctacaccaacacccggatcgagaagtacgaggacggcggcgtgctgcacgtgtccttcagctacagatacgaggccggcagagtgatcggcgacttcaaagtgatgggcaccggattccccgaggacagcgtgatcttcaccgacaagatcatccggtccaacgccaccgtggaacatctgcaccccatgggcgacaacgacctggacggcagcttcaccagaaccttctccctgcgggatggcggctactacagcagcgtggtggacagccacatgcacttcaagagcgccatccaccccagcatcctccagaacggcggacccatgttcgccttcagacgggtggaagaggaccacagcaacaccgagctgggcatcgtggaataccagcacgccttcaagacccccgatgccgatgccggcgaggaaggcagtggagagggcagaggaagtctgctaacatgtggtgacgtcgaggagaatcctggcccaatggagtcgcgcggtcgccgttgtcccgaaatgatatccgtactgggtcccatttcggggcacgtgctgaaagccgtgtttagtcgcggcgatacgccggtgctgccgcacgagacgcgactcctgcagacgggtatccacgtacgcgtgagccagccctcgctgatcttggtatcgcagtacacgcccgactcgacgccatgccaccgcggcgacaatcagctgcaggtgcagcacacgtactttacgggcagcgaggtggagaacgtgtcggtcaacgtgcacaaccccacgggccgaagcatctgccccagccaggagcccatgtcgatctatgtgtacgcgctgccgctcaagatgctgaacatccccagcgctaacgaaacccactacccgtcggcggccgagcgcaaacaccgacacctgcccgtagctgacgctgtgattcacgcgtcgggcaagcagatgtggcaggcgcgtctcacggtctcgggactggcctggacgcgtcagcagaaccagtggaaagagcccgacgtctactacacgtcagcgttcgtgtttcccaccaaggacgtggcactgcggcacgtggtgtgcgcgcacgagctggtttgctccatggagaacacgcgcgcaaccaagatgcaggtgataggtgaccagtacgtcaaggtgtacctggagtccttctgcgaggacgtgccctccggcaagctctttatgcacgtcacgctgggctctgacgtggaagaggacctgacgatgacccgcaacccgcaacccttcatgcgcccccacgagcgcaacggctttacggtgttgtgtcccaaaaatatgataatcaaaccgggcaagatctcgcacatcatgctggatgtggcttttacctcacacgagcattttgggctgctgtgtcccaagagcatcccgggcctgagcatctcaggtaacctgttgatgaacgggcagcagatcttcctggaggtacaagccatacgcgagaccgtggaactgcgtcagtacgatcccgtggctgcgctcttctttttcgatatcgacttgctgctgcagcgcgggcctcagtacagcgagcaccccaccttcaccagccagtatcgcatccagggcaagcttgagtaccgacacacctgggaccggcacgacgagggtgccgcccagggcgacgacgacgtctggaccagcggatcggactccgacgaagaactcgtaaccaccgagcgcaagacgccccgcgtcaccggcggcggcgccatggcgggcgcctccacttccgcgggccgcaaacgcaaatcagcatcctcggcgacggcgtgcacgtcgggcgttatgacacgcggccgccttaaggccgagtccaccgtcgcgcccgaagaggacaccgacgaggattccgacaacgaaatccacaatccggccgtgttcacctggccgccctggcaggccggcatcctggcccgcaacctggtgcccatggtggctacggttcagggtcagaatctgaagtaccaggagttcttctgggacgccaacgacatctaccgcatcttcgccgaattggaaggcgtatggcagcccgctgcgcaacccaaacgtcgccgccaccggcaagacgccttgcccgggccatgcatcgcctcgacgcccaaaaagcaccgaggttgatctagacctgatcataatcaagccatatcacatctgtagaggtttacttgctttaaaaaacctccacacctccccctgaacctgaaacataaaatgaatgcaattgttgttgttaacttgtttattgcagcttataatggttacaaataaagcaatagcatcacaaatttcacaaataaagcatttttttcactgcattctagttgtggtttgtccaaactcatcaatgtatcttatcatgtctggatctgcggatcaggattggtgacagaaaagccccatccttaggcctcctccttcctagtctcctgatattgggtctaacccccacctcctgttaggcagattccttatctggtgacacacccccatttcctggagccatctctctccttgccagaacctctaaggtttgcttacgatggagccagagaggatcctgggagggagagcttggcagggggtgggagggaagggggggatgcgtgacctgcccggttctcagtggccaccctgcgctaccctctcccagaacctgagctgctctgacgcggctgtctggtgcgtttcactgatcctggtgctgcagcttccttacacttcccaagaggagaagcagtttggaaaaacaaaatcagaataagttggtcctgagttctaactttggctcttcacctttctagtccccaatttatattgttcctccgtgcgtcagttttacctgtgagataaggccagtagccagccccgtcctggcagggctgtggtgaggaggggggtgtccgtgtggaaaactccctttgtgagaatggtgcgtcctcgagctgggcctcatgggccttccgctcactgcccgctttccagtcgggaaacctgtcgtgccagctgcattaacatggtcatagctgtttccttgcgtattgggcgctctccgcttcctcgctcactgactcgctgcgctcggtcgttcgggtaaagcctggggtgcctaatgagcaaaaggccagcaaaaggccaggaaccgtaaaaaggccgcgttgctggcgtttttccataggctccgcccccctgacgagcatcacaaaaatcgacgctcaagtcagaggtggcgaaacccgacaggactataaagataccaggcgtttccccctggaagctccctcgtgcgctctcctgttccgaccctgccgcttaccggatacctgtccgcctttctcccttcgggaagcgtggcgctttctcatagctcacgctgtaggtatctcagttcggtgtaggtcgttcgctccaagctgggctgtgtgcacgaaccccccgttcagcccgaccgctgcgccttatccggtaactatcgtcttgagtccaacccggtaagacacgacttatcgccactggcagcagccactggtaacaggattagcagagcgaggtatgtaggcggtgctacagagttcttgaagtggtggcctaactacggctacactagaagaacagtatttggtatctgcgctctgctgaagccagttaccttcggaaaaagagttggtagctcttgatccggcaaacaaaccaccgctggtagcggtggtttttttgtttgcaagcagcagattacgcgcagaaaaaaaggatctcaagaagatcctttgatcttttctacggggtctgacgctcagtggaacgaaaactcacgttaagggattttggtcatgagattatcaaaaaggatcttcacctagatccttttaaattaaaaatgaagttttaaatcaatctaaagtatatatgagtaaacttggtctgacagttaccaatgcttaatcagtgaggcacctatctcagcgatctgtctatttcgttcatccatagttgcctgactccccgtcgtgtagataactacgatacgggagggcttaccatctggccccagtgctgcaatgataccgcgagaaccacgctcaccggctccagatttatcagcaataaaccagccagccggaagggccgagcgcagaagtggtcctgcaactttatccgcctccatccagtctattaattgttgccgggaagctagagtaagtagttcgccagttaatagtttgcgcaacgttgttgccattgctacaggcatcgtggtgtcacgctcgtcgtttggtatggcttcattcagctccggttcccaacgatcaaggcgagttacatgatcccccatgttgtgcaaaaaagcggttagctccttcggtcctccgatcgttgtcagaagtaagttggccgcagtgttatcactcatggttatggcagcactgcataattctcttactgtcatgccatccgtaagatgcttttctgtgactggtgagtactcaaccaagtcattctgagaatagtgtatgcggcgaccgagttgctcttgcccggcgtcaatacgggataataccgcgccacatagcagaactttaaaagtgctcatcattggaaaacgttcttcggggcgaaaactctcaaggatcttaccgctgttgagatccagttcgatgtaacccactcgtgcacccaactgatcttcagcatcttttactttcaccagcgtttctgggtgagcaaaaacaggaaggcaaaatgccgcaaaaaagggaataagggcgacacggaaatgttgaatactcatactcttcctttttcaatattattgaagcatttatcagggttattgtctcatgagcggatacatatttgaatgtatttagaaaaataaacaaataggggttccgcgcacatttccccgaaaagtgccac

SEQ ID NO: 15 - DNA, 7062 bp, Artificial Sequence
  AAVS1-l_GFP_HCMVpp65 AIN vector V1.H.1
ctaaattgtaagcgttaatattttgttaaaattcgcgttaaatttttgttaaatcagctcattttttaaccaataggccgaaatcggcaaaatcccttataaatcaaaagaatagaccgagatagggttgagtggccgctacagggcgctcccattcgccattcaggctgcgcaactgttgggaagggcgtttcggtgcgggcctcttcgctattacgccagctggcgaaagggggatgtgctgcaaggcgattaagttgggtaacgccagggttttcccagtcacgacgttgtaaaacgacggccagtgagcgcgacgtaatacgactcactatagggcgaattggcggaaggccgtcaaggccgcatgaattgagctctactggcttctgcgccgcctctggcccactgtttccccttcccaggcaggtcctgctttctctgacctgcattctctcccctgggcctgtgccgctttctgtctgcagcttgtggcctgggtcacctctacggctggcccagatccttccctgccgcctccttcaggttccgtcttcctccactccctcttccccttgctctctgctgtgttgctgcccaaggatgctctttccggagcacttccttctcggcgctgcaccacgtgatgtcctctgagcggatcctccccgtgtctgggtcctctccgggcatctctcctccctcacccaaccccatgccgtcttcactcgctgggttcccttttccttctccttctggggcctgtgccatctctcgtttcttaggatggccttctccgacggatgtctcccttgcgtcccgcctccccttcttgtaggcctgcatcatcaccgtttttctggacaaccccaaagtaccccgtctccctggctttagccacctctccatcctcttgctttctttgcctggacaccccgttctcctgtggattcgggtcacctctcactcctttcatttgggcagctcccctaccccccttacctctctagtctgtgctagctcttccagccccctgtcatggcatcttccaggggtccgagagctcagctagtcttcttcctccaacccgggcccctatgtccacttcaggacagcatgtttgctgcctccagggatcctgtgtccccgagctgggaccaccttatattcccagggccggttaatgtggctctggttctgggtacttttatctgtcccctccaccggtatagtaatcaattacggggtcattagttcatagcccatatatggagttccgcgttacataacttacggtaaatggcccgcctggctgaccgcccaacgacccccgcccattgacgtcaataatgacgtatgttcccatagtaacgccaatagggactttccattgacgtcaatgggtggagtatttacggtaaactgcccacttggcagtacatcaagtgtatcatatgccaagtacgccccctattgacgtcaatgacggtaaatggcccgcctggcattatgcccagtacatgaccttatgggactttcctacttggcagtacatctacgtattagtcatcgctattaccatggtgatgcggttttggcagtacatcaatgggcgtggatagcggtttgactcacggggatttccaagtctccaccccattgacgtcaatgggagtttgttttggcaccaaaatcaacgggactttccaaaatgtcgtaacaactccgccccattgacgcaaatgggcggtaggcgtgtacggtgggaggtctatataagcagagctggtttagtgaaccgtcagatcaggtaccgccaccatggaatccgatgagtctggcctgcccgccatggaaatcgagtgcagaatcaccggcaccctgaacggcgtggaatttgagctcgtgggcggaggcgagggcacacctgaacagggcagaatgaccaacaagatgaagtccaccaagggggccctgaccttcagcccctacctgctgtctcacgtgatgggctacggcttctaccacttcggcacctaccccagcggctacgagaaccctttcctgcacgccatcaacaacggcggctacaccaacacccggatcgagaagtacgaggacggcggcgtgctgcacgtgtccttcagctacagatacgaggccggcagagtgatcggcgacttcaaagtgatgggcaccggattccccgaggacagcgtgatcttcaccgacaagatcatccggtccaacgccaccgtggaacatctgcaccccatgggcgacaacgacctggacggcagcttcaccagaaccttctccctgcgggatggcggctactacagcagcgtggtggacagccacatgcacttcaagagcgccatccaccccagcatcctccagaacggcggacccatgttcgccttcagacgggtggaagaggaccacagcaacaccgagctgggcatcgtggaataccagcacgccttcaagacccccgatgccgatgccggcgaggaaggcagtggagagggcagaggaagtctgctaacatgtggtgacgtcgaggagaatcctggcccaatggagtcgcgcggtcgccgttgtcccgaaatgatatccgtactgggtcccatttcggggcacgtgctgaaagccgtgtttagtcgcggcgatacgccggtgctgccgcacgagacgcgactcctgcagacgggtatccacgtacgcgtgagccagccctcgctgatcttggtatcgcagtacacgcccgactcgacgccatgccaccgcggcgacaatcagctgcaggtgcagcacacgtactttacgggcagcgaggtggagaacgtgtcggtcaacgtgcacaaccccacgggccgaagcatctgccccagccaggagcccatgtcgatctatgtgtacgcgctgccgctcaagatgctgaacatccccagcatcaacgtgcaccactacccgtcggcggccgagcgcaaacaccgacacctgcccgtagctgacgctgtgattcacgcgtcgggcaagcagatgtggcaggcgcgtctcacggtctcgggactggcctggacgcgtcagcagaaccagtggaaagagcccgacgtctactacacgtcagcgttcgtgtttcccaccaaggacgtggcactgcggcacgtggtgtgcgcgcacgagctggtttgctccatggagaacacgcgcgcaaccaagatgcaggtgataggtgaccagtacgtcaaggtgtacctggagtccttctgcgaggacgtgccctccggcaagctctttatgcacgtcacgctgggctctgacgtggaagaggacctgacgatgacccgcaacccgcaacccttcatgcgcccccacgagcgcaacggctttacggtgttgtgtcccaaaaatatgataatcaaaccgggcaagatctcgcacatcatgctggatgtggcttttacctcacacgagcattttgggctgctgtgtcccaagagcatcccgggcctgagcatctcaggtaacctgttgatgaacgggcagcagatcttcctggaggtacaagccatacgcgagaccgtggaactgcgtcagtacgatcccgtggctgcgctcttctttttcgatatcgacttgctgctgcagcgcgggcctcagtacagcgagcaccccaccttcaccagccagtatcgcatccagggcaagcttgagtaccgacacacctgggaccggcacgacgagggtgccgcccagggcgacgacgacgtctggaccagcggatcggactccgacgaagaactcgtaaccaccgagcgcaagacgccccgcgtcaccggcggcggcgccatggcgggcgcctccacttccgcgggccgcaaacgcaaatcagcatcctcggcgacggcgtgcacgtcgggcgttatgacacgcggccgccttaaggccgagtccaccgtcgcgcccgaagaggacaccgacgaggattccgacaacgaaatccacaatccggccgtgttcacctggccgccctggcaggccggcatcctggcccgcaacctggtggcaattaatgctacggttcagggtcagaatctgaagtaccaggagttcttctgggacgccaacgacatctaccgcatcttcgccgaattggaaggcgtatggcagcccgctgcgcaacccaaacgtcgccgccaccggcaagacgccttgcccgggccatgcatcgcctcgacgcccaaaaagcaccgaggttgatctagacctgatcataatcaagccatatcacatctgtagaggtttacttgctttaaaaaacctccacacctccccctgaacctgaaacataaaatgaatgcaattgttgttgttaacttgtttattgcagcttataatggttacaaataaagcaatagcatcacaaatttcacaaataaagcatttttttcactgcattctagttgtggtttgtccaaactcatcaatgtatcttatcatgtctggatctgcggatcaggattggtgacagaaaagccccatccttaggcctcctccttcctagtctcctgatattgggtctaacccccacctcctgttaggcagattccttatctggtgacacacccccatttcctggagccatctctctccttgccagaacctctaaggtttgcttacgatggagccagagaggatcctgggagggagagcttggcagggggtgggagggaagggggggatgcgtgacctgcccggttctcagtggccaccctgcgctaccctctcccagaacctgagctgctctgacgcggctgtctggtgcgtttcactgatcctggtgctgcagcttccttacacttcccaagaggagaagcagtttggaaaaacaaaatcagaataagttggtcctgagttctaactttggctcttcacctttctagtccccaatttatattgttcctccgtgcgtcagttttacctgtgagataaggccagtagccagccccgtcctggcagggctgtggtgaggaggggggtgtccgtgtggaaaactccctttgtgagaatggtgcgtcctcgagctgggcctcatgggccttccgctcactgcccgctttccagtcgggaaacctgtcgtgccagctgcattaacatggtcatagctgtttccttgcgtattgggcgctctccgcttcctcgctcactgactcgctgcgctcggtcgttcgggtaaagcctggggtgcctaatgagcaaaaggccagcaaaaggccaggaaccgtaaaaaggccgcgttgctggcgtttttccataggctccgcccccctgacgagcatcacaaaaatcgacgctcaagtcagaggtggcgaaacccgacaggactataaagataccaggcgtttccccctggaagctccctcgtgcgctctcctgttccgaccctgccgcttaccggatacctgtccgcctttctcccttcgggaagcgtggcgctttctcatagctcacgctgtaggtatctcagttcggtgtaggtcgttcgctccaagctgggctgtgtgcacgaaccccccgttcagcccgaccgctgcgccttatccggtaactatcgtcttgagtccaacccggtaagacacgacttatcgccactggcagcagccactggtaacaggattagcagagcgaggtatgtaggcggtgctacagagttcttgaagtggtggcctaactacggctacactagaagaacagtatttggtatctgcgctctgctgaagccagttaccttcggaaaaagagttggtagctcttgatccggcaaacaaaccaccgctggtagcggtggtttttttgtttgcaagcagcagattacgcgcagaaaaaaaggatctcaagaagatcctttgatcttttctacggggtctgacgctcagtggaacgaaaactcacgttaagggattttggtcatgagattatcaaaaaggatcttcacctagatccttttaaattaaaaatgaagttttaaatcaatctaaagtatatatgagtaaacttggtctgacagttaccaatgcttaatcagtgaggcacctatctcagcgatctgtctatttcgttcatccatagttgcctgactccccgtcgtgtagataactacgatacgggagggcttaccatctggccccagtgctgcaatgataccgcgagaaccacgctcaccggctccagatttatcagcaataaaccagccagccggaagggccgagcgcagaagtggtcctgcaactttatccgcctccatccagtctattaattgttgccgggaagctagagtaagtagttcgccagttaatagtttgcgcaacgttgttgccattgctacaggcatcgtggtgtcacgctcgtcgtttggtatggcttcattcagctccggttcccaacgatcaaggcgagttacatgatcccccatgttgtgcaaaaaagcggttagctccttcggtcctccgatcgttgtcagaagtaagttggccgcagtgttatcactcatggttatggcagcactgcataattctcttactgtcatgccatccgtaagatgcttttctgtgactggtgagtactcaaccaagtcattctgagaatagtgtatgcggcgaccgagttgctcttgcccggcgtcaatacgggataataccgcgccacatagcagaactttaaaagtgctcatcattggaaaacgttcttcggggcgaaaactctcaaggatcttaccgctgttgagatccagttcgatgtaacccactcgtgcacccaactgatcttcagcatcttttactttcaccagcgtttctgggtgagcaaaaacaggaaggcaaaatgccgcaaaaaagggaataagggcgacacggaaatgttgaatactcatactcttcctttttcaatattattgaagcatttatcagggttattgtctcatgagcggatacatatttgaatgtatttagaaaaataaacaaataggggttccgcgcacatttccccgaaaagtgccac

SEQ ID NO: 16 - DNA, 6348 bp, Artificial Sequence
  AAVS1_DRA_Flag-DRB1_6xHis vector V1.I.5
ctaaattgtaagcgttaatattttgttaaaattcgcgttaaatttttgttaaatcagctcattttttaaccaataggccgaaatcggcaaaatcccttataaatcaaaagaatagaccgagatagggttgagtggccgctacagggcgctcccattcgccattcaggctgcgcaactgttgggaagggcgtttcggtgcgggcctcttcgctattacgccagctggcgaaagggggatgtgctgcaaggcgattaagttgggtaacgccagggttttcccagtcacgacgttgtaaaacgacggccagtgagcgcgacgtaatacgactcactatagggcgaattggcggaaggccgtcaaggccgcatgaattgagctctactggcttctgcgccgcctctggcccactgtttccccttcccaggcaggtcctgctttctctgacctgcattctctcccctgggcctgtgccgctttctgtctgcagcttgtggcctgggtcacctctacggctggcccagatccttccctgccgcctccttcaggttccgtcttcctccactccctcttccccttgctctctgctgtgttgctgcccaaggatgctctttccggagcacttccttctcggcgctgcaccacgtgatgtcctctgagcggatcctccccgtgtctgggtcctctccgggcatctctcctccctcacccaaccccatgccgtcttcactcgctgggttcccttttccttctccttctggggcctgtgccatctctcgtttcttaggatggccttctccgacggatgtctcccttgcgtcccgcctccccttcttgtaggcctgcatcatcaccgtttttctggacaaccccaaagtaccccgtctccctggctttagccacctctccatcctcttgctttctttgcctggacaccccgttctcctgtggattcgggtcacctctcactcctttcatttgggcagctcccctaccccccttacctctctagtctgtgctagctcttccagccccctgtcatggcatcttccaggggtccgagagctcagctagtcttcttcctccaacccgggcccctatgtccacttcaggacagcatgtttgctgcctccagggatcctgtgtccccgagctgggaccaccttatattcccagggccggttaatgtggctctggttctgggtacttttatctgtcccctccaccggtatagtaatcaattacggggtcattagttcatagcccatatatggagttccgcgttacataacttacggtaaatggcccgcctggctgaccgcccaacgacccccgcccattgacgtcaataatgacgtatgttcccatagtaacgccaatagggactttccattgacgtcaatgggtggagtatttacggtaaactgcccacttggcagtacatcaagtgtatcatatgccaagtacgccccctattgacgtcaatgacggtaaatggcccgcctggcattatgcccagtacatgaccttatgggactttcctacttggcagtacatctacgtattagtcatcgctattaccatggtgatgcggttttggcagtacatcaatgggcgtggatagcggtttgactcacggggatttccaagtctccaccccattgacgtcaatgggagtttgttttggcaccaaaatcaacgggactttccaaaatgtcgtaacaactccgccccattgacgcaaatgggcggtaggcgtgtacggtgggaggtctatataagcagagctggtttagtgaaccgtcagatcaggtaccatggccataagtggagtccctgtgctaggatttttcatcatagctgtgctgatgagcgctcaggaatcatgggctatcaaagaagaacatgtgatcatccaggccgagttctatctgaatcctgaccaatcaggcgagtttatgtttgactttgatggtgatgagattttccatgtggatatggcaaagaaggagacggtctggcggcttgaagaatttggacgatttgccagctttgaggctcaaggtgcattggccaacatagctgtggacaaagccaacctggaaatcatgacaaagcgctccaactatactccgatcaccaatgtacctccagaggtaactgtgctcacgaacagccctgtggaactgagagagcccaacgtcctcatctgtttcatcgacaagttcaccccaccagtggtcaatgtcacgtggcttcgaaatggaaaacctgtcaccacaggagtgtcagagacagtctttctgcccagggaagatcaccttttccgcaagttccactatctccccttcctgccctcaactgaggacgtttacgactgcagggtggagcactggggcttggatgagcctcttctcaagcactgggagtttgatgctccaagccctctcccagagactacagagaacgtggtgtgtgccctgggcctgactgtgggtctggtgggcatcattattgggaccatcttcatcatcaagggagtgcgcaaaagcaatgcagcagaacgcagaggacctctgcccgggatggactataaggaccacgacggagactacaaggatcatgatattgattacaaagacgatgacgataagggatccggagccacgaacttctctctgttaaagcaagcaggagacgtggaagagaaccctggtcctatggtgtgtctgaagctccctggaggctcctgcatgacagcgctgacagtgacactgatggtgctgagctccccactggctttggctggggacacccgaccacgtttcttgtggcagcttaagttcgaatgtcatttcttcaatgggacggagagagtgcggttgctggaaagatgcatctataaccaagaggagtccgtgcgcttcgacagcgacgtgggggagtaccgggctgtgacggagctgggaaggcctgatgccgagtactggaacagccagaaggacctcctggagcagaggagagccgctgtggacacctactgcagacacaactacggggttggtgagagcttcacagtgcagcggcgagttgagcctaaggtgactgtgtatccttcaaagacccagcccctgcagcaccacaacctcctggtctgctctgtgagtggtttctatccaggcagcattgaagtcaggtggttccggaacggccaggaagagaaggctggggtggtgtccacaggcctgatccagaatggagattggaccttccagaccctggtgatgctggaaacagttcctcggagtggagaggtttacacctgccaagtggagcacccaagtgtgacgagccctctcacagtggaatggagagcacggtctgaatctgcacagagcaagatgctgagtggagtcgggggcttcgtgctgggcctgctcttccttggggccgggctgttcatctacttcaggaatcagaaaggacactctggacttcagccaacaggattcctgagccccgggcatcatcaccatcaccactgactatagtcgtctagacctgatcataatcaagccatatcacatctgtagaggtttacttgctttaaaaaacctccacacctccccctgaacctgaaacataaaatgaatgcaattgttgttgttaacttgtttattgcagcttataatggttacaaataaagcaatagcatcacaaatttcacaaataaagcatttttttcactgcattctagttgtggtttgtccaaactcatcaatgtatcttatcatgtctggatctgcggatcaggattggtgacagaaaagccccatccttaggcctcctccttcctagtctcctgatattgggtctaacccccacctcctgttaggcagattccttatctggtgacacacccccatttcctggagccatctctctccttgccagaacctctaaggtttgcttacgatggagccagagaggatcctgggagggagagcttggcagggggtgggagggaagggggggatgcgtgacctgcccggttctcagtggccaccctgcgctaccctctcccagaacctgagctgctctgacgcggctgtctggtgcgtttcactgatcctggtgctgcagcttccttacacttcccaagaggagaagcagtttggaaaaacaaaatcagaataagttggtcctgagttctaactttggctcttcacctttctagtccccaatttatattgttcctccgtgcgtcagttttacctgtgagataaggccagtagccagccccgtcctggcagggctgtggtgaggaggggggtgtccgtgtggaaaactccctttgtgagaatggtgcgtcctcgagctgggcctcatgggccttccgctcactgcccgctttccagtcgggaaacctgtcgtgccagctgcattaacatggtcatagctgtttccttgcgtattgggcgctctccgcttcctcgctcactgactcgctgcgctcggtcgttcgggtaaagcctggggtgcctaatgagcaaaaggccagcaaaaggccaggaaccgtaaaaaggccgcgttgctggcgtttttccataggctccgcccccctgacgagcatcacaaaaatcgacgctcaagtcagaggtggcgaaacccgacaggactataaagataccaggcgtttccccctggaagctccctcgtgcgctctcctgttccgaccctgccgcttaccggatacctgtccgcctttctcccttcgggaagcgtggcgctttctcatagctcacgctgtaggtatctcagttcggtgtaggtcgttcgctccaagctgggctgtgtgcacgaaccccccgttcagcccgaccgctgcgccttatccggtaactatcgtcttgagtccaacccggtaagacacgacttatcgccactggcagcagccactggtaacaggattagcagagcgaggtatgtaggcggtgctacagagttcttgaagtggtggcctaactacggctacactagaagaacagtatttggtatctgcgctctgctgaagccagttaccttcggaaaaagagttggtagctcttgatccggcaaacaaaccaccgctggtagcggtggtttttttgtttgcaagcagcagattacgcgcagaaaaaaaggatctcaagaagatcctttgatcttttctacggggtctgacgctcagtggaacgaaaactcacgttaagggattttggtcatgagattatcaaaaaggatcttcacctagatccttttaaattaaaaatgaagttttaaatcaatctaaagtatatatgagtaaacttggtctgacagttaccaatgcttaatcagtgaggcacctatctcagcgatctgtctatttcgttcatccatagttgcctgactccccgtcgtgtagataactacgatacgggagggcttaccatctggccccagtgctgcaatgataccgcgagaaccacgctcaccggctccagatttatcagcaataaaccagccagccggaagggccgagcgcagaagtggtcctgcaactttatccgcctccatccagtctattaattgttgccgggaagctagagtaagtagttcgccagttaatagtttgcgcaacgttgttgccattgctacaggcatcgtggtgtcacgctcgtcgtttggtatggcttcattcagctccggttcccaacgatcaaggcgagttacatgatcccccatgttgtgcaaaaaagcggttagctccttcggtcctccgatcgttgtcagaagtaagttggccgcagtgttatcactcatggttatggcagcactgcataattctcttactgtcatgccatccgtaagatgcttttctgtgactggtgagtactcaaccaagtcattctgagaatagtgtatgcggcgaccgagttgctcttgcccggcgtcaatacgggataataccgcgccacatagcagaactttaaaagtgctcatcattggaaaacgttcttcggggcgaaaactctcaaggatcttaccgctgttgagatccagttcgatgtaacccactcgtgcacccaactgatcttcagcatcttttactttcaccagcgtttctgggtgagcaaaaacaggaaggcaaaatgccgcaaaaaagggaataagggcgacacggaaatgttgaatactcatactcttcctttttcaatattattgaagcatttatcagggttattgtctcatgagcggatacatatttgaatgtatttagaaaaataaacaaataggggttccgcgcacatttccccgaaaagtgccac

SEQ ID NO: 17 - DNA, 6342 bp, Artificial Sequence
  AAVS1_DPA1_Flag-DPB1_6xHis vector V1.I.7
ctaaattgtaagcgttaatattttgttaaaattcgcgttaaatttttgttaaatcagctcattttttaaccaataggccgaaatcggcaaaatcccttataaatcaaaagaatagaccgagatagggttgagtggccgctacagggcgctcccattcgccattcaggctgcgcaactgttgggaagggcgtttcggtgcgggcctcttcgctattacgccagctggcgaaagggggatgtgctgcaaggcgattaagttgggtaacgccagggttttcccagtcacgacgttgtaaaacgacggccagtgagcgcgacgtaatacgactcactatagggcgaattggcggaaggccgtcaaggccgcatgaattgagctctactggcttctgcgccgcctctggcccactgtttccccttcccaggcaggtcctgctttctctgacctgcattctctcccctgggcctgtgccgctttctgtctgcagcttgtggcctgggtcacctctacggctggcccagatccttccctgccgcctccttcaggttccgtcttcctccactccctcttccccttgctctctgctgtgttgctgcccaaggatgctctttccggagcacttccttctcggcgctgcaccacgtgatgtcctctgagcggatcctccccgtgtctgggtcctctccgggcatctctcctccctcacccaaccccatgccgtcttcactcgctgggttcccttttccttctccttctggggcctgtgccatctctcgtttcttaggatggccttctccgacggatgtctcccttgcgtcccgcctccccttcttgtaggcctgcatcatcaccgtttttctggacaaccccaaagtaccccgtctccctggctttagccacctctccatcctcttgctttctttgcctggacaccccgttctcctgtggattcgggtcacctctcactcctttcatttgggcagctcccctaccccccttacctctctagtctgtgctagctcttccagccccctgtcatggcatcttccaggggtccgagagctcagctagtcttcttcctccaacccgggcccctatgtccacttcaggacagcatgtttgctgcctccagggatcctgtgtccccgagctgggaccaccttatattcccagggccggttaatgtggctctggttctgggtacttttatctgtcccctccaccggtatagtaatcaattacggggtcattagttcatagcccatatatggagttccgcgttacataacttacggtaaatggcccgcctggctgaccgcccaacgacccccgcccattgacgtcaataatgacgtatgttcccatagtaacgccaatagggactttccattgacgtcaatgggtggagtatttacggtaaactgcccacttggcagtacatcaagtgtatcatatgccaagtacgccccctattgacgtcaatgacggtaaatggcccgcctggcattatgcccagtacatgaccttatgggactttcctacttggcagtacatctacgtattagtcatcgctattaccatggtgatgcggttttggcagtacatcaatgggcgtggatagcggtttgactcacggggatttccaagtctccaccccattgacgtcaatgggagtttgttttggcaccaaaatcaacgggactttccaaaatgtcgtaacaactccgccccattgacgcaaatgggcggtaggcgtgtacggtgggaggtctatataagcagagctggtttagtgaaccgtcagatcaggtaccatgcgccctgaggacagaatgttccatatcagagctgtgatcttgagagccctctccttggctttcctgctgagtctccgaggagctggggccatcaaggcggaccatgtgtcaacttatgccgcgtttgtacagacgcatagaccaacaggggagtttatgtttgaatttgatgaagatgagatgttctatgtggatctggacaagaaggagaccgtctggcatctggaggagtttggccaagccttttcctttgaggctcagggcgggctggctaacattgctatattgaacaacaacttgaataccttgatccagcgttccaaccacactcaggccaccaacgatccccctgaggtgaccgtgtttcccaaggagcctgtggagctgggccagcccaacaccctcatctgccacattgacaagttcttcccaccagtgctcaacgtcacgtggctgtgcaacggggagctggtcactgagggtgtcgctgagagcctcttcctgcccagaacagattacagcttccacaagttccattacctgacctttgtgccctcagcagaggacttctatgactgcagggtggagcactggggcttggaccagccgctcctcaagcactgggaggcccaagagccaatccagatgcctgagacaacggagactgtgctctgtgccctgggcctggtgctgggcctagtcggcatcatcgtgggcaccgtcctcatcataaagtctctgcgttctggccatgaccctagagcccagggaaccctgcccgggatggactataaggaccacgacggagactacaaggatcatgatattgattacaaagacgatgacgataagggatccggagccacgaacttctctctgttaaagcaagcaggagacgtggaagagaaccctggtcctatgatggttctgcaggtttctgcggccccccggacagtggctctgacggcgttactgatggtgctgctcacatctgtggtccagggcagggccactccagagaattaccttttccagggacggcaggaatgctacgcgtttaatgggacacagcgcttcctggagagatacatctacaaccgggaggagttcgcgcgcttcgacagcgacgtgggggagttccgggcggtgacggagctggggcggcctgctgcggagtactggaacagccagaaggacatcctggaggagaagcgggcagtgccggacaggatgtgcagacacaactacgagctgggcgggcccatgaccctgcagcgccgagtccagcctagggtgaatgtttccccctccaagaaggggcccttgcagcaccacaacctgcttgtctgccacgtgacggatttctacccaggcagcattcaagtccgatggttcctgaatggacaggaggaaacagctggggtcgtgtccaccaacctgatccgtaatggagactggaccttccagatcctggtgatgctggaaatgaccccccagcagggagatgtctacacctgccaagtggagcacaccagcctggatagtcctgtcaccgtggagtggaaggcacagtctgattctgcccggagtaagacattgacgggagctgggggcttcgtgctggggctcatcatctgtggagtgggcatcttcatgcacaggaggagcaagaaagttcaacgaggatctgcacccgggcatcatcaccatcaccactgactatagtcgtctagacctgatcataatcaagccatatcacatctgtagaggtttacttgctttaaaaaacctccacacctccccctgaacctgaaacataaaatgaatgcaattgttgttgttaacttgtttattgcagcttataatggttacaaataaagcaatagcatcacaaatttcacaaataaagcatttttttcactgcattctagttgtggtttgtccaaactcatcaatgtatcttatcatgtctggatctgcggatcaggattggtgacagaaaagccccatccttaggcctcctccttcctagtctcctgatattgggtctaacccccacctcctgttaggcagattccttatctggtgacacacccccatttcctggagccatctctctccttgccagaacctctaaggtttgcttacgatggagccagagaggatcctgggagggagagcttggcagggggtgggagggaagggggggatgcgtgacctgcccggttctcagtggccaccctgcgctaccctctcccagaacctgagctgctctgacgcggctgtctggtgcgtttcactgatcctggtgctgcagcttccttacacttcccaagaggagaagcagtttggaaaaacaaaatcagaataagttggtcctgagttctaactttggctcttcacctttctagtccccaatttatattgttcctccgtgcgtcagttttacctgtgagataaggccagtagccagccccgtcctggcagggctgtggtgaggaggggggtgtccgtgtggaaaactccctttgtgagaatggtgcgtcctcgagctgggcctcatgggccttccgctcactgcccgctttccagtcgggaaacctgtcgtgccagctgcattaacatggtcatagctgtttccttgcgtattgggcgctctccgcttcctcgctcactgactcgctgcgctcggtcgttcgggtaaagcctggggtgcctaatgagcaaaaggccagcaaaaggccaggaaccgtaaaaaggccgcgttgctggcgtttttccataggctccgcccccctgacgagcatcacaaaaatcgacgctcaagtcagaggtggcgaaacccgacaggactataaagataccaggcgtttccccctggaagctccctcgtgcgctctcctgttccgaccctgccgcttaccggatacctgtccgcctttctcccttcgggaagcgtggcgctttctcatagctcacgctgtaggtatctcagttcggtgtaggtcgttcgctccaagctgggctgtgtgcacgaaccccccgttcagcccgaccgctgcgccttatccggtaactatcgtcttgagtccaacccggtaagacacgacttatcgccactggcagcagccactggtaacaggattagcagagcgaggtatgtaggcggtgctacagagttcttgaagtggtggcctaactacggctacactagaagaacagtatttggtatctgcgctctgctgaagccagttaccttcggaaaaagagttggtagctcttgatccggcaaacaaaccaccgctggtagcggtggtttttttgtttgcaagcagcagattacgcgcagaaaaaaaggatctcaagaagatcctttgatcttttctacggggtctgacgctcagtggaacgaaaactcacgttaagggattttggtcatgagattatcaaaaaggatcttcacctagatccttttaaattaaaaatgaagttttaaatcaatctaaagtatatatgagtaaacttggtctgacagttaccaatgcttaatcagtgaggcacctatctcagcgatctgtctatttcgttcatccatagttgcctgactccccgtcgtgtagataactacgatacgggagggcttaccatctggccccagtgctgcaatgataccgcgagaaccacgctcaccggctccagatttatcagcaataaaccagccagccggaagggccgagcgcagaagtggtcctgcaactttatccgcctccatccagtctattaattgttgccgggaagctagagtaagtagttcgccagttaatagtttgcgcaacgttgttgccattgctacaggcatcgtggtgtcacgctcgtcgtttggtatggcttcattcagctccggttcccaacgatcaaggcgagttacatgatcccccatgttgtgcaaaaaagcggttagctccttcggtcctccgatcgttgtcagaagtaagttggccgcagtgttatcactcatggttatggcagcactgcataattctcttactgtcatgccatccgtaagatgcttttctgtgactggtgagtactcaaccaagtcattctgagaatagtgtatgcggcgaccgagttgctcttgcccggcgtcaatacgggataataccgcgccacatagcagaactttaaaagtgctcatcattggaaaacgttcttcggggcgaaaactctcaaggatcttaccgctgttgagatccagttcgatgtaacccactcgtgcacccaactgatcttcagcatcttttactttcaccagcgtttctgggtgagcaaaaacaggaaggcaaaatgccgcaaaaaagggaataagggcgacacggaaatgttgaatactcatactcttcctttttcaatattattgaagcatttatcagggttattgtctcatgagcggatacatatttgaatgtatttagaaaaataaacaaataggggttccgcgcacatttccccgaaaagtgccac

SEQ ID NO: 18 - DNA, 2762 bp, Artificial Sequence
  HLA-A-sg-sp-opti1 vector V2.A.1
ctaaattgtaagcgttaatattttgttaaaattcgcgttaaatttttgttaaatcagctcattttttaaccaataggccgaaatcggcaaaatcccttataaatcaaaagaatagaccgagatagggttgagtggccgctacagggcgctcccattcgccattcaggctgcgcaactgttgggaagggcgtttcggtgcgggcctcttcgctattacgccagctggcgaaagggggatgtgctgcaaggcgattaagttgggtaacgccagggttttcccagtcacgacgttgtaaaacgacggccagtgagcgcgacgtaatacgactcactatagggcgaattggcggaaggccgtcaaggccgcatggatccaaggtcgggcaggaagagggcctatttcccatgattccttcatatttgcatatacgatacaaggctgttagagagataattagaattaatttgactgtaaacacaaagatattagtacaaaatacgtgacgtagaaagtaataatttcttgggtagtttgcagttttaaaattatgttttaaaatggactatcatatgcttaccgtaacttgaaagtatttcgatttcttggctttatatatcttgtggaaaggacgaaacaccgagggttcggggcgccatgagtttaagagctatgctggaaacagcatagcaagtttaaataaggctagtccgttatcaacttgaaaaagtggcaccgagtcggtgctttttttcagacatccatagatctagctcgagttttttttctagactgggcctcatgggccttccgctcactgcccgctttccagtcgggaaacctgtcgtgccagctgcattaacatggtcatagctgtttccttgcgtattgggcgctctccgcttcctcgctcactgactcgctgcgctcggtcgttcgggtaaagcctggggtgcctaatgagcaaaaggccagcaaaaggccaggaaccgtaaaaaggccgcgttgctggcgtttttccataggctccgcccccctgacgagcatcacaaaaatcgacgctcaagtcagaggtggcgaaacccgacaggactataaagataccaggcgtttccccctggaagctccctcgtgcgctctcctgttccgaccctgccgcttaccggatacctgtccgcctttctcccttcgggaagcgtggcgctttctcatagctcacgctgtaggtatctcagttcggtgtaggtcgttcgctccaagctgggctgtgtgcacgaaccccccgttcagcccgaccgctgcgccttatccggtaactatcgtcttgagtccaacccggtaagacacgacttatcgccactggcagcagccactggtaacaggattagcagagcgaggtatgtaggcggtgctacagagttcttgaagtggtggcctaactacggctacactagaagaacagtatttggtatctgcgctctgctgaagccagttaccttcggaaaaagagttggtagctcttgatccggcaaacaaaccaccgctggtagcggtggtttttttgtttgcaagcagcagattacgcgcagaaaaaaaggatctcaagaagatcctttgatcttttctacggggtctgacgctcagtggaacgaaaactcacgttaagggattttggtcatgagattatcaaaaaggatcttcacctagatccttttaaattaaaaatgaagttttaaatcaatctaaagtatatatgagtaaacttggtctgacagttaccaatgcttaatcagtgaggcacctatctcagcgatctgtctatttcgttcatccatagttgcctgactccccgtcgtgtagataactacgatacgggagggcttaccatctggccccagtgctgcaatgataccgcgagaaccacgctcaccggctccagatttatcagcaataaaccagccagccggaagggccgagcgcagaagtggtcctgcaactttatccgcctccatccagtctattaattgttgccgggaagctagagtaagtagttcgccagttaatagtttgcgcaacgttgttgccattgctacaggcatcgtggtgtcacgctcgtcgtttggtatggcttcattcagctccggttcccaacgatcaaggcgagttacatgatcccccatgttgtgcaaaaaagcggttagctccttcggtcctccgatcgttgtcagaagtaagttggccgcagtgttatcactcatggttatggcagcactgcataattctcttactgtcatgccatccgtaagatgcttttctgtgactggtgagtactcaaccaagtcattctgagaatagtgtatgcggcgaccgagttgctcttgcccggcgtcaatacgggataataccgcgccacatagcagaactttaaaagtgctcatcattggaaaacgttcttcggggcgaaaactctcaaggatcttaccgctgttgagatccagttcgatgtaacccactcgtgcacccaactgatcttcagcatcttttactttcaccagcgtttctgggtgagcaaaaacaggaaggcaaaatgccgcaaaaaagggaataagggcgacacggaaatgttgaatactcatactcttcctttttcaatattattgaagcatttatcagggttattgtctcatgagcggatacatatttgaatgtatttagaaaaataaacaaataggggttccgcgcacatttccccgaaaagtgccac

SEQ ID NO: 19 - DNA, 2762 bp, Artificial Sequence
  HLA-B-sg-sp-3 vector V2.A.7
ctaaattgtaagcgttaatattttgttaaaattcgcgttaaatttttgttaaatcagctcattttttaaccaataggccgaaatcggcaaaatcccttataaatcaaaagaatagaccgagatagggttgagtggccgctacagggcgctcccattcgccattcaggctgcgcaactgttgggaagggcgtttcggtgcgggcctcttcgctattacgccagctggcgaaagggggatgtgctgcaaggcgattaagttgggtaacgccagggttttcccagtcacgacgttgtaaaacgacggccagtgagcgcgacgtaatacgactcactatagggcgaattggcggaaggccgtcaaggccgcatggatccaaggtcgggcaggaagagggcctatttcccatgattccttcatatttgcatatacgatacaaggctgttagagagataattagaattaatttgactgtaaacacaaagatattagtacaaaatacgtgacgtagaaagtaataatttcttgggtagtttgcagttttaaaattatgttttaaaatggactatcatatgcttaccgtaacttgaaagtatttcgatttcttggctttatatatcttgtggaaaggacgaaacaccgtagaaatacctcatggagtgtttaagagctatgctggaaacagcatagcaagtttaaataaggctagtccgttatcaacttgaaaaagtggcaccgagtcggtgctttttttcagacatccatagatctagctcgagttttttttctagactgggcctcatgggccttccgctcactgcccgctttccagtcgggaaacctgtcgtgccagctgcattaacatggtcatagctgtttccttgcgtattgggcgctctccgcttcctcgctcactgactcgctgcgctcggtcgttcgggtaaagcctggggtgcctaatgagcaaaaggccagcaaaaggccaggaaccgtaaaaaggccgcgttgctggcgtttttccataggctccgcccccctgacgagcatcacaaaaatcgacgctcaagtcagaggtggcgaaacccgacaggactataaagataccaggcgtttccccctggaagctccctcgtgcgctctcctgttccgaccctgccgcttaccggatacctgtccgcctttctcccttcgggaagcgtggcgctttctcatagctcacgctgtaggtatctcagttcggtgtaggtcgttcgctccaagctgggctgtgtgcacgaaccccccgttcagcccgaccgctgcgccttatccggtaactatcgtcttgagtccaacccggtaagacacgacttatcgccactggcagcagccactggtaacaggattagcagagcgaggtatgtaggcggtgctacagagttcttgaagtggtggcctaactacggctacactagaagaacagtatttggtatctgcgctctgctgaagccagttaccttcggaaaaagagttggtagctcttgatccggcaaacaaaccaccgctggtagcggtggtttttttgtttgcaagcagcagattacgcgcagaaaaaaaggatctcaagaagatcctttgatcttttctacggggtctgacgctcagtggaacgaaaactcacgttaagggattttggtcatgagattatcaaaaaggatcttcacctagatccttttaaattaaaaatgaagttttaaatcaatctaaagtatatatgagtaaacttggtctgacagttaccaatgcttaatcagtgaggcacctatctcagcgatctgtctatttcgttcatccatagttgcctgactccccgtcgtgtagataactacgatacgggagggcttaccatctggccccagtgctgcaatgataccgcgagaaccacgctcaccggctccagatttatcagcaataaaccagccagccggaagggccgagcgcagaagtggtcctgcaactttatccgcctccatccagtctattaattgttgccgggaagctagagtaagtagttcgccagttaatagtttgcgcaacgttgttgccattgctacaggcatcgtggtgtcacgctcgtcgtttggtatggcttcattcagctccggttcccaacgatcaaggcgagttacatgatcccccatgttgtgcaaaaaagcggttagctccttcggtcctccgatcgttgtcagaagtaagttggccgcagtgttatcactcatggttatggcagcactgcataattctcttactgtcatgccatccgtaagatgcttttctgtgactggtgagtactcaaccaagtcattctgagaatagtgtatgcggcgaccgagttgctcttgcccggcgtcaatacgggataataccgcgccacatagcagaactttaaaagtgctcatcattggaaaacgttcttcggggcgaaaactctcaaggatcttaccgctgttgagatccagttcgatgtaacccactcgtgcacccaactgatcttcagcatcttttactttcaccagcgtttctgggtgagcaaaaacaggaaggcaaaatgccgcaaaaaagggaataagggcgacacggaaatgttgaatactcatactcttcctttttcaatattattgaagcatttatcagggttattgtctcatgagcggatacatatttgaatgtatttagaaaaataaacaaataggggttccgcgcacatttccccgaaaagtgccac

SEQ ID NO: 20 - DNA, 2762 bp, Artificial Sequence
  HLA-C-sg-sp-4 vector V2.B.3
ctaaattgtaagcgttaatattttgttaaaattcgcgttaaatttttgttaaatcagctcattttttaaccaataggccgaaatcggcaaaatcccttataaatcaaaagaatagaccgagatagggttgagtggccgctacagggcgctcccattcgccattcaggctgcgcaactgttgggaagggcgtttcggtgcgggcctcttcgctattacgccagctggcgaaagggggatgtgctgcaaggcgattaagttgggtaacgccagggttttcccagtcacgacgttgtaaaacgacggccagtgagcgcgacgtaatacgactcactatagggcgaattggcggaaggccgtcaaggccgcatggatccaaggtcgggcaggaagagggcctatttcccatgattccttcatatttgcatatacgatacaaggctgttagagagataattagaattaatttgactgtaaacacaaagatattagtacaaaatacgtgacgtagaaagtaataatttcttgggtagtttgcagttttaaaattatgttttaaaatggactatcatatgcttaccgtaacttgaaagtatttcgatttcttggctttatatatcttgtggaaaggacgaaacaccggggccggagtattgggaccgtttaagagctatgctggaaacagcatagcaagtttaaataaggctagtccgttatcaacttgaaaaagtggcaccgagtcggtgctttttttcagacatccatagatctagctcgagttttttttctagactgggcctcatgggccttccgctcactgcccgctttccagtcgggaaacctgtcgtgccagctgcattaacatggtcatagctgtttccttgcgtattgggcgctctccgcttcctcgctcactgactcgctgcgctcggtcgttcgggtaaagcctggggtgcctaatgagcaaaaggccagcaaaaggccaggaaccgtaaaaaggccgcgttgctggcgtttttccataggctccgcccccctgacgagcatcacaaaaatcgacgctcaagtcagaggtggcgaaacccgacaggactataaagataccaggcgtttccccctggaagctccctcgtgcgctctcctgttccgaccctgccgcttaccggatacctgtccgcctttctcccttcgggaagcgtggcgctttctcatagctcacgctgtaggtatctcagttcggtgtaggtcgttcgctccaagctgggctgtgtgcacgaaccccccgttcagcccgaccgctgcgccttatccggtaactatcgtcttgagtccaacccggtaagacacgacttatcgccactggcagcagccactggtaacaggattagcagagcgaggtatgtaggcggtgctacagagttcttgaagtggtggcctaactacggctacactagaagaacagtatttggtatctgcgctctgctgaagccagttaccttcggaaaaagagttggtagctcttgatccggcaaacaaaccaccgctggtagcggtggtttttttgtttgcaagcagcagattacgcgcagaaaaaaaggatctcaagaagatcctttgatcttttctacggggtctgacgctcagtggaacgaaaactcacgttaagggattttggtcatgagattatcaaaaaggatcttcacctagatccttttaaattaaaaatgaagttttaaatcaatctaaagtatatatgagtaaacttggtctgacagttaccaatgcttaatcagtgaggcacctatctcagcgatctgtctatttcgttcatccatagttgcctgactccccgtcgtgtagataactacgatacgggagggcttaccatctggccccagtgctgcaatgataccgcgagaaccacgctcaccggctccagatttatcagcaataaaccagccagccggaagggccgagcgcagaagtggtcctgcaactttatccgcctccatccagtctattaattgttgccgggaagctagagtaagtagttcgccagttaatagtttgcgcaacgttgttgccattgctacaggcatcgtggtgtcacgctcgtcgtttggtatggcttcattcagctccggttcccaacgatcaaggcgagttacatgatcccccatgttgtgcaaaaaagcggttagctccttcggtcctccgatcgttgtcagaagtaagttggccgcagtgttatcactcatggttatggcagcactgcataattctcttactgtcatgccatccgtaagatgcttttctgtgactggtgagtactcaaccaagtcattctgagaatagtgtatgcggcgaccgagttgctcttgcccggcgtcaatacgggataataccgcgccacatagcagaactttaaaagtgctcatcattggaaaacgttcttcggggcgaaaactctcaaggatcttaccgctgttgagatccagttcgatgtaacccactcgtgcacccaactgatcttcagcatcttttactttcaccagcgtttctgggtgagcaaaaacaggaaggcaaaatgccgcaaaaaagggaataagggcgacacggaaatgttgaatactcatactcttcctttttcaatattattgaagcatttatcagggttattgtctcatgagcggatacatatttgaatgtatttagaaaaataaacaaataggggttccgcgcacatttccccgaaaagtgccac

SEQ ID NO: 21 - DNA, 2762 bp, Artificial Sequence
  HLA-A-ex2-3_sg-sp-opti_1 vector V2.I.10
ctaaattgtaagcgttaatattttgttaaaattcgcgttaaatttttgttaaatcagctcattttttaaccaataggccgaaatcggcaaaatcccttataaatcaaaagaatagaccgagatagggttgagtggccgctacagggcgctcccattcgccattcaggctgcgcaactgttgggaagggcgtttcggtgcgggcctcttcgctattacgccagctggcgaaagggggatgtgctgcaaggcgattaagttgggtaacgccagggttttcccagtcacgacgttgtaaaacgacggccagtgagcgcgacgtaatacgactcactatagggcgaattggcggaaggccgtcaaggccgcatggatccaaggtcgggcaggaagagggcctatttcccatgattccttcatatttgcatatacgatacaaggctgttagagagataattagaattaatttgactgtaaacacaaagatattagtacaaaatacgtgacgtagaaagtaataatttcttgggtagtttgcagttttaaaattatgttttaaaatggactatcatatgcttaccgtaacttgaaagtatttcgatttcttggctttatatatcttgtggaaaggacgaaacaccgtccccaggctctcactgaagtttaagagctatgctggaaacagcatagcaagtttaaataaggctagtccgttatcaacttgaaaaagtggcaccgagtcggtgctttttttcagacatccatagatctagctcgagttttttttctagactgggcctcatgggccttccgctcactgcccgctttccagtcgggaaacctgtcgtgccagctgcattaacatggtcatagctgtttccttgcgtattgggcgctctccgcttcctcgctcactgactcgctgcgctcggtcgttcgggtaaagcctggggtgcctaatgagcaaaaggccagcaaaaggccaggaaccgtaaaaaggccgcgttgctggcgtttttccataggctccgcccccctgacgagcatcacaaaaatcgacgctcaagtcagaggtggcgaaacccgacaggactataaagataccaggcgtttccccctggaagctccctcgtgcgctctcctgttccgaccctgccgcttaccggatacctgtccgcctttctcccttcgggaagcgtggcgctttctcatagctcacgctgtaggtatctcagttcggtgtaggtcgttcgctccaagctgggctgtgtgcacgaaccccccgttcagcccgaccgctgcgccttatccggtaactatcgtcttgagtccaacccggtaagacacgacttatcgccactggcagcagccactggtaacaggattagcagagcgaggtatgtaggcggtgctacagagttcttgaagtggtggcctaactacggctacactagaagaacagtatttggtatctgcgctctgctgaagccagttaccttcggaaaaagagttggtagctcttgatccggcaaacaaaccaccgctggtagcggtggtttttttgtttgcaagcagcagattacgcgcagaaaaaaaggatctcaagaagatcctttgatcttttctacggggtctgacgctcagtggaacgaaaactcacgttaagggattttggtcatgagattatcaaaaaggatcttcacctagatccttttaaattaaaaatgaagttttaaatcaatctaaagtatatatgagtaaacttggtctgacagttaccaatgcttaatcagtgaggcacctatctcagcgatctgtctatttcgttcatccatagttgcctgactccccgtcgtgtagataactacgatacgggagggcttaccatctggccccagtgctgcaatgataccgcgagaaccacgctcaccggctccagatttatcagcaataaaccagccagccggaagggccgagcgcagaagtggtcctgcaactttatccgcctccatccagtctattaattgttgccgggaagctagagtaagtagttcgccagttaatagtttgcgcaacgttgttgccattgctacaggcatcgtggtgtcacgctcgtcgtttggtatggcttcattcagctccggttcccaacgatcaaggcgagttacatgatcccccatgttgtgcaaaaaagcggttagctccttcggtcctccgatcgttgtcagaagtaagttggccgcagtgttatcactcatggttatggcagcactgcataattctcttactgtcatgccatccgtaagatgcttttctgtgactggtgagtactcaaccaagtcattctgagaatagtgtatgcggcgaccgagttgctcttgcccggcgtcaatacgggataataccgcgccacatagcagaactttaaaagtgctcatcattggaaaacgttcttcggggcgaaaactctcaaggatcttaccgctgttgagatccagttcgatgtaacccactcgtgcacccaactgatcttcagcatcttttactttcaccagcgtttctgggtgagcaaaaacaggaaggcaaaatgccgcaaaaaagggaataagggcgacacggaaatgttgaatactcatactcttcctttttcaatattattgaagcatttatcagggttattgtctcatgagcggatacatatttgaatgtatttagaaaaataaacaaataggggttccgcgcacatttccccgaaaagtgccac

SEQ ID NO: 22 - DNA, 2763 bp, Artificial Sequence
  HLA-A-ex2-3_sg-sp-opti_2 vector V2.J.1
ctaaattgtaagcgttaatattttgttaaaattcgcgttaaatttttgttaaatcagctcattttttaaccaataggccgaaatcggcaaaatcccttataaatcaaaagaatagaccgagatagggttgagtggccgctacagggcgctcccattcgccattcaggctgcgcaactgttgggaagggcgtttcggtgcgggcctcttcgctattacgccagctggcgaaagggggatgtgctgcaaggcgattaagttgggtaacgccagggttttcccagtcacgacgttgtaaaacgacggccagtgagcgcgacgtaatacgactcactatagggcgaattggcggaaggccgtcaaggccgcatggatccaaggtcgggcaggaagagggcctatttcccatgattccttcatatttgcatatacgatacaaggctgttagagagataattagaattaatttgactgtaaacacaaagatattagtacaaaatacgtgacgtagaaagtaataatttcttgggtagtttgcagttttaaaattatgttttaaaatggactatcatatgcttaccgtaacttgaaagtatttcgatttcttggctttatatatcttgtggaaaggacgaaacaccgcaggctctcactgaacgggagtttaagagctatgctggaaacagcatagcaagtttaaataaggctagtccgttatcaacttgaaaaagtggcaccgagtcggtgctttttttcagacatccatagatctagctcgagttttttttctagactgggcctcatgggccttccgctcactgcccgctttccagtcgggaaacctgtcgtgccagctgcattaacatggtcatagctgtttccttgcgtattgggcgctctccgcttcctcgctcactgactcgctgcgctcggtcgttcgggtaaagcctggggtgcctaatgagcaaaaggccagcaaaaggccaggaaccgtaaaaaggccgcgttgctggcgtttttccataggctccgcccccctgacgagcatcacaaaaatcgacgctcaagtcagaggtggcgaaacccgacaggactataaagataccaggcgtttccccctggaagctccctcgtgcgctctcctgttccgaccctgccgcttaccggatacctgtccgcctttctcccttcgggaagcgtggcgctttctcatagctcacgctgtaggtatctcagttcggtgtaggtcgttcgctccaagctgggctgtgtgcacgaaccccccgttcagcccgaccgctgcgccttatccggtaactatcgtcttgagtccaacccggtaagacacgacttatcgccactggcagcagccactggtaacaggattagcagagcgaggtatgtaggcggtgctacagagttcttgaagtggtggcctaactacggctacactagaagaacagtatttggtatctgcgctctgctgaagccagttaccttcggaaaaagagttggtagctcttgatccggcaaacaaaccaccgctggtagcggtggtttttttgtttgcaagcagcagattacgcgcagaaaaaaaggatctcaagaagatcctttgatcttttctacggggtctgacgctcagtggaacgaaaactcacgttaagggattttggtcatgagattatcaaaaaggatcttcacctagatccttttaaattaaaaatgaagttttaaatcaatctaaagtatatatgagtaaacttggtctgacagttaccaatgcttaatcagtgaggcacctatctcagcgatctgtctatttcgttcatccatagttgcctgactccccgtcgtgtagataactacgatacgggagggcttaccatctggccccagtgctgcaatgataccgcgagaaccacgctcaccggctccagatttatcagcaataaaccagccagccggaagggccgagcgcagaagtggtcctgcaactttatccgcctccatccagtctattaattgttgccgggaagctagagtaagtagttcgccagttaatagtttgcgcaacgttgttgccattgctacaggcatcgtggtgtcacgctcgtcgtttggtatggcttcattcagctccggttcccaacgatcaaggcgagttacatgatcccccatgttgtgcaaaaaagcggttagctccttcggtcctccgatcgttgtcagaagtaagttggccgcagtgttatcactcatggttatggcagcactgcataattctcttactgtcatgccatccgtaagatgcttttctgtgactggtgagtactcaaccaagtcattctgagaatagtgtatgcggcgaccgagttgctcttgcccggcgtcaatacgggataataccgcgccacatagcagaactttaaaagtgctcatcattggaaaacgttcttcggggcgaaaactctcaaggatcttaccgctgttgagatccagttcgatgtaacccactcgtgcacccaactgatcttcagcatcttttactttcaccagcgtttctgggtgagcaaaaacaggaaggcaaaatgccgcaaaaaagggaataagggcgacacggaaatgttgaatactcatactcttcctttttcaatattattgaagcatttatcagggttattgtctcatgagcggatacatatttgaatgtatttagaaaaataaacaaataggggttccgcgcacatttccccgaaaagtgccac

SEQ ID NO: 23 - DNA, 2762 bp, Artificial Sequence
  AAVSI_sg-sp-opti_3 vector V2.J.6
ctaaattgtaagcgttaatattttgttaaaattcgcgttaaatttttgttaaatcagctcattttttaaccaataggccgaaatcggcaaaatcccttataaatcaaaagaatagaccgagatagggttgagtggccgctacagggcgctcccattcgccattcaggctgcgcaactgttgggaagggcgtttcggtgcgggcctcttcgctattacgccagctggcgaaagggggatgtgctgcaaggcgattaagttgggtaacgccagggttttcccagtcacgacgttgtaaaacgacggccagtgagcgcgacgtaatacgactcactatagggcgaattggcggaaggccgtcaaggccgcatggatccaaggtcgggcaggaagagggcctatttcccatgattccttcatatttgcatatacgatacaaggctgttagagagataattagaattaatttgactgtaaacacaaagatattagtacaaaatacgtgacgtagaaagtaataatttcttgggtagtttgcagttttaaaattatgttttaaaatggactatcatatgcttaccgtaacttgaaagtatttcgatttcttggctttatatatcttgtggaaaggacgaaacaccgtcaccaatcctgtccctaggtttaagagctatgctggaaacagcatagcaagtttaaataaggctagtccgttatcaacttgaaaaagtggcaccgagtcggtgctttttttcagacatccatagatctagctcgagttttttttctagactgggcctcatgggccttccgctcactgcccgctttccagtcgggaaacctgtcgtgccagctgcattaacatggtcatagctgtttccttgcgtattgggcgctctccgcttcctcgctcactgactcgctgcgctcggtcgttcgggtaaagcctggggtgcctaatgagcaaaaggccagcaaaaggccaggaaccgtaaaaaggccgcgttgctggcgtttttccataggctccgcccccctgacgagcatcacaaaaatcgacgctcaagtcagaggtggcgaaacccgacaggactataaagataccaggcgtttccccctggaagctccctcgtgcgctctcctgttccgaccctgccgcttaccggatacctgtccgcctttctcccttcgggaagcgtggcgctttctcatagctcacgctgtaggtatctcagttcggtgtaggtcgttcgctccaagctgggctgtgtgcacgaaccccccgttcagcccgaccgctgcgccttatccggtaactatcgtcttgagtccaacccggtaagacacgacttatcgccactggcagcagccactggtaacaggattagcagagcgaggtatgtaggcggtgctacagagttcttgaagtggtggcctaactacggctacactagaagaacagtatttggtatctgcgctctgctgaagccagttaccttcggaaaaagagttggtagctcttgatccggcaaacaaaccaccgctggtagcggtggtttttttgtttgcaagcagcagattacgcgcagaaaaaaaggatctcaagaagatcctttgatcttttctacggggtctgacgctcagtggaacgaaaactcacgttaagggattttggtcatgagattatcaaaaaggatcttcacctagatccttttaaattaaaaatgaagttttaaatcaatctaaagtatatatgagtaaacttggtctgacagttaccaatgcttaatcagtgaggcacctatctcagcgatctgtctatttcgttcatccatagttgcctgactccccgtcgtgtagataactacgatacgggagggcttaccatctggccccagtgctgcaatgataccgcgagaaccacgctcaccggctccagatttatcagcaataaaccagccagccggaagggccgagcgcagaagtggtcctgcaactttatccgcctccatccagtctattaattgttgccgggaagctagagtaagtagttcgccagttaatagtttgcgcaacgttgttgccattgctacaggcatcgtggtgtcacgctcgtcgtttggtatggcttcattcagctccggttcccaacgatcaaggcgagttacatgatcccccatgttgtgcaaaaaagcggttagctccttcggtcctccgatcgttgtcagaagtaagttggccgcagtgttatcactcatggttatggcagcactgcataattctcttactgtcatgccatccgtaagatgcttttctgtgactggtgagtactcaaccaagtcattctgagaatagtgtatgcggcgaccgagttgctcttgcccggcgtcaatacgggataataccgcgccacatagcagaactttaaaagtgctcatcattggaaaacgttcttcggggcgaaaactctcaaggatcttaccgctgttgagatccagttcgatgtaacccactcgtgcacccaactgatcttcagcatcttttactttcaccagcgtttctgggtgagcaaaaacaggaaggcaaaatgccgcaaaaaagggaataagggcgacacggaaatgttgaatactcatactcttcctttttcaatattattgaagcatttatcagggttattgtctcatgagcggatacatatttgaatgtatttagaaaaataaacaaataggggttccgcgcacatttccccgaaaagtgccac

SEQ ID NO: 24 - DNA, 6125 bp, Artificial Sequence
  AAVS_Efla-intron_F14_RFPnls_F15 vector V4.B.2
ctaaattgtaagcgttaatattttgttaaaattcgcgttaaatttttgttaaatcagctcattttttaaccaataggccgaaatcggcaaaatcccttataaatcaaaagaatagaccgagatagggttgagtggccgctacagggcgctcccattcgccattcaggctgcgcaactgttgggaagggcgtttcggtgcgggcctcttcgctattacgccagctggcgaaagggggatgtgctgcaaggcgattaagttgggtaacgccagggttttcccagtcacgacgttgtaaaacgacggccagtgagcgcgacgtaatacgactcactatagggcgaattggcggaaggccgtcaaggccgcatgaattgagctctactggcttctgcgccgcctctggcccactgtttccccttcccaggcaggtcctgctttctctgacctgcattctctcccctgggcctgtgccgctttctgtctgcagcttgtggcctgggtcacctctacggctggcccagatccttccctgccgcctccttcaggttccgtcttcctccactccctcttccccttgctctctgctgtgttgctgcccaaggatgctctttccggagcacttccttctcggcgctgcaccacgtgatgtcctctgagcggatcctccccgtgtctgggtcctctccgggcatctctcctccctcacccaaccccatgccgtcttcactcgctgggttcccttttccttctccttctggggcctgtgccatctctcgtttcttaggatggccttctccgacggatgtctcccttgcgtcccgcctccccttcttgtaggcctgcatcatcaccgtttttctggacaaccccaaagtaccccgtctccctggctttagccacctctccatcctcttgctttctttgcctggacaccccgttctcctgtggattcgggtcacctctcactcctttcatttgggcagctcccctaccccccttacctctctagtctgtgctagctcttccagccccctgtcatggcatcttccaggggtccgagagctcagctagtcttcttcctccaacccgggcccctatgtccacttcaggacagcatgtttgctgcctccagggatcctgtgtccccgagctgggaccaccttatattcccagggccggttaatgtggctctggttctgggtacttttatctgtcccctccaccgggtggctccggtgcccgtcagtgggcagagcgcacatcgcccacagtccccgagaagttggggggaggggtcggcaattgaaccggtgcctagagaaggtggcgcggggtaaactgggaaagtgatgtcgtgtactggctccgcctttttcccgagggtgggggagaaccgtatataagtgcagtagtcgccgtgaacgttctttttcgcaacgggtttgccgccagaacacaggtaagtgccgtgtgtggttcccgcgggcctggcctctttacgggttatggcccttgcgtgccttgaattacttccactggctgcagtacgtgattcttgatcccgagcttcgggttggaagtgggtgggagagttcgaggccttgcgcttaaggagccccttcgcctcgtgcttgagttgaggcctggcctgggcgctggggccgccgcgtgcgaatctggtggcaccttcgcgcctgtctcgctgctttcgataagtctctagccatttaaaatttttgatgacctgctgcgacgctttttttctggcaagatagtcttgtaaatgcgggccaagatctgcacactggtatttcggtttttggggccgcgggcggcgacggggcccgtgcgtcccagcgcacatgttcggcgaggcggggcctgcgagcgcggccaccgagaatcggacgggggtagtctcaagctggccggcctgctctggtgcctggcctcgcgccgccgtgtatcgccccgccctgggcggcaaggctggcccggtcggcaccagttgcgtgagcggaaagatggccgcttcccggccctgctgcagggagctcaaaatggaggacgcggcgctcgggagagcgggcgggtgagtcacccacacaaaggaaaagggcctttccgtcctcagccgtcgcttcatgtgactccacggagtaccgggcgccgtccaggcacctcgattagttctcgagcttttggagtacgtcgtctttaggttggggggaggggttttatgcgatggagtttccccacactgagtgggtggagactgaagttaggccagcttggcacttgatgtaattctccttggaatttgccctttttgagtttggatcttggttcattctcaagcctcagacagtggttcaaagtttttttcttccatttcaggtgtcgtgactggtaccggaagttcctattccgaagttcctattctatcagaagtataggaacttcgtaccgagaccatggccccaaagaagaagcggaaggtcggtatccacggagtcccagcagccatgagcgagctgatcaaagaaaacatgcacatgaagctgtacatggaaggcaccgtgaacaaccaccacttcaagtgcaccagcgagggcgagggcaagccttacgagggcacccagaccatgaagatcaaggtggtggaaggcggccctctgcccttcgcctttgatatcctggccaccagctttatgtacggcagcaaggccttcatcaaccacacccagggcatccccgatttcttcaagcagagcttccccgagggcttcacctgggagcggatcaccacatacgaggacggcggagtgctgaccgccacccaggataccagcttccagaacggctgcatcatctacaacgtgaagattaacggcgtgaatttccccagcaacggccccgtgatgcagaagaaaaccagaggctgggaggccaacaccgagatgctgtaccctgccgatggcggcctgagaggccattctcagatggccctgaaactcgtgggcggaggctacctgcactgctccttcaagaccacctacagaagcaagaagcccgccaagaacctgaagatgcccggcttccacttcgtggaccaccggctggaacggatcaaagaggccgacaaagaaacctacgtggaacagcacgagatggccgtggccaagtactgcgacctgcctagcaagctgggccacagaaaaaggccggcggccacgaaaaaggccggccaggcaaaaaagaaaaagtgaggtctctctaggaagttcctattccgaagttcctattcttataggagtataggaacttctctagacctgatcataatcaagccatatcacatctgtagaggtttacttgctttaaaaaacctccacacctccccctgaacctgaaacataaaatgaatgcaattgttgttgttaacttgtttattgcagcttataatggttacaaataaagcaatagcatcacaaatttcacaaataaagcatttttttcactgcattctagttgtggtttgtccaaactcatcaatgtatcttatcatgtctggatctgcggatcaggattggtgacagaaaagccccatccttaggcctcctccttcctagtctcctgatattgggtctaacccccacctcctgttaggcagattccttatctggtgacacacccccatttcctggagccatctctctccttgccagaacctctaaggtttgcttacgatggagccagagaggatcctgggagggagagcttggcagggggtgggagggaagggggggatgcgtgacctgcccggttctcagtggccaccctgcgctaccctctcccagaacctgagctgctctgacgcggctgtctggtgcgtttcactgatcctggtgctgcagcttccttacacttcccaagaggagaagcagtttggaaaaacaaaatcagaataagttggtcctgagttctaactttggctcttcacctttctagtccccaatttatattgttcctccgtgcgtcagttttacctgtgagataaggccagtagccagccccgtcctggcagggctgtggtgaggaggggggtgtccgtgtggaaaactccctttgtgagaatggtgcgtcctcgagctgggcctcatgggccttccgctcactgcccgctttccagtcgggaaacctgtcgtgccagctgcattaacatggtcatagctgtttccttgcgtattgggcgctctccgcttcctcgctcactgactcgctgcgctcggtcgttcgggtaaagcctggggtgcctaatgagcaaaaggccagcaaaaggccaggaaccgtaaaaaggccgcgttgctggcgtttttccataggctccgcccccctgacgagcatcacaaaaatcgacgctcaagtcagaggtggcgaaacccgacaggactataaagataccaggcgtttccccctggaagctccctcgtgcgctctcctgttccgaccctgccgcttaccggatacctgtccgcctttctcccttcgggaagcgtggcgctttctcatagctcacgctgtaggtatctcagttcggtgtaggtcgttcgctccaagctgggctgtgtgcacgaaccccccgttcagcccgaccgctgcgccttatccggtaactatcgtcttgagtccaacccggtaagacacgacttatcgccactggcagcagccactggtaacaggattagcagagcgaggtatgtaggcggtgctacagagttcttgaagtggtggcctaactacggctacactagaagaacagtatttggtatctgcgctctgctgaagccagttaccttcggaaaaagagttggtagctcttgatccggcaaacaaaccaccgctggtagcggtggtttttttgtttgcaagcagcagattacgcgcagaaaaaaaggatctcaagaagatcctttgatcttttctacggggtctgacgctcagtggaacgaaaactcacgttaagggattttggtcatgagattatcaaaaaggatcttcacctagatccttttaaattaaaaatgaagttttaaatcaatctaaagtatatatgagtaaacttggtctgacagttaccaatgcttaatcagtgaggcacctatctcagcgatctgtctatttcgttcatccatagttgcctgactccccgtcgtgtagataactacgatacgggagggcttaccatctggccccagtgctgcaatgataccgcgagaaccacgctcaccggctccagatttatcagcaataaaccagccagccggaagggccgagcgcagaagtggtcctgcaactttatccgcctccatccagtctattaattgttgccgggaagctagagtaagtagttcgccagttaatagtttgcgcaacgttgttgccattgctacaggcatcgtggtgtcacgctcgtcgtttggtatggcttcattcagctccggttcccaacgatcaaggcgagttacatgatcccccatgttgtgcaaaaaagcggttagctccttcggtcctccgatcgttgtcagaagtaagttggccgcagtgttatcactcatggttatggcagcactgcataattctcttactgtcatgccatccgtaagatgcttttctgtgactggtgagtactcaaccaagtcattctgagaatagtgtatgcggcgaccgagttgctcttgcccggcgtcaatacgggataataccgcgccacatagcagaactttaaaagtgctcatcattggaaaacgttcttcggggcgaaaactctcaaggatcttaccgctgttgagatccagttcgatgtaacccactcgtgcacccaactgatcttcagcatcttttactttcaccagcgtttctgggtgagcaaaaacaggaaggcaaaatgccgcaaaaaagggaataagggcgacacggaaatgttgaatactcatactcttcctttttcaatattattgaagcatttatcagggttattgtctcatgagcggatacatatttgaatgtatttagaaaaataaacaaataggggttccgcgcacatttccccgaaaagtgccac

SEQ ID NO: 25 - DNA, 6131 bp, Artificial Sequence
  AAVS_Efla-intron_FRT_BFPnls_F3 vector V4.B.3
ctaaattgtaagcgttaatattttgttaaaattcgcgttaaatttttgttaaatcagctcattttttaaccaataggccgaaatcggcaaaatcccttataaatcaaaagaatagaccgagatagggttgagtggccgctacagggcgctcccattcgccattcaggctgcgcaactgttgggaagggcgtttcggtgcgggcctcttcgctattacgccagctggcgaaagggggatgtgctgcaaggcgattaagttgggtaacgccagggttttcccagtcacgacgttgtaaaacgacggccagtgagcgcgacgtaatacgactcactatagggcgaattggcggaaggccgtcaaggccgcatgaattgagctctactggcttctgcgccgcctctggcccactgtttccccttcccaggcaggtcctgctttctctgacctgcattctctcccctgggcctgtgccgctttctgtctgcagcttgtggcctgggtcacctctacggctggcccagatccttccctgccgcctccttcaggttccgtcttcctccactccctcttccccttgctctctgctgtgttgctgcccaaggatgctctttccggagcacttccttctcggcgctgcaccacgtgatgtcctctgagcggatcctccccgtgtctgggtcctctccgggcatctctcctccctcacccaaccccatgccgtcttcactcgctgggttcccttttccttctccttctggggcctgtgccatctctcgtttcttaggatggccttctccgacggatgtctcccttgcgtcccgcctccccttcttgtaggcctgcatcatcaccgtttttctggacaaccccaaagtaccccgtctccctggctttagccacctctccatcctcttgctttctttgcctggacaccccgttctcctgtggattcgggtcacctctcactcctttcatttgggcagctcccctaccccccttacctctctagtctgtgctagctcttccagccccctgtcatggcatcttccaggggtccgagagctcagctagtcttcttcctccaacccgggcccctatgtccacttcaggacagcatgtttgctgcctccagggatcctgtgtccccgagctgggaccaccttatattcccagggccggttaatgtggctctggttctgggtacttttatctgtcccctccaccgggtggctccggtgcccgtcagtgggcagagcgcacatcgcccacagtccccgagaagttggggggaggggtcggcaattgaaccggtgcctagagaaggtggcgcggggtaaactgggaaagtgatgtcgtgtactggctccgcctttttcccgagggtgggggagaaccgtatataagtgcagtagtcgccgtgaacgttctttttcgcaacgggtttgccgccagaacacaggtaagtgccgtgtgtggttcccgcgggcctggcctctttacgggttatggcccttgcgtgccttgaattacttccactggctgcagtacgtgattcttgatcccgagcttcgggttggaagtgggtgggagagttcgaggccttgcgcttaaggagccccttcgcctcgtgcttgagttgaggcctggcctgggcgctggggccgccgcgtgcgaatctggtggcaccttcgcgcctgtctcgctgctttcgataagtctctagccatttaaaatttttgatgacctgctgcgacgctttttttctggcaagatagtcttgtaaatgcgggccaagatctgcacactggtatttcggtttttggggccgcgggcggcgacggggcccgtgcgtcccagcgcacatgttcggcgaggcggggcctgcgagcgcggccaccgagaatcggacgggggtagtctcaagctggccggcctgctctggtgcctggcctcgcgccgccgtgtatcgccccgccctgggcggcaaggctggcccggtcggcaccagttgcgtgagcggaaagatggccgcttcccggccctgctgcagggagctcaaaatggaggacgcggcgctcgggagagcgggcgggtgagtcacccacacaaaggaaaagggcctttccgtcctcagccgtcgcttcatgtgactccacggagtaccgggcgccgtccaggcacctcgattagttctcgagcttttggagtacgtcgtctttaggttggggggaggggttttatgcgatggagtttccccacactgagtgggtggagactgaagttaggccagcttggcacttgatgtaattctccttggaatttgccctttttgagtttggatcttggttcattctcaagcctcagacagtggttcaaagtttttttcttccatttcaggtgtcgtgactggtaccggaagttcctattccgaagttcctattctctagaaagtataggaacttcgtaccgagaccatggccccaaagaagaagcggaaggtcggtatccacggagtcccagcagccatgagcgagctgattaaggagaacatgcacatgaagctgtacatggagggcaccgtggacaaccatcacttcaagtgcacatccgagggcgaaggcaagccctacgagggcacccagaccatgagaatcaaggtggtcgagggcggccctctccccttcgccttcgacatcctggctactagcttcctctacggcagcaagaccttcatcaaccacacccagggcatccccgacttcttcaagcagtccttccctgagggcttcacatgggagagagtcaccacatacgaggacgggggcgtgctgaccgctacccaggacaccagcctccaggacggctgcctcatctacaacgtcaagatcagaggggtgaatttcacatccaacggccctgtgatgcagaagaaaacactcggctgggaggccttcaccgagacgctgtaccccgctgacggcggcctggaaggcagaaacgacatggccctgaagctcgtgggcgggagccatctgatcgcaaacatcaagaccacatatagatccaagaaacccgctaagaacctcaagatgcctggcgtctactatgtggactacagactggaaagaatcaaggaggccaacaacgagacatacgtcgagcagcacgaggtggcagtggccagatactgcgacctccctagcaaactggggcacaagcttaataaaaggccggcggccacgaaaaaggccggccaggcaaaaaagaaaaagtaaggtctctctaggaagttcctattccgaagttcctattcttcaaatagtataggaacttctctagacctgatcataatcaagccatatcacatctgtagaggtttacttgctttaaaaaacctccacacctccccctgaacctgaaacataaaatgaatgcaattgttgttgttaacttgtttattgcagcttataatggttacaaataaagcaatagcatcacaaatttcacaaataaagcatttttttcactgcattctagttgtggtttgtccaaactcatcaatgtatcttatcatgtctggatctgcggatcaggattggtgacagaaaagccccatccttaggcctcctccttcctagtctcctgatattgggtctaacccccacctcctgttaggcagattccttatctggtgacacacccccatttcctggagccatctctctccttgccagaacctctaaggtttgcttacgatggagccagagaggatcctgggagggagagcttggcagggggtgggagggaagggggggatgcgtgacctgcccggttctcagtggccaccctgcgctaccctctcccagaacctgagctgctctgacgcggctgtctggtgcgtttcactgatcctggtgctgcagcttccttacacttcccaagaggagaagcagtttggaaaaacaaaatcagaataagttggtcctgagttctaactttggctcttcacctttctagtccccaatttatattgttcctccgtgcgtcagttttacctgtgagataaggccagtagccagccccgtcctggcagggctgtggtgaggaggggggtgtccgtgtggaaaactccctttgtgagaatggtgcgtcctcgagctgggcctcatgggccttccgctcactgcccgctttccagtcgggaaacctgtcgtgccagctgcattaacatggtcatagctgtttccttgcgtattgggcgctctccgcttcctcgctcactgactcgctgcgctcggtcgttcgggtaaagcctggggtgcctaatgagcaaaaggccagcaaaaggccaggaaccgtaaaaaggccgcgttgctggcgtttttccataggctccgcccccctgacgagcatcacaaaaatcgacgctcaagtcagaggtggcgaaacccgacaggactataaagataccaggcgtttccccctggaagctccctcgtgcgctctcctgttccgaccctgccgcttaccggatacctgtccgcctttctcccttcgggaagcgtggcgctttctcatagctcacgctgtaggtatctcagttcggtgtaggtcgttcgctccaagctgggctgtgtgcacgaaccccccgttcagcccgaccgctgcgccttatccggtaactatcgtcttgagtccaacccggtaagacacgacttatcgccactggcagcagccactggtaacaggattagcagagcgaggtatgtaggcggtgctacagagttcttgaagtggtggcctaactacggctacactagaagaacagtatttggtatctgcgctctgctgaagccagttaccttcggaaaaagagttggtagctcttgatccggcaaacaaaccaccgctggtagcggtggtttttttgtttgcaagcagcagattacgcgcagaaaaaaaggatctcaagaagatcctttgatcttttctacggggtctgacgctcagtggaacgaaaactcacgttaagggattttggtcatgagattatcaaaaaggatcttcacctagatccttttaaattaaaaatgaagttttaaatcaatctaaagtatatatgagtaaacttggtctgacagttaccaatgcttaatcagtgaggcacctatctcagcgatctgtctatttcgttcatccatagttgcctgactccccgtcgtgtagataactacgatacgggagggcttaccatctggccccagtgctgcaatgataccgcgagaaccacgctcaccggctccagatttatcagcaataaaccagccagccggaagggccgagcgcagaagtggtcctgcaactttatccgcctccatccagtctattaattgttgccgggaagctagagtaagtagttcgccagttaatagtttgcgcaacgttgttgccattgctacaggcatcgtggtgtcacgctcgtcgtttggtatggcttcattcagctccggttcccaacgatcaaggcgagttacatgatcccccatgttgtgcaaaaaagcggttagctccttcggtcctccgatcgttgtcagaagtaagttggccgcagtgttatcactcatggttatggcagcactgcataattctcttactgtcatgccatccgtaagatgcttttctgtgactggtgagtactcaaccaagtcattctgagaatagtgtatgcggcgaccgagttgctcttgcccggcgtcaatacgggataataccgcgccacatagcagaactttaaaagtgctcatcattggaaaacgttcttcggggcgaaaactctcaaggatcttaccgctgttgagatccagttcgatgtaacccactcgtgcacccaactgatcttcagcatcttttactttcaccagcgtttctgggtgagcaaaaacaggaaggcaaaatgccgcaaaaaagggaataagggcgacacggaaatgttgaatactcatactcttcctttttcaatattattgaagcatttatcagggttattgtctcatgagcggatacatatttgaatgtatttagaaaaataaacaaataggggttccgcgcacatttccccgaaaagtgccac

SEQ ID NO: 26 - DNA, 3602 bp, Artificial Sequence
  pMA_FRT_HLA-A*02:01-6xHis_F3 vector V4.D.2
ctaaattgtaagcgttaatattttgttaaaattcgcgttaaatttttgttaaatcagctcattttttaaccaataggccgaaatcggcaaaatcccttataaatcaaaagaatagaccgagatagggttgagtggccgctacagggcgctcccattcgccattcaggctgcgcaactgttgggaagggcgtttcggtgcgggcctcttcgctattacgccagctggcgaaagggggatgtgctgcaaggcgattaagttgggtaacgccagggttttcccagtcacgacgttgtaaaacgacggccagtgagcgcgacgtaatacgactcactatagggcgaattggcggaaggccgtcaaggccgcatgaattcgctaccgggaagttcctattccgaagttcctattctctagaaagtataggaacttcaggtaccatggccgtcatggcgccccgaaccctcgtcctgctactctcgggggctctggccctgacccagacctgggcgggctctcactccatgaggtatttcttcacatccgtgtctcggccaggacgcggagagccacgcttcatcgcagtgggctacgtggacgacacgcagttcgtgcggttcgacagcgacgccgcgagccagaggatggagccgcgggcgccgtggatagagcaggagggtccggagtattgggacggggagacacggaaagtgaaggcccactcacagactcaccgagtggacctggggaccctgcgcggctactacaaccagagcgaggccggttctcacaccgtccagaggatgtatggctgcgacgtggggtcggactggcgcttcctccgcggataccaccagtacgcctacgacggcaaggattacatcgccctgaaagaggacctgcgctcttggaccgcggcggacatggcagctcagaccaccaagcacaagtgggaggcggcccatgtggcggagcagttgagagcctacctggagggcacgtgcgtggagtggctccgcagatacctggagaacgggaaggagacgctgcagcgcacggacgcccccaaaacgcatatgactcaccacgctgtctctgaccatgaagccaccctgaggtgctgggccctgagcttctaccctgcggagatcacactgacctggcagcgggatggggaggaccagacccaggacacggagctcgtggagaccaggcctgcaggggatggaaccttccagaagtgggcggctgtggtggtgccttctggacaggagcagagatacacctgccatgtgcagcatgagggtttgcccaagcccctcaccctgagatgggagccgtcttcccagcccaccatccccatcgtgggcatcattgctggcctggttctctttggagctgtgatcactggagctgtggtcgctgctgtgatgtggaggaggaagagctcagatagaaaaggagggagctactctcaggctgcaagcagtgacagtgcccagggctctgatgtgtctctcacagcttgtaaagtgcccgggcatcatcaccatcaccactgactatagtcgtctagacgaagttcctattccgaagttcctattcttcaaatagtataggaacttcctcgagctgggcctcatgggccttccgctcactgcccgctttccagtcgggaaacctgtcgtgccagctgcattaacatggtcatagctgtttccttgcgtattgggcgctctccgcttcctcgctcactgactcgctgcgctcggtcgttcgggtaaagcctggggtgcctaatgagcaaaaggccagcaaaaggccaggaaccgtaaaaaggccgcgttgctggcgtttttccataggctccgcccccctgacgagcatcacaaaaatcgacgctcaagtcagaggtggcgaaacccgacaggactataaagataccaggcgtttccccctggaagctccctcgtgcgctctcctgttccgaccctgccgcttaccggatacctgtccgcctttctcccttcgggaagcgtggcgctttctcatagctcacgctgtaggtatctcagttcggtgtaggtcgttcgctccaagctgggctgtgtgcacgaaccccccgttcagcccgaccgctgcgccttatccggtaactatcgtcttgagtccaacccggtaagacacgacttatcgccactggcagcagccactggtaacaggattagcagagcgaggtatgtaggcggtgctacagagttcttgaagtggtggcctaactacggctacactagaagaacagtatttggtatctgcgctctgctgaagccagttaccttcggaaaaagagttggtagctcttgatccggcaaacaaaccaccgctggtagcggtggtttttttgtttgcaagcagcagattacgcgcagaaaaaaaggatctcaagaagatcctttgatcttttctacggggtctgacgctcagtggaacgaaaactcacgttaagggattttggtcatgagattatcaaaaaggatcttcacctagatccttttaaattaaaaatgaagttttaaatcaatctaaagtatatatgagtaaacttggtctgacagttaccaatgcttaatcagtgaggcacctatctcagcgatctgtctatttcgttcatccatagttgcctgactccccgtcgtgtagataactacgatacgggagggcttaccatctggccccagtgctgcaatgataccgcgagaaccacgctcaccggctccagatttatcagcaataaaccagccagccggaagggccgagcgcagaagtggtcctgcaactttatccgcctccatccagtctattaattgttgccgggaagctagagtaagtagttcgccagttaatagtttgcgcaacgttgttgccattgctacaggcatcgtggtgtcacgctcgtcgtttggtatggcttcattcagctccggttcccaacgatcaaggcgagttacatgatcccccatgttgtgcaaaaaagcggttagctccttcggtcctccgatcgttgtcagaagtaagttggccgcagtgttatcactcatggttatggcagcactgcataattctcttactgtcatgccatccgtaagatgcttttctgtgactggtgagtactcaaccaagtcattctgagaatagtgtatgcggcgaccgagttgctcttgcccggcgtcaatacgggataataccgcgccacatagcagaactttaaaagtgctcatcattggaaaacgttcttcggggcgaaaactctcaaggatcttaccgctgttgagatccagttcgatgtaacccactcgtgcacccaactgatcttcagcatcttttactttcaccagcgtttctgggtgagcaaaaacaggaaggcaaaatgccgcaaaaaagggaataagggcgacacggaaatgttgaatactcatactcttcctttttcaatattattgaagcatttatcagggttattgtctcatgagcggatacatatttgaatgtatttagaaaaataaacaaataggggttccgcgcacatttccccgaaaagtgccac

SEQ ID NO: 27 - DNA, 3602 bp, Artificial Sequence
  pMA_F14_HLA-A*02:01-6xHis_F15 vector V4.H.5
ctaaattgtaagcgttaatattttgttaaaattcgcgttaaatttttgttaaatcagctcattttttaaccaataggccgaaatcggcaaaatcccttataaatcaaaagaatagaccgagatagggttgagtggccgctacagggcgctcccattcgccattcaggctgcgcaactgttgggaagggcgtttcggtgcgggcctcttcgctattacgccagctggcgaaagggggatgtgctgcaaggcgattaagttgggtaacgccagggttttcccagtcacgacgttgtaaaacgacggccagtgagcgcgacgtaatacgactcactatagggcgaattggcggaaggccgtcaaggccgcatgaattcgctaccgggaagttcctattccgaagttcctattctatcagaagtataggaacttcaggtaccatggccgtcatggcgccccgaaccctcgtcctgctactctcgggggctctggccctgacccagacctgggcgggctctcactccatgaggtatttcttcacatccgtgtctcggccaggacgcggagagccacgcttcatcgcagtgggctacgtggacgacacgcagttcgtgcggttcgacagcgacgccgcgagccagaggatggagccgcgggcgccgtggatagagcaggagggtccggagtattgggacggggagacacggaaagtgaaggcccactcacagactcaccgagtggacctggggaccctgcgcggctactacaaccagagcgaggccggttctcacaccgtccagaggatgtatggctgcgacgtggggtcggactggcgcttcctccgcggataccaccagtacgcctacgacggcaaggattacatcgccctgaaagaggacctgcgctcttggaccgcggcggacatggcagctcagaccaccaagcacaagtgggaggcggcccatgtggcggagcagttgagagcctacctggagggcacgtgcgtggagtggctccgcagatacctggagaacgggaaggagacgctgcagcgcacggacgcccccaaaacgcatatgactcaccacgctgtctctgaccatgaagccaccctgaggtgctgggccctgagcttctaccctgcggagatcacactgacctggcagcgggatggggaggaccagacccaggacacggagctcgtggagaccaggcctgcaggggatggaaccttccagaagtgggcggctgtggtggtgccttctggacaggagcagagatacacctgccatgtgcagcatgagggtttgcccaagcccctcaccctgagatgggagccgtcttcccagcccaccatccccatcgtgggcatcattgctggcctggttctctttggagctgtgatcactggagctgtggtcgctgctgtgatgtggaggaggaagagctcagatagaaaaggagggagctactctcaggctgcaagcagtgacagtgcccagggctctgatgtgtctctcacagcttgtaaagtgcccgggcatcatcaccatcaccactgactatagtcgtctagacgaagttcctattccgaagttcctattcttataggagtataggaacttcctcgagctgggcctcatgggccttccgctcactgcccgctttccagtcgggaaacctgtcgtgccagctgcattaacatggtcatagctgtttccttgcgtattgggcgctctccgcttcctcgctcactgactcgctgcgctcggtcgttcgggtaaagcctggggtgcctaatgagcaaaaggccagcaaaaggccaggaaccgtaaaaaggccgcgttgctggcgtttttccataggctccgcccccctgacgagcatcacaaaaatcgacgctcaagtcagaggtggcgaaacccgacaggactataaagataccaggcgtttccccctggaagctccctcgtgcgctctcctgttccgaccctgccgcttaccggatacctgtccgcctttctcccttcgggaagcgtggcgctttctcatagctcacgctgtaggtatctcagttcggtgtaggtcgttcgctccaagctgggctgtgtgcacgaaccccccgttcagcccgaccgctgcgccttatccggtaactatcgtcttgagtccaacccggtaagacacgacttatcgccactggcagcagccactggtaacaggattagcagagcgaggtatgtaggcggtgctacagagttcttgaagtggtggcctaactacggctacactagaagaacagtatttggtatctgcgctctgctgaagccagttaccttcggaaaaagagttggtagctcttgatccggcaaacaaaccaccgctggtagcggtggtttttttgtttgcaagcagcagattacgcgcagaaaaaaaggatctcaagaagatcctttgatcttttctacggggtctgacgctcagtggaacgaaaactcacgttaagggattttggtcatgagattatcaaaaaggatcttcacctagatccttttaaattaaaaatgaagttttaaatcaatctaaagtatatatgagtaaacttggtctgacagttaccaatgcttaatcagtgaggcacctatctcagcgatctgtctatttcgttcatccatagttgcctgactccccgtcgtgtagataactacgatacgggagggcttaccatctggccccagtgctgcaatgataccgcgagaaccacgctcaccggctccagatttatcagcaataaaccagccagccggaagggccgagcgcagaagtggtcctgcaactttatccgcctccatccagtctattaattgttgccgggaagctagagtaagtagttcgccagttaatagtttgcgcaacgttgttgccattgctacaggcatcgtggtgtcacgctcgtcgtttggtatggcttcattcagctccggttcccaacgatcaaggcgagttacatgatcccccatgttgtgcaaaaaagcggttagctccttcggtcctccgatcgttgtcagaagtaagttggccgcagtgttatcactcatggttatggcagcactgcataattctcttactgtcatgccatccgtaagatgcttttctgtgactggtgagtactcaaccaagtcattctgagaatagtgtatgcggcgaccgagttgctcttgcccggcgtcaatacgggataataccgcgccacatagcagaactttaaaagtgctcatcattggaaaacgttcttcggggcgaaaactctcaaggatcttaccgctgttgagatccagttcgatgtaacccactcgtgcacccaactgatcttcagcatcttttactttcaccagcgtttctgggtgagcaaaaacaggaaggcaaaatgccgcaaaaaagggaataagggcgacacggaaatgttgaatactcatactcttcctttttcaatattattgaagcatttatcagggttattgtctcatgagcggatacatatttgaatgtatttagaaaaataaacaaataggggttccgcgcacatttccccgaaaagtgccac

SEQ ID NO: 28 - DNA, 3602 bp, Artificial Sequence
  pMA_F14_HLA-A*24:02-6xHis_F15 vector V4.H.6
ctaaattgtaagcgttaatattttgttaaaattcgcgttaaatttttgttaaatcagctcattttttaaccaataggccgaaatcggcaaaatcccttataaatcaaaagaatagaccgagatagggttgagtggccgctacagggcgctcccattcgccattcaggctgcgcaactgttgggaagggcgtttcggtgcgggcctcttcgctattacgccagctggcgaaagggggatgtgctgcaaggcgattaagttgggtaacgccagggttttcccagtcacgacgttgtaaaacgacggccagtgagcgcgacgtaatacgactcactatagggcgaattggcggaaggccgtcaaggccgcatgaattcgctaccgggaagttcctattccgaagttcctattctatcagaagtataggaacttcaggtaccatggccgtcatggcgccccgaaccctcgtcctgctactctcgggggccctggccctgacccagacctgggcaggctcccactccatgaggtatttctccacatccgtgtctcggccaggacgcggagagccacgcttcatcgccgtgggctacgtggacgacacgcagttcgtgcggttcgacagcgacgccgcgagccagaggatggagccgcgggcgccgtggatagagcaggaggggccggagtattgggacgaggagacagggaaagtgaaggcccactcacagactgaccgagagaacctgcggatcgcgctccgctactacaaccagagcgaggccggttctcacaccctccagatgatgtttggctgcgacgtggggtcggacgggcgcttcctccgcggataccaccagtacgcctacgacggcaaggattacatcgccctgaaagaggacctgcgctcttggaccgcggcggacatggcggctcagatcaccaagcgcaagtgggaggcggcccatgtggcggagcagcagagagcctacctggagggcacgtgcgtggacgggctccgcagatacctggagaacgggaaggagacgctgcagcgcacggacccccccaagacacatatgacccaccaccccatctctgaccatgaggccactctgagatgctgggccctgggcttctaccctgcggagatcacactgacctggcagcgggatggggaggaccagacccaggacacggagcttgtggagaccaggcctgcaggggatggaaccttccagaagtgggcagctgtggtggttccttctggagaggagcagagatacacctgccatgtgcagcatgagggtctgcccaagcccctcaccctgagatgggagccatcttcccagcccaccgtccccatcgtgggcatcattgctggcctggttctccttggagctgtgatcactggagctgtggtcgctgctgtgatgtggaggaggaacagctcagatagaaaaggagggagctactctcaggctgcaagcagtgacagtgcccagggctctgatgtgtctctcacagcttgtaaagtgcccgggcatcatcaccatcaccactgactatagtcgtctagacgaagttcctattccgaagttcctattcttataggagtataggaacttcctcgagctgggcctcatgggccttccgctcactgcccgctttccagtcgggaaacctgtcgtgccagctgcattaacatggtcatagctgtttccttgcgtattgggcgctctccgcttcctcgctcactgactcgctgcgctcggtcgttcgggtaaagcctggggtgcctaatgagcaaaaggccagcaaaaggccaggaaccgtaaaaaggccgcgttgctggcgtttttccataggctccgcccccctgacgagcatcacaaaaatcgacgctcaagtcagaggtggcgaaacccgacaggactataaagataccaggcgtttccccctggaagctccctcgtgcgctctcctgttccgaccctgccgcttaccggatacctgtccgcctttctcccttcgggaagcgtggcgctttctcatagctcacgctgtaggtatctcagttcggtgtaggtcgttcgctccaagctgggctgtgtgcacgaaccccccgttcagcccgaccgctgcgccttatccggtaactatcgtcttgagtccaacccggtaagacacgacttatcgccactggcagcagccactggtaacaggattagcagagcgaggtatgtaggcggtgctacagagttcttgaagtggtggcctaactacggctacactagaagaacagtatttggtatctgcgctctgctgaagccagttaccttcggaaaaagagttggtagctcttgatccggcaaacaaaccaccgctggtagcggtggtttttttgtttgcaagcagcagattacgcgcagaaaaaaaggatctcaagaagatcctttgatcttttctacggggtctgacgctcagtggaacgaaaactcacgttaagggattttggtcatgagattatcaaaaaggatcttcacctagatccttttaaattaaaaatgaagttttaaatcaatctaaagtatatatgagtaaacttggtctgacagttaccaatgcttaatcagtgaggcacctatctcagcgatctgtctatttcgttcatccatagttgcctgactccccgtcgtgtagataactacgatacgggagggcttaccatctggccccagtgctgcaatgataccgcgagaaccacgctcaccggctccagatttatcagcaataaaccagccagccggaagggccgagcgcagaagtggtcctgcaactttatccgcctccatccagtctattaattgttgccgggaagctagagtaagtagttcgccagttaatagtttgcgcaacgttgttgccattgctacaggcatcgtggtgtcacgctcgtcgtttggtatggcttcattcagctccggttcccaacgatcaaggcgagttacatgatcccccatgttgtgcaaaaaagcggttagctccttcggtcctccgatcgttgtcagaagtaagttggccgcagtgttatcactcatggttatggcagcactgcataattctcttactgtcatgccatccgtaagatgcttttctgtgactggtgagtactcaaccaagtcattctgagaatagtgtatgcggcgaccgagttgctcttgcccggcgtcaatacgggataataccgcgccacatagcagaactttaaaagtgctcatcattggaaaacgttcttcggggcgaaaactctcaaggatcttaccgctgttgagatccagttcgatgtaacccactcgtgcacccaactgatcttcagcatcttttactttcaccagcgtttctgggtgagcaaaaacaggaaggcaaaatgccgcaaaaaagggaataagggcgacacggaaatgttgaatactcatactcttcctttttcaatattattgaagcatttatcagggttattgtctcatgagcggatacatatttgaatgtatttagaaaaataaacaaataggggttccgcgcacatttccccgaaaagtgccac

SEQ ID NO: 29 - DNA, 3593 bp, Artificial Sequence
  pMA_F14_HLA-B*07:02-6xHis_F15 vector V4.H.7
ctaaattgtaagcgttaatattttgttaaaattcgcgttaaatttttgttaaatcagctcattttttaaccaataggccgaaatcggcaaaatcccttataaatcaaaagaatagaccgagatagggttgagtggccgctacagggcgctcccattcgccattcaggctgcgcaactgttgggaagggcgtttcggtgcgggcctcttcgctattacgccagctggcgaaagggggatgtgctgcaaggcgattaagttgggtaacgccagggttttcccagtcacgacgttgtaaaacgacggccagtgagcgcgacgtaatacgactcactatagggcgaattggcggaaggccgtcaaggccgcatgaattcgctaccgggaagttcctattccgaagttcctattctatcagaagtataggaacttcaggtaccatgctggtcatggcgccccgaaccgtcctcctgctgctctcggcggccctggccctgaccgagacctgggccggctcccactccatgaggtatttctacacctccgtgtctcggccaggacgcggagagccacgcttcatctcagtgggctacgtggacgacacccagttcgtgaggttcgacagcgacgccgcgagtccgagagaggagccgcgggcgccgtggatagagcaggaggggccggagtattgggaccggaacacacagatctacaaggcccaggcacagactgaccgagagagcctgcggaacctgcgcggctactacaaccagagcgaggccgggtctcacaccctccagagcatgtacggctgcgacgtggggccggacgggcgcctcctccgcgggcatgaccagtacgcctacgacggcaaggattacatcgccctgaacgaggacctgcgctcctggaccgccgcggacacggcggctcagatcacccagcgcaagtgggaggcggcccgtgaggcggagcagcggagagcctacctggagggcgagtgcgtggagtggctccgcagatacctggagaacgggaaggacaaacttgagcgcgcagaccctccaaagacacacgtgacccaccaccccatctctgaccatgaggccaccctgaggtgctgggccctgggtttctaccctgcggagatcacactgacctggcagcgggatggcgaggaccaaactcaggacactgagcttgtggagaccagaccagcaggagatagaaccttccagaagtgggcagctgtggtggtgccttctggagaagagcagagatacacatgccatgtacagcatgaggggctgccgaagcccctcaccctgagatgggagccgtcttcccagtccaccgtccccatcgtgggcattgttgctggcctggctgtcctagcagttgtggtcatcggagctgtggtcgctgctgtgatgtgtaggaggaagagttcaggtggaaaaggagggagctactctcaggctgcgtgcagcgacagtgcccagggctctgatgtgtctctcacagctcccgggcatcatcaccatcaccactgactatagtcgtctagacgaagttcctattccgaagttcctattcttataggagtataggaacttcctcgagctgggcctcatgggccttccgctcactgcccgctttccagtcgggaaacctgtcgtgccagctgcattaacatggtcatagctgtttccttgcgtattgggcgctctccgcttcctcgctcactgactcgctgcgctcggtcgttcgggtaaagcctggggtgcctaatgagcaaaaggccagcaaaaggccaggaaccgtaaaaaggccgcgttgctggcgtttttccataggctccgcccccctgacgagcatcacaaaaatcgacgctcaagtcagaggtggcgaaacccgacaggactataaagataccaggcgtttccccctggaagctccctcgtgcgctctcctgttccgaccctgccgcttaccggatacctgtccgcctttctcccttcgggaagcgtggcgctttctcatagctcacgctgtaggtatctcagttcggtgtaggtcgttcgctccaagctgggctgtgtgcacgaaccccccgttcagcccgaccgctgcgccttatccggtaactatcgtcttgagtccaacccggtaagacacgacttatcgccactggcagcagccactggtaacaggattagcagagcgaggtatgtaggcggtgctacagagttcttgaagtggtggcctaactacggctacactagaagaacagtatttggtatctgcgctctgctgaagccagttaccttcggaaaaagagttggtagctcttgatccggcaaacaaaccaccgctggtagcggtggtttttttgtttgcaagcagcagattacgcgcagaaaaaaaggatctcaagaagatcctttgatcttttctacggggtctgacgctcagtggaacgaaaactcacgttaagggattttggtcatgagattatcaaaaaggatcttcacctagatccttttaaattaaaaatgaagttttaaatcaatctaaagtatatatgagtaaacttggtctgacagttaccaatgcttaatcagtgaggcacctatctcagcgatctgtctatttcgttcatccatagttgcctgactccccgtcgtgtagataactacgatacgggagggcttaccatctggccccagtgctgcaatgataccgcgagaaccacgctcaccggctccagatttatcagcaataaaccagccagccggaagggccgagcgcagaagtggtcctgcaactttatccgcctccatccagtctattaattgttgccgggaagctagagtaagtagttcgccagttaatagtttgcgcaacgttgttgccattgctacaggcatcgtggtgtcacgctcgtcgtttggtatggcttcattcagctccggttcccaacgatcaaggcgagttacatgatcccccatgttgtgcaaaaaagcggttagctccttcggtcctccgatcgttgtcagaagtaagttggccgcagtgttatcactcatggttatggcagcactgcataattctcttactgtcatgccatccgtaagatgcttttctgtgactggtgagtactcaaccaagtcattctgagaatagtgtatgcggcgaccgagttgctcttgcccggcgtcaatacgggataataccgcgccacatagcagaactttaaaagtgctcatcattggaaaacgttcttcggggcgaaaactctcaaggatcttaccgctgttgagatccagttcgatgtaacccactcgtgcacccaactgatcttcagcatcttttactttcaccagcgtttctgggtgagcaaaaacaggaaggcaaaatgccgcaaaaaagggaataagggcgacacggaaatgttgaatactcatactcttcctttttcaatattattgaagcatttatcagggttattgtctcatgagcggatacatatttgaatgtatttagaaaaataaacaaataggggttccgcgcacatttccccgaaaagtgccac

SEQ ID NO: 30 - DNA, 3593 bp, Artificial Sequence
  pMA_F14_HLA-B*35:01-6xHis_F15 vector V4.H.8
ctaaattgtaagcgttaatattttgttaaaattcgcgttaaatttttgttaaatcagctcattttttaaccaataggccgaaatcggcaaaatcccttataaatcaaaagaatagaccgagatagggttgagtggccgctacagggcgctcccattcgccattcaggctgcgcaactgttgggaagggcgtttcggtgcgggcctcttcgctattacgccagctggcgaaagggggatgtgctgcaaggcgattaagttgggtaacgccagggttttcccagtcacgacgttgtaaaacgacggccagtgagcgcgacgtaatacgactcactatagggcgaattggcggaaggccgtcaaggccgcatgaattcgctaccgggaagttcctattccgaagttcctattctatcagaagtataggaacttcaggtaccatgcgggtcacggcgccccgaaccgtcctcctgctgctctggggggcagtggccctgaccgagacctgggccggctcccactccatgaggtatttctacaccgccatgtcccggccaggacgcggagagccacgcttcatcgcagtgggctacgtggacgacacccagttcgtgaggttcgacagcgacgccgcgagtccgaggacggagcctcgggcgccatggatagagcaggaggggccggagtattgggaccggaacacacagatcttcaagaccaacacacagacttaccgagagagcctgcggaacctgcgcggctactacaaccagagcgaggccgggtctcacatcatccagaggatgtatggctgcgacctggggcccgacgggcgcctcctccgcgggcatgaccagtccgcctacgacggcaaggattacatcgccctgaacgaggacctgagctcctggaccgcggcggacaccgcggctcagatcacccagcgcaagtgggaggcggcccgtgtggcggagcagctgagagcctacctggagggcctgtgcgtggagtggctccgcagatacctggagaacgggaaggagactcttcagcgcgcagatcctccaaagacacacgtgacccaccaccccgtctctgaccatgaggccaccctgaggtgctgggccctgggcttctaccctgcggagatcacactgacctggcagcgggatggcgaggaccaaactcaggacactgagcttgtggagaccagaccagcaggagatagaaccttccagaagtgggcagctgtggtggtgccttctggagaagagcagagatacacatgccatgtacagcatgaggggctgccgaagcccctcaccctgagatgggagccatcttcccagtccaccatccccatcgtgggcattgttgctggcctggctgtcctagcagttgtggtcatcggagctgtggtcgctactgtgatgtgtaggaggaagagctcaggtggaaaaggagggagctactctcaggctgcgtccagcgacagtgcccagggctctgatgtgtctctcacagctcccgggcatcatcaccatcaccactgactatagtcgtctagacgaagttcctattccgaagttcctattcttataggagtataggaacttcctcgagctgggcctcatgggccttccgctcactgcccgctttccagtcgggaaacctgtcgtgccagctgcattaacatggtcatagctgtttccttgcgtattgggcgctctccgcttcctcgctcactgactcgctgcgctcggtcgttcgggtaaagcctggggtgcctaatgagcaaaaggccagcaaaaggccaggaaccgtaaaaaggccgcgttgctggcgtttttccataggctccgcccccctgacgagcatcacaaaaatcgacgctcaagtcagaggtggcgaaacccgacaggactataaagataccaggcgtttccccctggaagctccctcgtgcgctctcctgttccgaccctgccgcttaccggatacctgtccgcctttctcccttcgggaagcgtggcgctttctcatagctcacgctgtaggtatctcagttcggtgtaggtcgttcgctccaagctgggctgtgtgcacgaaccccccgttcagcccgaccgctgcgccttatccggtaactatcgtcttgagtccaacccggtaagacacgacttatcgccactggcagcagccactggtaacaggattagcagagcgaggtatgtaggcggtgctacagagttcttgaagtggtggcctaactacggctacactagaagaacagtatttggtatctgcgctctgctgaagccagttaccttcggaaaaagagttggtagctcttgatccggcaaacaaaccaccgctggtagcggtggtttttttgtttgcaagcagcagattacgcgcagaaaaaaaggatctcaagaagatcctttgatcttttctacggggtctgacgctcagtggaacgaaaactcacgttaagggattttggtcatgagattatcaaaaaggatcttcacctagatccttttaaattaaaaatgaagttttaaatcaatctaaagtatatatgagtaaacttggtctgacagttaccaatgcttaatcagtgaggcacctatctcagcgatctgtctatttcgttcatccatagttgcctgactccccgtcgtgtagataactacgatacgggagggcttaccatctggccccagtgctgcaatgataccgcgagaaccacgctcaccggctccagatttatcagcaataaaccagccagccggaagggccgagcgcagaagtggtcctgcaactttatccgcctccatccagtctattaattgttgccgggaagctagagtaagtagttcgccagttaatagtttgcgcaacgttgttgccattgctacaggcatcgtggtgtcacgctcgtcgtttggtatggcttcattcagctccggttcccaacgatcaaggcgagttacatgatcccccatgttgtgcaaaaaagcggttagctccttcggtcctccgatcgttgtcagaagtaagttggccgcagtgttatcactcatggttatggcagcactgcataattctcttactgtcatgccatccgtaagatgcttttctgtgactggtgagtactcaaccaagtcattctgagaatagtgtatgcggcgaccgagttgctcttgcccggcgtcaatacgggataataccgcgccacatagcagaactttaaaagtgctcatcattggaaaacgttcttcggggcgaaaactctcaaggatcttaccgctgttgagatccagttcgatgtaacccactcgtgcacccaactgatcttcagcatcttttactttcaccagcgtttctgggtgagcaaaaacaggaaggcaaaatgccgcaaaaaagggaataagggcgacacggaaatgttgaatactcatactcttcctttttcaatattattgaagcatttatcagggttattgtctcatgagcggatacatatttgaatgtatttagaaaaataaacaaataggggttccgcgcacatttccccgaaaagtgccac

SEQ ID NO: 31 - DNA, 4542 bp, Artificial Sequence
  CMVpro_FLP_Sv40pA_V2 vector V4.1.8
ctaaattgtaagcgttaatattttgttaaaattcgcgttaaatttttgttaaatcagctcattttttaaccaataggccgaaatcggcaaaatcccttataaatcaaaagaatagaccgagatagggttgagtggccgctacagggcgctcccattcgccattcaggctgcgcaactgttgggaagggcgtttcggtgcgggcctcttcgctattacgccagctggcgaaagggggatgtgctgcaaggcgattaagttgggtaacgccagggttttcccagtcacgacgttgtaaaacgacggccagtgagcgcgacgtaatacgactcactatagggcgaattggcggaaggccgtcaaggccgcatgaattcgctaccggtatagtaatcaattacggggtcattagttcatagcccatatatggagttccgcgttacataacttacggtaaatggcccgcctggctgaccgcccaacgacccccgcccattgacgtcaataatgacgtatgttcccatagtaacgccaatagggactttccattgacgtcaatgggtggagtatttacggtaaactgcccacttggcagtacatcaagtgtatcatatgccaagtacgccccctattgacgtcaatgacggtaaatggcccgcctggcattatgcccagtacatgaccttatgggactttcctacttggcagtacatctacgtattagtcatcgctattaccatggtgatgcggttttggcagtacatcaatgggcgtggatagcggtttgactcacggggatttccaagtctccaccccattgacgtcaatgggagtttgttttggcaccaaaatcaacgggactttccaaaatgtcgtaacaactccgccccattgacgcaaatgggcggtaggcgtgtacggtgggaggtctatataagcagagctggtttagtgaaccgtcagatcaggtaccatggcccccaagaaaaagcggaaagtgggcatccacggcgtgccagctgcaggcggctctatgagccagttcgacatcctgtgcaagaccccacctaaggtgctcgtgcggcagttcgtggaaagattcgagaggcctagcggcgagaagatcgcctcttgtgctgccgagctgacctacctgtgctggatgatcacccacaacggcaccgccatcaagcgggccaccttcatgagctacaataccatcatcagcaacagcctgagcttcgacatcgtgaacaagagcctgcagttcaagtacaagacccagaaggccaccatcctggaagccagcctgaagaaactgatccccgcctgggagtttaccatcatcccatacaatggccagaaacatcagagcgacattaccgatatcgtgtccagcctccagctgcagttcgagagtagcgaagaagccgacaagggcaacagccacagcaagaagatgctgaaggccctgctgagcgagggcgagagcatctgggagatcacagagaagatcctgaacagcttcgagtacaccagccggttcaccaagaccaagaccctgtaccagttcctgttcctggccacctttatcaactgcggccggttctccgacatcaagaacgtggaccccaagagcttcaagctggtgcagaacaagtacctgggcgtgatcattcagtgcctcgtgaccgagacaaagaccagcgtgtcccggcacatctactttttcagcgccagaggccggatcgaccccctggtgtacctggacgagttcctgagaaacagcgagcccgtgctgaagagagtgaaccggaccggcaacagcagctccaacaagcaggaataccagctgctgaaggacaacctcgtgcggtcctacaacaaggccctgaagaaaaacgccccctaccccatcttcgccattaagaacggccccaagtcccacatcggccggcacctgatgaccagctttctgagcatgaagggcctgacagagctgaccaacgtcgtgggcaattggagcgacaagagggcctctgccgtggccagaaccacctacacccaccagatcacagccatccccgaccactacttcgccctggtgtctcggtactacgcctacgaccccatcagcaaagagatgatcgccctgaaggacgagacaaaccccatcgaggaatggcagcacatcgagcagctgaagggcagcgccgagggcagcatcagataccctgcctggaacggcatcatctcccaggaagtgctggactacctgagcagctacatcaaccggcggatctgatctagacctgatcataatcaagccatatcacatctgtagaggtttacttgctttaaaaaacctccacacctccccctgaacctgaaacataaaatgaatgcaattgttgttgttaacttgtttattgcagcttataatggttacaaataaagcaatagcatcacaaatttcacaaataaagcatttttttcactgcattctagttgtggtttgtccaaactcatcaatgtatcttatcatgtctggatctgcggatccaatctcgagctgggcctcatgggccttccgctcactgcccgctttccagtcgggaaacctgtcgtgccagctgcattaacatggtcatagctgtttccttgcgtattgggcgctctccgcttcctcgctcactgactcgctgcgctcggtcgttcgggtaaagcctggggtgcctaatgagcaaaaggccagcaaaaggccaggaaccgtaaaaaggccgcgttgctggcgtttttccataggctccgcccccctgacgagcatcacaaaaatcgacgctcaagtcagaggtggcgaaacccgacaggactataaagataccaggcgtttccccctggaagctccctcgtgcgctctcctgttccgaccctgccgcttaccggatacctgtccgcctttctcccttcgggaagcgtggcgctttctcatagctcacgctgtaggtatctcagttcggtgtaggtcgttcgctccaagctgggctgtgtgcacgaaccccccgttcagcccgaccgctgcgccttatccggtaactatcgtcttgagtccaacccggtaagacacgacttatcgccactggcagcagccactggtaacaggattagcagagcgaggtatgtaggcggtgctacagagttcttgaagtggtggcctaactacggctacactagaagaacagtatttggtatctgcgctctgctgaagccagttaccttcggaaaaagagttggtagctcttgatccggcaaacaaaccaccgctggtagcggtggtttttttgtttgcaagcagcagattacgcgcagaaaaaaaggatctcaagaagatcctttgatcttttctacggggtctgacgctcagtggaacgaaaactcacgttaagggattttggtcatgagattatcaaaaaggatcttcacctagatccttttaaattaaaaatgaagttttaaatcaatctaaagtatatatgagtaaacttggtctgacagttaccaatgcttaatcagtgaggcacctatctcagcgatctgtctatttcgttcatccatagttgcctgactccccgtcgtgtagataactacgatacgggagggcttaccatctggccccagtgctgcaatgataccgcgagaaccacgctcaccggctccagatttatcagcaataaaccagccagccggaagggccgagcgcagaagtggtcctgcaactttatccgcctccatccagtctattaattgttgccgggaagctagagtaagtagttcgccagttaatagtttgcgcaacgttgttgccattgctacaggcatcgtggtgtcacgctcgtcgtttggtatggcttcattcagctccggttcccaacgatcaaggcgagttacatgatcccccatgttgtgcaaaaaagcggttagctccttcggtcctccgatcgttgtcagaagtaagttggccgcagtgttatcactcatggttatggcagcactgcataattctcttactgtcatgccatccgtaagatgcttttctgtgactggtgagtactcaaccaagtcattctgagaatagtgtatgcggcgaccgagttgctcttgcccggcgtcaatacgggataataccgcgccacatagcagaactttaaaagtgctcatcattggaaaacgttcttcggggcgaaaactctcaaggatcttaccgctgttgagatccagttcgatgtaacccactcgtgcacccaactgatcttcagcatcttttactttcaccagcgtttctgggtgagcaaaaacaggaaggcaaaatgccgcaaaaaagggaataagggcgacacggaaatgttgaatactcatactcttcctttttcaatattattgaagcatttatcagggttattgtctcatgagcggatacatatttgaatgtatttagaaaaataaacaaataggggttccgcgcacatttccccgaaaagtgccac

SEQ ID NO: 32 - DNA, 3172 bp, Artificial Sequence
  FRT_HCMVpp28-3xMYC_F3 vector V9.E.6
ggcggttcctctacatccggtggatctggatctggagaacaaaagctcatctctgaggaggaccttggggagcagaagctaatcagtgaagaagacctcggagagcagaaattgattagcgaggaggatctttaaagactaggcacgaagttcctattccgaagttcctattcttcaaatagtataggaacttccgctctgaccagctgcattaacatggtcatagctgtttccttgcgtattgggcgctctccgcttcctcgctcactgactcgctgcgctcggtcgttcgggtaaagcctggggtgcctaatgagcaaaaggccagcaaaaggccaggaaccgtaaaaaggccgcgttgctggcgtttttccataggctccgcccccctgacgagcatcacaaaaatcgacgctcaagtcagaggtggcgaaacccgacaggactataaagataccaggcgtttccccctggaagctccctcgtgcgctctcctgttccgaccctgccgcttaccggatacctgtccgcctttctcccttcgggaagcgtggcgctttctcatagctcacgctgtaggtatctcagttcggtgtaggtcgttcgctccaagctgggctgtgtgcacgaaccccccgttcagcccgaccgctgcgccttatccggtaactatcgtcttgagtccaacccggtaagacacgacttatcgccactggcagcagccactggtaacaggattagcagagcgaggtatgtaggcggtgctacagagttcttgaagtggtggcctaactacggctacactagaagaacagtatttggtatctgcgctctgctgaagccagttaccttcggaaaaagagttggtagctcttgatccggcaaacaaaccaccgctggtagcggtggtttttttgtttgcaagcagcagattacgcgcagaaaaaaaggatctcaagaagatcctttgatcttttctacggggtctgacgctcagtggaacgaaaactcacgttaagggattttggtcatgagattatcaaaaaggatcttcacctagatccttttaaattaaaaatgaagttttaaatcaatctaaagtatatatgagtaaacttggtctgacagttaccaatgcttaatcagtgaggcacctatctcagcgatctgtctatttcgttcatccatagttgcctgactccccgtcgtgtagataactacgatacgggagggcttaccatctggccccagtgctgcaatgataccgcgagaaccacgctcaccggctccagatttatcagcaataaaccagccagccggaagggccgagcgcagaagtggtcctgcaactttatccgcctccatccagtctattaattgttgccgggaagctagagtaagtagttcgccagttaatagtttgcgcaacgttgttgccattgctacaggcatcgtggtgtcacgctcgtcgtttggtatggcttcattcagctccggttcccaacgatcaaggcgagttacatgatcccccatgttgtgcaaaaaagcggttagctccttcggtcctccgatcgttgtcagaagtaagttggccgcagtgttatcactcatggttatggcagcactgcataattctcttactgtcatgccatccgtaagatgcttttctgtgactggtgagtactcaaccaagtcattctgagaatagtgtatgcggcgaccgagttgctcttgcccggcgtcaatacgggataataccgcgccacatagcagaactttaaaagtgctcatcattggaaaacgttcttcggggcgaaaactctcaaggatcttaccgctgttgagatccagttcgatgtaacccactcgtgcacccaactgatcttcagcatcttttactttcaccagcgtttctgggtgagcaaaaacaggaaggcaaaatgccgcaaaaaagggaataagggcgacacggaaatgttgaatactcatactcttcctttttcaatattattgaagcatttatcagggttattgtctcatgagcggatacatatttgaatgtatttagaaaaataaacaaataggggttccgcgcacatttccccgaaaagtgccacctaaattgtaagcgttaatattttgttaaaattcgcgttaaatttttgttaaatcagctcattttttaaccaataggccgaaatcggcaaaatcccttataaatcaaaagaatagaccgagatagggttgagtggccgctacagggcgctcccattcgccattcaggctgcgcaactgttgggaagggcgtttcggtgcgggcctcttcgctattacgccagctggcgaaagggggatgtgctgcaaggcgattaagttgggtaacgccagggttttcccagtcacgacgttgtaaaacgacggccagtgagcgcgacgtaatacgactcactatagggcgaattggcggaaggccgtcaaggccgcatgaattcgctaccgggagttggtaggtaagtatcaaggttacaagacaggtttaaggaggaagttcctattccgaagttcctattctctagaaagtataggaacttcgactctcaccatgggtgccgaactctgcaaacgaatatgttgtgagttcggtaccacgtccggtgagcccctgaaagatgctctgggtcgccaggtgtctctacgctcctacgacaacatccctccgacttcctcctcggacgaaggggaggacgatgacgacggggaggatgacgataacgaggagcggcaacagaagctgcggctctgcggtagtggctgcggaggaaacgacagtagcagtggcagccaccgagaggccacccacgacggccctaagaagaacgctgtgcgctcgacgtttcgcgaggacaaggctccgaaaccgagcaagcagtccaagaagaaaaagaaaccctcaaagcatcaccaccatcagcaaagctccattatgcaggagacggacgacttagacgaagaggacacctcaatttacctgtcccctccccctgttccaccagttcaggtggtggctaagcgactgccgcgtcccgacacacccaggactccgcgccagaagaagatttcacaacgtccacccacacccgggaccaaaaagcccgctgcctccttgcccttt

SEQ ID NO: 33 - DNA, 3900 bp, Artificial Sequence
  FRT_HCMVpp52-3xMYC_F3 vector V9.E.7
ggcggttcctctacatccggtggatctggatctggagaacaaaagctcatctctgaggaggaccttggggagcagaagctaatcagtgaagaagacctcggagagcagaaattgattagcgaggaggatctttaaagactaggcacgaagttcctattccgaagttcctattcttcaaatagtataggaacttccgctctgaccagctgcattaacatggtcatagctgtttccttgcgtattgggcgctctccgcttcctcgctcactgactcgctgcgctcggtcgttcgggtaaagcctggggtgcctaatgagcaaaaggccagcaaaaggccaggaaccgtaaaaaggccgcgttgctggcgtttttccataggctccgcccccctgacgagcatcacaaaaatcgacgctcaagtcagaggtggcgaaacccgacaggactataaagataccaggcgtttccccctggaagctccctcgtgcgctctcctgttccgaccctgccgcttaccggatacctgtccgcctttctcccttcgggaagcgtggcgctttctcatagctcacgctgtaggtatctcagttcggtgtaggtcgttcgctccaagctgggctgtgtgcacgaaccccccgttcagcccgaccgctgcgccttatccggtaactatcgtcttgagtccaacccggtaagacacgacttatcgccactggcagcagccactggtaacaggattagcagagcgaggtatgtaggcggtgctacagagttcttgaagtggtggcctaactacggctacactagaagaacagtatttggtatctgcgctctgctgaagccagttaccttcggaaaaagagttggtagctcttgatccggcaaacaaaccaccgctggtagcggtggtttttttgtttgcaagcagcagattacgcgcagaaaaaaaggatctcaagaagatcctttgatcttttctacggggtctgacgctcagtggaacgaaaactcacgttaagggattttggtcatgagattatcaaaaaggatcttcacctagatccttttaaattaaaaatgaagttttaaatcaatctaaagtatatatgagtaaacttggtctgacagttaccaatgcttaatcagtgaggcacctatctcagcgatctgtctatttcgttcatccatagttgcctgactccccgtcgtgtagataactacgatacgggagggcttaccatctggccccagtgctgcaatgataccgcgagaaccacgctcaccggctccagatttatcagcaataaaccagccagccggaagggccgagcgcagaagtggtcctgcaactttatccgcctccatccagtctattaattgttgccgggaagctagagtaagtagttcgccagttaatagtttgcgcaacgttgttgccattgctacaggcatcgtggtgtcacgctcgtcgtttggtatggcttcattcagctccggttcccaacgatcaaggcgagttacatgatcccccatgttgtgcaaaaaagcggttagctccttcggtcctccgatcgttgtcagaagtaagttggccgcagtgttatcactcatggttatggcagcactgcataattctcttactgtcatgccatccgtaagatgcttttctgtgactggtgagtactcaaccaagtcattctgagaatagtgtatgcggcgaccgagttgctcttgcccggcgtcaatacgggataataccgcgccacatagcagaactttaaaagtgctcatcattggaaaacgttcttcggggcgaaaactctcaaggatcttaccgctgttgagatccagttcgatgtaacccactcgtgcacccaactgatcttcagcatcttttactttcaccagcgtttctgggtgagcaaaaacaggaaggcaaaatgccgcaaaaaagggaataagggcgacacggaaatgttgaatactcatactcttcctttttcaatattattgaagcatttatcagggttattgtctcatgagcggatacatatttgaatgtatttagaaaaataaacaaataggggttccgcgcacatttccccgaaaagtgccacctaaattgtaagcgttaatattttgttaaaattcgcgttaaatttttgttaaatcagctcattttttaaccaataggccgaaatcggcaaaatcccttataaatcaaaagaatagaccgagatagggttgagtggccgctacagggcgctcccattcgccattcaggctgcgcaactgttgggaagggcgtttcggtgcgggcctcttcgctattacgccagctggcgaaagggggatgtgctgcaaggcgattaagttgggtaacgccagggttttcccagtcacgacgttgtaaaacgacggccagtgagcgcgacgtaatacgactcactatagggcgaattggcggaaggccgtcaaggccgcatgaattcgctaccgggagttggtaggtaagtatcaaggttacaagacaggtttaaggaggaagttcctattccgaagttcctattctctagaaagtataggaacttcgactctaccaccatggatcgcaagacgcgcctctcggagccgccgacgctggcgctgcggctgaagccgtacaagacggctatccagcagctgcgatctgtgatccgtgcgctcaaggagaacaccacggttaccttcttgcccacaccgtcgcttatcttgcaaacggtacgcagtcactgcgtgtcaaagatcacttttaacagctcatgcctctacatcactgacaagtcgtttcagcccaagaccattaacaattccacgcctctgctgggtaacttcatgtacctgacttccagcaaggacctgaccaagttctacgtgcaggacatctcggacctgtcggccaagatctccatgtgcgcacccgatttcaatatggagttcagctcggcctgcgtgcacggccaagacattgtgcgcgaaagcgagaattcggccgtgcacgtggatctagatttcggcgtggtggccgacctgcttaagtggatcgggccgcatacccgcgtcaagcgtaacgtgaagaaagcgccctgccctacgggcaccgtgcagattctggtgcacgccggtccaccggccatcaagttcatcctgaccaacggcagcgagctggaattcacagccaataaccgcgtcagtttccacggcgtgaaaaacatgcgtatcaacgtgcagctgaagaacttctaccagacgctgctcaattgcgccgtcaccaaactgccgtgcacgttgcgtatagttacggagcacgacacgctgttgtacgtggccagccgcaacggtctgttcgccgtggagaattttctcaccgaggaacctttccagcgtggcgatcccttcgacaagaattacgtcgggaacagcggcaaatcgcgtggcggaggcggtggtagcggcagcctctcttcgctggctaatgccggcggtctgcacgacgacggtccgggtctggacaacgatatcatgaacgagcccatgggtctcggcggactgggaggtggcggaggagggggaggcaagaagcacgaccgcggaggtggcggtggttccggtacgcggaaaatgagcagcggtggcggaggtggagatcacgaccacggtctttcctccaaggaaaaatacgagcagcacaagatcaccagctacctgacgtccaaaggtggatcgggaggagggggtggaggcggaggtggaggtttggatcgcaactccggcaattacttcaacgacgcgaaagaggagagcgacagcgaggattctgtaacgttcgagttcgtccctaacaccaagaagcaaaagtgc

SEQ ID NO: 34 - DNA, 4286 bp, Artificial Sequence
  FRT_HCMVpp52-3xMYC_F3 vector V9.E.8
ggcggttcctctacatccggtggatctggatctggagaacaaaagctcatctctgaggaggaccttggggagcagaagctaatcagtgaagaagacctcggagagcagaaattgattagcgaggaggatctttaaagactaggcacgaagttcctattccgaagttcctattcttcaaatagtataggaacttccgctctgaccagctgcattaacatggtcatagctgtttccttgcgtattgggcgctctccgcttcctcgctcactgactcgctgcgctcggtcgttcgggtaaagcctggggtgcctaatgagcaaaaggccagcaaaaggccaggaaccgtaaaaaggccgcgttgctggcgtttttccataggctccgcccccctgacgagcatcacaaaaatcgacgctcaagtcagaggtggcgaaacccgacaggactataaagataccaggcgtttccccctggaagctccctcgtgcgctctcctgttccgaccctgccgcttaccggatacctgtccgcctttctcccttcgggaagcgtggcgctttctcatagctcacgctgtaggtatctcagttcggtgtaggtcgttcgctccaagctgggctgtgtgcacgaaccccccgttcagcccgaccgctgcgccttatccggtaactatcgtcttgagtccaacccggtaagacacgacttatcgccactggcagcagccactggtaacaggattagcagagcgaggtatgtaggcggtgctacagagttcttgaagtggtggcctaactacggctacactagaagaacagtatttggtatctgcgctctgctgaagccagttaccttcggaaaaagagttggtagctcttgatccggcaaacaaaccaccgctggtagcggtggtttttttgtttgcaagcagcagattacgcgcagaaaaaaaggatctcaagaagatcctttgatcttttctacggggtctgacgctcagtggaacgaaaactcacgttaagggattttggtcatgagattatcaaaaaggatcttcacctagatccttttaaattaaaaatgaagttttaaatcaatctaaagtatatatgagtaaacttggtctgacagttaccaatgcttaatcagtgaggcacctatctcagcgatctgtctatttcgttcatccatagttgcctgactccccgtcgtgtagataactacgatacgggagggcttaccatctggccccagtgctgcaatgataccgcgagaaccacgctcaccggctccagatttatcagcaataaaccagccagccggaagggccgagcgcagaagtggtcctgcaactttatccgcctccatccagtctattaattgttgccgggaagctagagtaagtagttcgccagttaatagtttgcgcaacgttgttgccattgctacaggcatcgtggtgtcacgctcgtcgtttggtatggcttcattcagctccggttcccaacgatcaaggcgagttacatgatcccccatgttgtgcaaaaaagcggttagctccttcggtcctccgatcgttgtcagaagtaagttggccgcagtgttatcactcatggttatggcagcactgcataattctcttactgtcatgccatccgtaagatgcttttctgtgactggtgagtactcaaccaagtcattctgagaatagtgtatgcggcgaccgagttgctcttgcccggcgtcaatacgggataataccgcgccacatagcagaactttaaaagtgctcatcattggaaaacgttcttcggggcgaaaactctcaaggatcttaccgctgttgagatccagttcgatgtaacccactcgtgcacccaactgatcttcagcatcttttactttcaccagcgtttctgggtgagcaaaaacaggaaggcaaaatgccgcaaaaaagggaataagggcgacacggaaatgttgaatactcatactcttcctttttcaatattattgaagcatttatcagggttattgtctcatgagcggatacatatttgaatgtatttagaaaaataaacaaataggggttccgcgcacatttccccgaaaagtgccacctaaattgtaagcgttaatattttgttaaaattcgcgttaaatttttgttaaatcagctcattttttaaccaataggccgaaatcggcaaaatcccttataaatcaaaagaatagaccgagatagggttgagtggccgctacagggcgctcccattcgccattcaggctgcgcaactgttgggaagggcgtttcggtgcgggcctcttcgctattacgccagctggcgaaagggggatgtgctgcaaggcgattaagttgggtaacgccagggttttcccagtcacgacgttgtaaaacgacggccagtgagcgcgacgtaatacgactcactatagggcgaattggcggaaggccgtcaaggccgcatgaattcgctaccgggagttggtaggtaagtatcaaggttacaagacaggtttaaggaggaagttcctattccgaagttcctattctctagaaagtataggaacttcgactctcaggtaccatggagtcgcgcggtcgccgttgtcccgaaatgatatccgtactgggtcccatttcggggcacgtgctgaaagccgtgtttagtcgcggcgatacgccggtgctgccgcacgagacgcgactcctgcagacgggtatccacgtacgcgtgagccagccctcgctgatcttggtatcgcagtacacgcccgactcgacgccatgccaccgcggcgacaatcagctgcaggtgcagcacacgtactttacgggcagcgaggtggagaacgtgtcggtcaacgtgcacaaccccacgggccgaagcatctgccccagccaggagcccatgtcgatctatgtgtacgcgctgccgctcaagatgctgaacatccccagcatcaacgtgcaccactacccgtcggcggccgagcgcaaacaccgacacctgcccgtagctgacgctgtgattcacgcgtcgggcaagcagatgtggcaggcgcgtctcacggtctcgggactggcctggacgcgtcagcagaaccagtggaaagagcccgacgtctactacacgtcagcgttcgtgtttcccaccaaggacgtggcactgcggcacgtggtgtgcgcgcacgagctggtttgctccatggagaacacgcgcgcaaccaagatgcaggtgataggtgaccagtacgtcaaggtgtacctggagtccttctgcgaggacgtgccctccggcaagctctttatgcacgtcacgctgggctctgacgtggaagaggacctgacgatgacccgcaacccgcaacccttcatgcgcccccacgagcgcaacggctttacggtgttgtgtcccaaaaatatgataatcaaaccgggcaagatctcgcacatcatgctggatgtggcttttacctcacacgagcattttgggctgctgtgtcccaagagcatcccgggcctgagcatctcaggtaacctgttgatgaacgggcagcagatcttcctggaggtacaagccatacgcgagaccgtggaactgcgtcagtacgatcccgtggctgcgctcttctttttcgatatcgacttgctgctgcagcgcgggcctcagtacagcgagcaccccaccttcaccagccagtatcgcatccagggcaagcttgagtaccgacacacctgggaccggcacgacgagggtgccgcccagggcgacgacgacgtctggaccagcggatcggactccgacgaagaactcgtaaccaccgagcgcaagacgccccgcgtcaccggcggcggcgccatggcgggcgcctccacttccgcgggccgcaaacgcaaatcagcatcctcggcgacggcgtgcacgtcgggcgttatgacacgcggccgccttaaggccgagtccaccgtcgcgcccgaagaggacaccgacgaggattccgacaacgaaatccacaatccggccgtgttcacctggccgccctggcaggccggcatcctggcccgcaacctggtgcccatggtggctacggttcagggtcagaatctgaagtaccaggagttcttctgggacgccaacgacatctaccgcatcttcgccgaattggaaggcgtatggcagcccgctgcgcaacccaaacgtcgccgccaccggcaagacgccttgcccgggccatgcatcgcctcgacgcccaaaaagcaccga

SEQ ID NO: 35 - DNA, 25 bp, Homo sapiens
  pMA-sv40_OE_F1 primer 1.C.2
cctgatcataatcaagccatatcac

SEQ ID NO: 36 - DNA, 25 bp, Homo sapiens
  pMA-sv40_OE_R1 primer 1.C.3
gtgatatggcttgattatgatcagg

SEQ ID NO: 37 - DNA, 20 bp, Homo sapiens
  HLA-A-GT-Rg3 primer 4.A.3 1
tcccgttctccaggtatctg

SEQ ID NO: 38 - DNA, 20 bp, Homo sapiens
  HLA-A-GT-Fg2 primer 4.A.4
gtgtcgggtttccagagaag

SEQ ID NO: 39 - DNA, 20 bp, Homo sapiens
  HLA-B-GT-Fg2 primer 4.A.7
gggtcccagttctaaagtcc

SEQ ID NO: 40 - DNA, 20 bp, Homo sapiens
  HLA-B-GT-Rg2 primer 4.B.1
ggggattttggcctcaactg

SEQ ID NO: 41 - DNA, 21 bp, Homo sapiens
  HLA-C-GT-Fg2 primer 4.B.5
tcttcctgaatactcatgacg

SEQ ID NO: 42 - DNA, 20 bp, Homo sapiens
  HLA-A-02_GT_Rg4 primer 4.I.9
ggagatctacaggcgatcag

SEQ ID NO: 43 - DNA, 28 bp, Homo sapiens
  HLA-A-Exon3_HA-RE-BglII_F1 primer 6.I.9
ggttagatctgggaaggagacgctgcag

SEQ ID NO: 44 - DNA, 20 bp, Homo sapiens
  HLA-C-04-GT-Rg1 primer 8.A.1
gatcccattttcctcccctc

SEQ ID NO: 45 - DNA, 27 bp, Homo sapiens
  CMV-pA-HLA-Ex3_Probe_F1 primer 8.B.2
atgtctggatctgcggatcagcgcacg

SEQ ID NO: 46 - DNA, 21 bp, Homo sapiens
  CMV-pro_GT_R1 primer 9.C.3
atgggctatgaactaatgacc

SEQ ID NO: 47 - DNA, 21 bp, Homo sapiens
  sv40pA_GT_F1 primer 9.C.4
cattctagttgtggtttgtcc

SEQ ID NO: 48 - DNA, 20 bp, Homo sapiens
  AAVS1_GT_F1 primer 9.C.5
cttacctctctagtctgtgc

SEQ ID NO: 49 - DNA, 19 bp, Homo sapiens
  AAVS1_GT_F3 primer 9.C.7
ccattgtcactttgcgctg

SEQ ID NO: 50 - DNA, 20 bp, Homo sapiens
  AAVS1_GT_F4 primer 9.C.8
tcctggactttgtctccttc

SEQ ID NO: 51 - DNA, 20 bp, Homo sapiens
  AAVS1_GT_R2 primer 9.C.10
agagatggctccaggaaatg

SEQ ID NO: 52 - DNA, 20 bp, Homo sapiens
  AAVS1_GT_R3 primer 9.D.1
aagagaaagggagtagaggc

SEQ ID NO: 53 - DNA, 18 bp, Homo sapiens
  AAVS1_GT_R4 primer 9.D.2
cccgaagagtgagtttgc

SEQ ID NO: 54 - DNA, 20 bp, Homo sapiens
  HLA-A-intron4_GT_R1 primer 9.D.6
gctaaaggtcagagaggctc

SEQ ID NO: 55 - DNA, 23 bp, Homo sapiens
  sv40pA-GT primer 9.D.7
ctgcattctagttgtggtttgtc

SEQ ID NO: 56 - DNA, 24 bp, Homo sapiens
  sv40pA-AAVS1-probe-FAM-F1 primer 9.J.2
tgcggatcaggattggtgacagaa

SEQ ID NO: 57 - DNA, 26 bp, Homo sapiens
  TRAC_TCRA-ex1_R1 primer 10.A.9
gacttgtcactggatttagagtctct

SEQ ID NO: 58 - DNA, 23 bp, Homo sapiens
  TRAC_TCRA-promoter_F1 primer 10.A.10
ctgatcctcttgtcccacagata

SEQ ID NO: 59 - DNA, 22 bp, Homo sapiens
  TRAC_probe (HEX) primer 10.B.6
atccagaaccctgaccctgccg

SEQ ID NO: 60 - DNA, 20 bp, Homo sapiens
  Pan-HLA_GT_F1 primer 8.B.3
aaggagggagctactctcag

SEQ ID NO: 61 - DNA, 24 bp, Homo sapiens
  SV40pA_GT_R1 primer 15.H.2
cctctacagatgtgatatggcttg

SEQ ID NO: 62 - DNA, 27 bp, Homo sapiens
  3xMyc_OE_R1 primer 10.C.4
ggagaacaaaagctcatctctgaggag

SEQ ID NO: 63 - DNA, 29 bp, Homo sapiens
  CtermCysLink_OE_R1 primer 10.D.1
agatccagatccaccggatgtagagcaac

SEQ ID NO: 64 - DNA, 20 bp, Homo sapiens
  Ef1a_intron_GT_F2 primer 15.H.4
tgggtggagactgaagttag

SEQ ID NO: 65 - DNA, 18 bp, Homo sapiens
  HCMVpp65_GT_F2ddPCR primer/probe 21.I.1
tcgacgcccaaaaagcac

SEQ ID NO: 66 - DNA, 17 bp, Homo sapiens
  HCMVpp28_GT_F1 ddPCR primer/probe 21.I.2
tgcctccttgccctttg

SEQ ID NO: 67 - DNA, 19 bp, Homo sapiens
  HCMVpp52_GT_F1 ddPCR primer/probe 21.I.3
cgtccctaacaccaagaag

SEQ ID NO: 68 - DNA, 19 bp, Homo sapiens
  Myc-Tag_GT_R1 ddPCR primer/probe 20.H.10
aaggtcctcctcagagatg

SEQ ID NO: 69 - DNA, 27 bp, Homo sapiens
  Linker-Myc_Probe_Fam ddPCR primer/probe 20.H.9
cttttgttctccagatccagatccacc

SEQ ID NO: 70 - DNA, 23 bp, Homo sapiens
  TRAC-TCRA-ex1-F1 ddPCR primer/probe 10.A.9
ctgatcctcttgtcccacagata

SEQ ID NO: 71 - DNA, 26 bp, Homo sapiens
  TRAC-TCRA-ex1-F1 ddPCR primer/probe
gacttgtcactggatttagagtctct

SEQ ID NO: 72 - DNA, 22 bp, Homo sapiens
  TRAC-probe (HEX) ddPCR primer/probe
atccagaaccctgaccctgccg